European Patent Specification EP 3 638 791 B1, published August 27, 2025. Title: Demethylation of Thebaine and Oripavine with Fungal and Mammalian Cytochrome P450. Applicant: Evolva SA River Stone Biotech ApS. The sequence listing filed with the application follows.

SEQUENCE LISTING (133 sequences)

SEQ ID NO: 1 - protein, 519 aa, Thamnostylum piriforme
MDNKAILRQAVYSYRYHIGIAAAVAIVCQQIYSRVFRVPKNLRHIPAISYWSQMKALLKKEAITPRTKRLVYPLLSKANGLYLNRMPFDWTVYVANPMIAKTVLFKPEFATKMSLIGSFSDDSAVLQFVGKDNIAVSNGHQWKKQRKIMNPAFHRSMPVALFASLMPKVFCMIDETQENGDSVGAIQLMQALTLEALGKAVFGFDFGGLDDKNSVWVKTYNEVFKAFTDFTVFLPRLNAFLRRVSPPHRSRHREMLKLIGLLDEMVDKKRQALLDAKNKSVEKVPEHEKDLLTLMLEAEMDGEGVWEKEELRHNIGILFVAGHDTTANSLAFAVYNLAVNKDVQDKARKEIIDLLGDEPKDVAPTLDDCKHMDYIDMIIKETLRMNAPANDLLARIASEDLELGGVLIPKGTMVSVDFHALHLHPDLWEDSERFNPQRFQDNGEHSKHEGVTWVPFSGGSRQCIGINFSMMEQRVALSTLLRKYEWELPADSIHRNGLVMDQPFSFAPSSLKIKFKKRY

SEQ ID NO: 2 - DNA, 1560 bp, Thamnostylum piriforme
atggacaacaaagcaattttacgacaagccgtttactcgtatcgttaccacatcgggatcgcggcggctgtagctatcgtttgccagcaaatatacagtcgcgtctttcgtgttcccaaaaatttgcgtcatattccagcaattagctattggagtcaaatgaaagcacttttgaaaaaggaggcaatcactccacgtacgaagaggctagtttacccgctgctttcaaaagcgaatggactctacctgaatcgaatgccatttgactggacagtttatgtcgcgaatccaatgattgcgaagactgtcttgtttaagccagagtttgcaaccaaaatgtcattaataggctcattcagcgatgatagtgcagttttgcaatttgttggaaaggataatattgcggtatcaaacggtcaccagtggaaaaagcaaagaaagattatgaaccctgctttccatcgatcaatgccggtagctctctttgcaagtctcatgccaaaggttttttgtatgattgatgaaacacaagagaacggtgattctgttggtgccatacaacttatgcaggcccttactcttgaagcgcttggaaaagcagttttcggttttgattttggaggattggacgataaaaattctgtttgggtcaagacatacaacgaagtattcaaggcatttacagacttcacggtattccttccacgacttaatgcttttcttcggcgggtaagcccaccgcatcgaagtcgtcatagagaaatgctcaagttgatcggccttctggatgaaatggtggacaaaaagagacaagcgctcttggatgccaagaataaatccgtcgagaaagtgcctgagcatgaaaaggatctacttactctcatgctcgaggctgaaatggatggtgaaggtgtttgggaaaaagaagaattacggcacaatatcgggatattattcgtggcagggcatgatacaaccgccaattcattggcatttgcggtttacaatctagccgtcaacaaagacgtacaagataaggcccgcaaagaaattatcgacttactaggagacgagcctaaggatgttgcgcccaccttggatgactgcaaacatatggattatatcgatatgattatcaaagagacgctccgcatgaatgctcctgcaaatgacttgcttgctcgaatagcatcggaagacttggaactaggaggggttttaatacccaaggggacaatggtctcggtcgactttcacgcactgcaccttcaccctgatttatgggaggattcagagcgtttcaacccgcagcgatttcaagataatggagagcatagcaaacacgaaggagtaacatgggttccttttagtggaggctcaagacaatgcattggaatcaattttagtatgatggagcaacgggtggccctatcgacgctattgagaaaatatgaatgggagctacctgctgattctatccaccgtaatggacttgtgatggatcaaccttttagttttgcaccaagctctctcaaaattaagtttaaaaaacgttattga

SEQ ID NO: 3 - DNA, 1560 bp, Thamnostylum piriforme
atggataataaagctattttgagacaagctgtttattcttatagataccatattggtattgctgctgctgttgctattgtttgtcaacaaatttattctagagtttttagagttccaaaaaatttgagacatattccagctatttcttattggtctcaaatgaaagcattgttgaaaaaagaagctattactccaagaactaaaagattggtttatccattgttgtctaaagctaatggtttgtatttgaatagaatgccatttgattggactgtttatgttgctaatccaatgattgctaaaactgttttgtttaaaccagaatttgctactaaaatgtctttgattggttctttttctgatgattctgctgttttgcaatttgttggtaaagataatattgctgtttctaatggtcatcaatggaaaaaacaaagaaaaattatgaatccagcttttcatagatctatgccagttgctttgtttgcttctttgatgccaaaagttttttgtatgattgatgaaactcaagaaaatggtgattctgttggtgctattcaattgatgcaagcattgactttggaagcattgggtaaagctgtttttggttttgattttggtggtttggatgataaaaattctgtttgggttaaaacttataatgaagtttttaaagcatttactgattttactgtttttttgccaagattgaatgcttttttgagaagagtttctccaccacatagatctagacatagagaaatgttgaaattgattggtttgttggatgaaatggttgataaaaaaagacaagcattgttggatgctaaaaataaatctgttgaaaaagttccagaacatgaaaaagatttgttgactttgatgttggaagctgaaatggatggtgaaggtgtttgggaaaaagaagaattgagacataatattggtattttgtttgttgctggtcatgatactactgctaattctttggcttttgctgtttataatttggctgttaataaagatgttcaagataaagctagaaaagaaattattgatttgttgggtgatgaaccaaaagatgttgctccaactttggatgattgtaaacatatggattatattgatatgattattaaagaaactttgagaatgaatgctccagctaatgatttgttggctagaattgcttctgaagatttggaattgggtggtgttttgattccaaaaggtactatggtttctgttgattttcatgctttgcatttgcatccagatttgtgggaagattctgaaagatttaatccacaaagatttcaagataatggtgaacattctaaacatgaaggtgttacttgggttccattttctggtggttctagacaatgtattggtattaatttttctatgatggaacaaagagttgctttgtctactttgttgagaaaatatgaatgggaattgccagctgattctattcatagaaatggtttggttatggatcaaccattttcttttgctccatcttctttgaaaattaaatttaaaaaaagatattga

SEQ ID NO: 4 - protein, 509 aa, Thamnostylum piriforme
MAILQNLVLQSDQRHLGVVTAAVFLSAYALYRHESKKELGNECPTVPYTNPMFGSTDEYRKNPAAFVEKWSAALGPVFRVHIFGRMQTVVSGRYVREVLFNDNFSFVEGIRTRFDLRLLTGIPNSHLNDKDVREVVVKSLTAQMKKYTPRAVHYLSVGLQEALGDLKDPRTLDNLFLTVQNMVAKASASIFVGEELCNNIELVDTFKHVTSDIGSEIRLDNTWLEFFKTINQIRMWYVGKHSPRVTKHRRQLIQAMAPEIDRRLQGLAGNDPSWTRPEDILQEIMENYPSPSTVPADIYTYYANWMIVLIFASVHTTTEHATIVLYRLLQQPELIDELLQEQKEALGQGTVFTGEVIRKLVKLDSVCRESLRIKNEYFGLPHRNMSHENISLSNGVVIKPGDNVMLNVWTNHHDSDLQKDVHGNHDKFEPFRYVNADRPATKIGDDYLIFGEGKHACPGRWFALQEIKTIVSVLIRDYTLTPCGPIVFPSGTSTGIPSGEVTIQRKSEV

SEQ ID NO: 5 - DNA, 1530 bp, Thamnostylum piriforme
atggcaattcttcaaaaccttgtcctacaatctgatcagcgacaccttggtgtcgttacagctgctgtttttttgtcagcgtacgcgctctatcgacatgagtcgaaaaaggaactggggaatgagtgtcctactgtaccctataccaatccaatgttcggttccactgacgaatatcgcaagaatccagccgcatttgttgaaaaatggagcgctgcacttggcccagtatttcgcgttcatatctttggcagaatgcagacggtagtttcgggccgttatgtccgcgaagttttgttcaacgacaactttagttttgtggaaggaatccggacacggtttgaccttcgattgctcaccggtatacctaacagtcacctcaatgacaaagatgttcgagaggttgttgtcaagtcgttgactgcgcaaatgaagaagtatacaccgcgcgcagtacactacctcagcgttggcttgcaagaggcactaggagatttgaaagatcctcgaactcttgacaacctattcttgactgttcaaaacatggtcgccaaagctagcgcctccatcttcgtcggtgaagaactttgtaacaatattgagttggttgacacattcaagcacgttacaagcgacattggttcggagatacgtctcgacaacacctggctggaattctttaaaacaataaaccaaattcgaatgtggtacgttggcaagcattctcccagagtgacaaagcacagacgacagctcatacaggcgatggcacctgaaatcgacagacggctgcaaggtcttgcagggaatgatccttcttggaccagaccagaagacattttgcaagagattatggaaaactatccttccccgtccactgtaccagcagatatttacacctattatgccaattggatgattgtgttgatatttgcatccgttcacacgaccactgagcatgcaacaattgtcctttaccgtttactccaacagcccgagcttatcgacgagcttcttcaagaacaaaaggaggcccttggccaaggcactgtatttacaggcgaggtcattcgcaaactggtgaaactggatagcgtgtgtcgtgagtctttgcggatcaaaaacgagtactttggtcttccacacaggaatatgtctcatgaaaatatttctttgagcaatggagttgttatcaaaccaggcgacaatgtcatgctgaatgtttggacaaaccatcatgacagtgacttgcaaaaggatgtacacggcaaccatgacaagtttgaacctttccgttacgttaatgctgatcgccctgcaacgaagattggtgatgattacttgatatttggggagggaaagcacgcttgccccggtcgatggtttgctttacaagaaattaagacgattgtatcagtactaattcgagattacacgctaacaccatgtggtccaattgtgtttccatccggcacaagtactggtattccaagtggagaagtgacaattcaacgaaagtcagaagtgtaa

SEQ ID NO: 6 - DNA, 1530 bp, Thamnostylum piriforme
atggctattttgcaaaatttggttttgcaatctgatcaaagacatttgggtgttgttactgctgctgtttttttgtctgcttatgctttgtatagacatgaatctaaaaaagaattgggtaatgaatgtccaactgttccatatactaatccaatgtttggttctactgatgaatatagaaaaaatccagcagcttttgttgaaaaatggtctgctgctttgggtccagtttttagagttcatatttttggtagaatgcaaactgttgtttctggtagatatgttagagaagttttgtttaatgataatttttcttttgttgaaggtattagaactagatttgatttgagattgttgactggtattccaaattctcatttgaatgataaagatgttagagaagttgttgttaaatctttgactgctcaaatgaaaaaatatactccaagagctgttcattatttgtctgttggtttgcaagaagcattgggtgatttgaaagatccaagaactttggataatttgtttttgactgttcaaaatatggttgctaaagcatctgcttctatttttgttggtgaagaattgtgtaataatattgaattggttgatacttttaaacatgttacttctgatattggttctgaaattagattggataatacttggttggaattttttaaaactattaatcaaattagaatgtggtatgttggtaaacattctccaagagttactaaacatagaagacaattgattcaagctatggctccagaaattgatagaagattgcaaggtttggctggtaatgatccatcttggactagaccagaagatattttgcaagaaattatggaaaattatccatctccatctactgttccagcagatatttatacttattatgctaattggatgattgttttgatttttgcttctgttcatactactactgaacatgctactattgttttgtatagattgttgcaacaaccagaattgattgatgaattgttgcaagaacaaaaagaagcattgggtcaaggtactgtttttactggtgaagttattagaaaattggttaaattggattctgtttgtagagaatctttgagaattaaaaatgaatattttggtttgccacatagaaatatgtctcatgaaaatatttctttgtctaatggtgttgttattaaaccaggtgataatgttatgttgaatgtttggactaatcatcatgattctgatttgcaaaaagatgttcatggtaatcatgataaatttgaaccatttagatatgttaatgctgatagaccagctactaaaattggtgatgattatttgatttttggtgaaggtaaacatgcttgtccaggtagatggtttgctttgcaagaaattaaaactattgtttctgttttgattagagattatactttgactccatgtggtccaattgtttttccatctggtacttctactggtattccatctggtgaagttactattcaaagaaaatctgaagtttaa

SEQ ID NO: 7 - protein, 514 aa, Lichtheimia ramosa
MTEIKEHIYRYRHYIGVAAAVALVCQQVYYRIFRIPKNLRHIPAIPYGQQLKALRSDEALTSRTKRLVFPLLSKCNGVYLNRMPFKWTIYVADPEIARAILFKPEFGHKTRSVTDSLDKNSSLFEFVGDDNIAIVNGHEWKEQRKIMNPAFHRATPVGMFGSLMPKVFRLVEEQPTLPALDLMQKLTLDALGKSVFGFEFGALDDPDSVWVKTYRQVFDSFTDVFSLVFPRLDPIYRYFSAKHREQYNAVYKLIDLLDGMADKKRSMLQDASNSDIKDVPDHEKDLLQLMLEAELRGEGSWTKRELRHNMAIFFVAGQDTTSHALTFCLYLLAKNQDIQKKAREEILNVFGDEPKDVFPTLEDCKKLNYLDMVIKESMRIYPPANDVLARDVNEDLNVKGVFIPKGSMVSVDIHALHHRPDLWHEPDKFNPDRFLPGGEHDSHVGVTYAPFSSGSRQCIALKFATMQQRVVLSMLLRKYEWELPKDSKHKDSIQFQIPFNIAPKDLELTFHKRY

SEQ ID NO: 8 - DNA, 1545 bp, Lichtheimia ramosa
atgactgaaattaaagaacatatttatagatatagacattatattggtgttgctgctgctgttgctttggtttgtcaacaagtttattatagaatttttagaataccaaaaaatttgagacatattccagctattccatatggtcaacaattgaaagcattgagatctgatgaagcattgacttctagaactaaaagattggtttttccattgttgtctaaatgtaatggtgtttatttgaatagaatgccatttaaatggactatttatgttgctgatccagaaattgctagagctattttgtttaaaccagaatttggtcataaaactagatctgttactgattctttggataaaaattcttctttgtttgaatttgttggtgatgataatattgctattgttaatggtcatgaatggaaagaacaaagaaaaattatgaatccagcttttcatagagctactccagttggtatgtttggttctttgatgccaaaagtttttagattggttgaagaacaaccaactttgccagctttggatttgatgcaaaaattgactttggatgctttgggtaaatctgtttttggttttgaatttggtgctttggatgatccagattctgtttgggttaaaacttatagacaagtttttgattcttttactgatgttttttctttggtttttccaagattggacccaatttatagatatttttctgctaaacatagagaacaatataatgctgtttataaattgattgatttgttggatggtatggctgataaaaaaagatctatgttgcaagatgcttctaattctgatattaaagatgttccagatcatgaaaaagatttgttgcaattgatgttggaagctgaattgagaggtgaaggttcttggactaaaagagaattgagacataatatggctattttttttgttgctggtcaagatactacttctcatgctttgactttttgtttgtatttgttggctaaaaatcaagatattcaaaaaaaagctagagaagaaattttgaatgtttttggtgatgaaccaaaagatgtttttccaactttggaagattgtaaaaaattgaattatttggatatggttattaaagaatctatgagaatttatccaccagctaatgatgttttggctagagatgttaatgaagatttgaatgttaaaggtgtttttattccaaaaggttctatggtttctgttgatattcatgctttgcatcatagaccagatttgtggcatgaaccagataaatttaatccagatagatttttgccaggtggtgaacatgattctcatgttggtgttacttatgctccattttcttctggttctagacaatgtattgctttgaaatttgctactatgcaacaaagagttgttttgtctatgttgttgagaaaatatgaatgggaattgccaaaagattctaaacataaagattctattcaatttcaaattccatttaatattgctccaaaagatttggaattgacttttcataaaagatattaa

SEQ ID NO: 9 - protein, 701 aa, Thamnostylum piriforme
MAQSSPALLDSLDIVFLGTIGLGTIAWFARRQIAERIFGSKDDANKNVGNGNAPTAPKRERNFVKVMQEQGRKVIFFYGSQTGTAEDYASRLAKECSQKYGVSCMTADIELYDLTYLDTVPEDFLVFFIMATYGEGEPTDNAVDFWEQLTEEEPQFSEGDTLGNLRYVVFGLGNKTYEHYNEVARRMDKLLTKLGAKRIGERGEGDDDASLEEDFLAWQDSMWPAFCDALGVDESNGSSGPRQAMYAVEELEGQEAVYLGELGEKPKEGVKVVYDAKRPYNAPLVSQDLFKNTDRHCLHIDIDVSDSNLSYQTGDHIAIWPTNSDDEVARLASLLGLTDKLDTSVMVKAIDSTASKQYPFPVPATYRSIFRHYLDICAPASRQTLMSLVEYAPTEASKEALRLLSKDKDEYRLKVGEAVRNLGEVLELAAGADARPGLFSTVPFDLIVESVSRLQPRYYSISSSAKESPKVIAVTAVTLTYNPDPTPERTVYGVNTNYLWQIHAAKHNVNDGQRYPTYDLAGPRNALQGAKVPVHIRRSQFKLPRNPTVPVIMVGPGTGVAPFRGFVRERAAQKTDGKPVGPTLLFFGCRNSQQDFLYKDEWPELFATLGDESRIVTAFSRETPQKVYVQHRLQENGEELWNLLQKGAYIYVCGDAKNMARDVNQTFVNFAIEFGGQTEEKAHDYVKNLRNSGRYQEDVWS

SEQ ID NO: 10 - DNA, 2106 bp, Thamnostylum piriforme
atggcgcaatcgtcacctgctcttctcgactctttggacattgtgttcctcggaacgattggtcttggcaccattgcctggtttgcacgtcgacagattgcagaacgaatctttggatccaaggatgatgcaaacaaaaacgtcggcaatggcaacgctcctactgcgccgaagcgagagcgcaactttgtcaaagtgatgcaagaacagggtcgcaaagtcatcttcttttacggttcgcagaccggcacggctgaagactacgcttctcggctagccaaggaatgctcgcaaaagtacggtgtgagctgtatgacagccgatatcgagctgtacgatctgacctatctggacactgtgcctgaagacttcttggtgttcttcatcatggcgacgtacggcgagggtgagcccaccgacaacgccgtcgacttctgggagcaattgacggaggaggagccccagttctcggaaggcgacactttgggtaacttgcgctatgtggtgtttggcctgggcaacaagacgtacgagcattacaacgaggtggctcgtcggatggacaagctgctgacgaagctgggtgccaagcgcattggcgagcggggcgaaggcgacgacgatgcttcgttggaagaggactttttggcgtggcaagatagcatgtggcccgcgttctgcgacgctctgggcgtggacgagagcaacggatccagcgggccccgccaggccatgtacgcggtggaggagcttgagggccaagaggccgtgtatctcggcgagctcggagagaagcccaaggagggcgttaaggttgtgtacgacgccaagcgcccctacaacgcgccgctcgtctcgcaggacctcttcaaaaacacagaccgccattgcctgcacatcgacatcgacgtctcggactccaacctgtcgtaccagaccggcgaccacatcgcgatctggcccaccaacagcgatgacgaagtggcgcgtctcgcttccctgctcggcctgaccgacaagctcgacaccagcgtcatggtcaaggccatcgactccaccgcctccaagcagtacccattccccgtgcccgccacctaccggtccattttccgccactacctcgacatctgcgcgcccgcgtcgcgccagacgctcatgtcgctggtcgagtacgcgcccacggaggcgtccaaagaggccttgcgtctgctgtccaaggacaaggacgagtaccgcctcaaggtcggcgaggctgtccgcaacctgggcgaggtgcttgagctggctgccggagcggatgcccgaccgggcctgttctccaccgtgccctttgacctgatcgtcgagagcgtgtcgcgcctgcagccccgctactactccatctcctcatcggccaaggagtcgcccaaggtcattgccgtcaccgccgtcaccttgacatacaacccagaccccacgcccgagcgcaccgtgtatggcgtcaacaccaactatttgtggcaaatccacgccgccaagcacaacgtcaacgacggccagcgctaccccacctacgacctggctggcccgcgcaacgccctgcaaggcgccaaggtccccgtccacatccgccgctcgcagttcaagctgccgcgcaaccccaccgtccctgtcatcatggtcggcccaggcaccggtgtcgcgcccttccgtggctttgttcgcgagcgtgccgcccaaaagaccgacggcaagcccgtcggccccaccctgctcttcttcggctgccgcaactcgcaacaggacttcttgtacaaggacgagtggcccgagctgttcgccacccttggcgacgagtcgcgtatcgtgactgcattctcgcgcgagactccccagaaggtctacgtccagcaccggctccaggagaacggcgaggagctgtggaatctgctgcaaaagggagcctacatttacgtgtgcggtgacgcaaagaacatggcacgcgatgtcaaccagaccttcgtcaactttgcgatcgagtttggcggccagaccgaagagaaggcgcatgactacgtcaagaacctcagaaacagcggtcgataccaggaggatgtgtggagctaa

SEQ ID NO: 11 - DNA, 2106 bp, Thamnostylum piriforme
atggctcaatcttctccagctttgttggattctttggatattgtttttttgggtactattggtttgggtactattgcttggtttgctagaagacaaattgctgaaagaatttttggttctaaagatgatgctaataaaaatgttggtaatggtaatgctccaactgctccaaaaagagaaagaaattttgttaaagttatgcaagaacaaggtagaaaagttatttttttttatggttctcaaactggtactgctgaagattatgcttctagattggctaaagaatgttctcaaaaatatggtgtttcttgtatgactgctgatattgaattgtatgatttgacttatttggatactgttccagaagattttttggttttttttattatggctacttatggtgaaggtgaaccaactgataatgctgttgatttttgggaacaattgactgaagaagaaccacaattttctgaaggtgatactttgggtaatttgagatatgttgtttttggtttgggtaataaaacttatgaacattataatgaagttgctagaagaatggataaattgttgactaaattgggtgctaaaagaattggtgaaagaggtgaaggtgatgatgatgcttctttggaagaagattttttggcttggcaagattctatgtggccagctttttgtgatgctttgggtgttgatgaatctaatggttcttctggtccaagacaagctatgtatgctgttgaagaattggaaggtcaagaagctgtttatttgggtgaattgggtgaaaaaccaaaagaaggtgttaaagttgtttatgatgctaaaagaccatataatgctccattggtttctcaagatttgtttaaaaatactgatagacattgtttgcatattgatattgatgtttctgattctaatttgtcttatcaaactggtgatcatattgctatttggccaactaattctgatgatgaagttgctagattggcttctttgttgggtttgactgataaattggatacttctgttatggttaaagctattgattctactgcttctaaacaatatccatttccagttccagctacttatagatctatttttagacattatttggatatttgtgctccagcttctagacaaactttgatgtctttggttgaatatgctccaactgaagcatctaaagaagcattgagattgttgtctaaagataaagatgaatatagattgaaagttggtgaagctgttagaaatttgggtgaagttttggaattggctgctggtgctgatgctagaccaggtttgttttctactgttccatttgatttgattgttgaatctgtttctagattgcaaccaagatattattctatttcttcttctgctaaagaatctccaaaagttattgctgttactgctgttactttgacttataatccagatccaactccagaaagaactgtttatggtgttaatactaattatttgtggcaaattcatgctgctaaacataatgttaatgatggtcaaagatacccaacttatgatttggctggtccaagaaatgctttgcaaggtgctaaagttccagttcatattagaagatctcaatttaaattgccaagaaatccaactgttccagttattatggttggtccaggtactggtgttgctccatttagaggttttgttagagaaagagctgctcaaaaaactgatggtaaaccagttggtccaactttgttgttttttggttgtagaaattctcaacaagattttttgtataaagatgaatggccagaattgtttgctactttgggtgatgaatctagaattgttactgctttttctagagaaactccacaaaaagtttatgttcaacatagattgcaagaaaatggtgaagaattgtggaatttgttgcaaaaaggtgcttatatttatgtttgtggtgatgctaaaaatatggctagagatgttaatcaaacttttgttaattttgctattgaatttggtggtcaaactgaagaaaaagctcatgattatgttaaaaatttgagaaattctggtagataccaagaagatgtttggtcttag

SEQ ID NO: 12 - protein, 707 aa, Thamnostylum piriforme
MSKKPTTFAISPLDLLLLGTLGIGALLYITRKLRAAPPPAAGDAARPSDKAPSNKPERNFVKLMEQQKRRVIFFYGSQTGTAEDYASRLAKESSQKYGVSSMAADIELYDLSYLDTVPEDKLVVFVMATYGEGEPTDNAVDFWETLTDEAPMFSLGEELAPLRNLNYIVFGLGNKTYEHYNEVARVLDKRLAALGATRHGVRGEGDDDASLEEDFLAWQEDMWPAFCAALNVDESNAQAGPRQAMYGVKELEGHDENGLFLGELGEWLQPEQLQKQTAVHDAKHPYLAPIAASRDLFSHAADRHCLHLEVDIASSNLTYQTGDHIAIWPTNNDVEVLRLATVLGLADKLDTAIMVKALDSAASKKYPFPVPTTYRAAFKHYLDICSPASRQTLISLVDYAPTASSKDALHKLATDKDAYKTQVSEAARNLAEVLELCQDDEGTTAAPGFFSTVPFDLIVESVSRLQPRYYSISSSSLTSPKSVAVTAVTLSYQPSTTKSRTVYGVNTNYLWRIHAPHDASVPAYDLDGPRNTLQGKKVPVHIRRSTFKLPRNTKLPVIMVGPGTGVAPFRGFIHDRVHQKQSGKEVGPTVLFYGCRHSKQDFLYAEEWPALFEALGEGSQLITAFSRESAQKVYVQHRLKEHGEQMWKYIEQGAYIYVCGDAKNMARDVQQTFIEFAQALGNKTESQAQDYVKNLRNTGRYQEDVWS

SEQ ID NO: 13 - DNA, 2124 bp, Thamnostylum piriforme
atgtcaaaaaagcctactacgtttgccatcagtccgcttgacctgctgctgctgggcacgctggggattggcgccctcctctacataacgagaaagctcagggcagcgcctccacccgcggctggcgacgcagcacgcccatccgataaagcgccgagcaacaagcctgaacggaacttcgtcaagctgatggagcagcagaaacggcgcgtcattttcttttacggatctcagacaggcactgcagaggattacgcctcacggctggccaaggaaagctcccagaaatatggcgtgagcagcatggcggccgacattgagctgtacgacctcagctacctggacaccgtacccgaggacaagctggtggtgtttgtcatggccacctacggcgagggcgagccgaccgacaacgccgtcgacttctgggaaacgctgaccgacgaagcgcccatgttctcgctgggagaagagttagcgccgctgcgaaacctgaactacattgtgtttggactgggcaacaagacctacgagcattacaacgaagtggcccgtgtccttgacaagcgccttgcggctctgggcgccacgcggcacggcgtgcggggcgaaggcgacgacgacgcttctctggaagaggactttctggcatggcaggaggatatgtggcctgcgttctgcgctgcgttgaatgtcgacgagagcaatgcgcaggcgggtccgcggcaggcgatgtacggcgtgaaggagctcgagggccacgacgaaaacggtctgtttttgggagagctgggcgagtggctgcagcctgaacagctgcagaagcagacagccgtgcatgacgccaaacatccgtacctggcccccatcgctgcctcgcgtgatctgttcagccacgccgccgaccgccactgcctgcacctggaagtcgacatcgccagcagcaacctcacctaccagaccggcgaccacatcgccatctggcccaccaacaacgacgtcgaggtgctgcgcctggccaccgtgctgggtctggcggacaagctggacaccgccatcatggtcaaggctttggacagcgccgcctccaaaaagtaccccttccctgtccccaccacgtaccgcgccgcattcaaacactacctcgatatctgctctcctgcatctcgccagacgctgatctcgttggtcgactacgcgcccaccgcgtcgtccaaggacgcgctgcacaaactggcaaccgacaaggacgcctataaaacgcaggtcagcgaggccgcgcgcaacctggccgaggtgctggagctgtgccaggacgacgagggcacgacagccgcgcctggcttcttttccaccgtgcccttcgacctgattgtcgaaagcgtgtcgcgtctccagccacggtactactccatctcgtcatcctcgctcacctctccgaaatccgtcgctgtcaccgccgtcacgctgtcctaccagccatccaccaccaaaagccgcaccgtctacggcgtcaacaccaactacctgtggcgcatccatgcaccgcacgacgcgtccgtcccagcctacgatctcgacggtccgcgcaacactctccaaggcaaaaaggtgccggtgcatatccgccgatcgaccttcaaactgccgcgcaacaccaagcttcccgtcatcatggtggggcctggcacgggcgtcgcgccgttccgcgggttcatccatgatcgcgtgcatcagaagcaaagtggcaaggaggtggggcccacggtgctgttctatggatgccgccattccaaacaggactttttgtatgcggaagaatggccggcgctctttgaggcgttgggcgaaggatcgcagttgatcaccgcgttttcgcgagaatcagcgcaaaaggtctatgttcagcaccggttaaaggagcacggcgagcagatgtggaagtatatcgagcagggagcgtatatctacgtttgcggtgacgccaaaaacatggccagggacgtgcagcagacgttcattgagtttgcacaggctctgggaaacaaaacggaaagccaggcacaggactacgtcaagaatctgcgaaacaccggacgctaccaggaggacgtgtggtcgtag

SEQ ID NO: 14 - DNA, 2124 bp, Thamnostylum piriforme
atgtctaaaaaaccaactacttttgctatttctccattggatttgttgttgttgggtactttgggtattggtgctttgttgtatattactagaaaattgagagctgctccaccaccagctgctggtgatgctgctagaccatctgataaagctccatctaataaaccagaaagaaattttgttaaattgatggaacaacaaaaaagaagagttatttttttttatggttctcaaactggtactgctgaagattatgcttctagattggctaaagaatcttctcaaaaatatggtgtttcttctatggctgctgatattgaattgtatgatttgtcttatttggatactgttccagaagataaattggttgtttttgttatggctacttatggtgaaggtgaaccaactgataatgctgttgatttttgggaaactttgactgatgaagctccaatgttttctttgggtgaagaattggctccattgagaaatttgaattatattgtttttggtttgggtaataaaacttatgaacattataatgaagttgctagagttttggataaaagattggctgctttgggtgctactagacatggtgttagaggtgaaggtgatgatgatgcttctttggaagaagattttttggcttggcaagaagatatgtggccagctttttgtgctgctttgaatgttgatgaatctaatgctcaagctggtccaagacaagctatgtatggtgttaaagaattggaaggtcatgatgaaaatggtttgtttttgggtgaattgggtgaatggttgcaaccagaacaattgcaaaaacaaactgctgttcatgatgctaaacatccatatttggctccaattgctgcttctagagatttgttttctcatgctgctgatagacattgtttgcatttggaagttgatattgcttcttctaatttgacttatcaaactggtgatcatattgctatttggccaactaataatgatgttgaagttttgagattggctactgttttgggtttggctgataaattggatactgctattatggttaaagcattggattctgctgcttctaaaaaatatccatttccagttccaactacttatagagctgcttttaaacattatttggatatttgttctccagcttctagacaaactttgatttctttggttgattatgctccaactgcttcttctaaagatgctttgcataaattggctactgataaagatgcttataaaactcaagtttctgaagctgctagaaatttggctgaagttttggaattgtgtcaagatgatgaaggtactactgctgctccaggttttttttctactgttccatttgatttgattgttgaatctgtttctagattgcaaccaagatattattctatttcttcttcttctttgacttctccaaaatctgttgctgttactgctgttactttgtcttatcaaccatctactactaaatctagaactgtttatggtgttaatactaattatttgtggagaatccatgctccacatgatgcttctgttccagcttatgatttggatggtccaagaaatactttgcaaggtaaaaaagttccagttcatattagaagatctacttttaaattgccaagaaatactaaattgccagttattatggttggtccaggtactggtgttgctccatttagaggttttattcatgatagagttcatcaaaaacaatctggtaaagaagttggtccaactgttttgttttatggttgtagacattctaaacaagattttttgtatgctgaagaatggccagctttgtttgaagcattgggtgaaggttctcaattgattactgctttttctagagaatctgctcaaaaagtttatgttcaacatagattgaaagaacatggtgaacaaatgtggaaatatattgaacaaggtgcttatatttatgtttgtggtgatgctaaaaatatggctagagatgttcaacaaacttttattgaatttgctcaagcattgggtaataaaactgaatctcaagctcaagattatgttaaaaatttgagaaatactggtagataccaagaagatgtttggtcttag

SEQ ID NO: 15 - DNA, 2085 bp, Thamnostylum piriforme
atggcaaaaaatactacattaaacaagcaagtggtgcttctcatcagtgccctgggcctgagcgctgttgcctacatggccagccgatacttttttggaaacagcgcaagcacccctgaacaatcgaaaaagcccattcaaccagaagaaaaagaagacgaatcaaactttgtgcaaaccatgaagaagcagaatcgtaaagtagtgatcttttatggttcgcaaacaggcacggctgaagattgtgcgcagcgacttggcaagcagtgcaaaaagcaattcggcgttcctgctttggttcttgatatcgaacaatgcaacatgtcgtacttggatcagattcccgaggactgtgttgcgatatttgtcatggcaacttatggcgaaggtgaacccactgacaacgccactgacttttgggaaatgcttgaagcccatcctgaattttcccaaagcgacaacctcaagaatctccgatacttcatcttcggacttggcaacagctcctatacctattacaactgggtctccaaaactgtcgacaagaaactcactgaattaggcgcgacacgacttggcaaacttggcttgggcgacgacgaaaagtcgctcgaagacgactttgaagcatggcaggaaggcatgtggcctatttttggagaagctgtggaaacggacgccgccagcaatatcagcggcggacacgagcccacataccatgtggtggagctaaccgaacatgacggccacgtgtattctggtgaattgggagacaaatcgcaagctctctatagcggcaagaagccttacccagcacctattaccacgcgcgatttgttgaacggatcggatcgccactgtctacacctggaagtcgatatcagtggatcaggcatgagctataccactggcgatcatattgccatctggcccacaaacagcgaagacgaggtcttgagcttggcacgcgccattggtctcgaaaacaagctggataccgtcatttgcgttactgctgcggatgagacgtccgccaagcaatcaccgttccctcagccaacaacataccgtgccatgctgcgacactacttggatatttgccaaatgccatcacggcagacactggagatgctcgtaccttttgcaccgtcgcccgaagctgcagagactctagaaaagctggcaaaggacaaggatgagcatcgtcgagtggttctgggaccagttcgtaacttggctgctgtgctgagttatgcgtcgtcgggcgctgcatacaagatcccatccgatgtgctgcttgagtgccttggtcgactacagccccgatattactcgatttcctcctctgccttggagagcccaaacagtgtcagtgtcactgccgttacactcaaattcaaccccgaaccaacgcctgagcgcactgtctttggcgtcaataccaactacctgtgggccgtccataccgcgctcaacgatgacgacgaggcaatccaagttgaaaccgagtattccatcggtggacctaacggtcaatactttgacgagaagctcaaaactgcaagattgcctgttcacatccgccaatcaaacttcaagctgccagcagacacaactaagccagtgatcatgattggccccggcaccggtgtcgctcctttccgagccttcgttcgcgagcgtgcctatcaaaagaagcaccttggcaaatccatcggtccaactattctgtactttggctgccgacgttccaacgaggactttttgtatcaggaagagtggccagagctctttaacgaattgggcggctcctctcgattgatcactgcattctcccgggaaacggatcgaaaagtatacgtccaagacaagctcaacgagaacggcccagagacttgggatttgattaataacaagggcgcctatgtctatgtttgtggcgacgctaagcgtatggccaaagacgtccagtccgcacttgttagttttgcaaagcagtatggcagctatgacgacgctggtgcagctgactacatcagcaagttaagagatgccggacgatatcaagaagacgtctgggcataa

SEQ ID NO: 16 - protein, 710 aa, Cunninghamella elegans
MAQQTPAVIDTLDLILLGSIGLGTIAWFTRRQLSERLFGTGQSNATPKPTTPQAPKRERNFVKVMEQQGRKVIFFYGSQTGTAEDFASRLAKQCSQKYGVSCMTADIEMYDLSYLDTLSEDSLVCFVMATYGEGEPTDNAVDFWEQFITDESPVFSEGGETLENLRYLMFGLGNKTYEHYNAVARILDKKLTGLGAKRIGERGEGDDDGSLEEDFLAWQESMWPTFCDALGVDENNAQQGPRQASYSVDELKEEYKNDDVYFGELGTKSKDSSRVVYDAKRPYNAPITTRELFNSSERHCLHVDIDISGTNLSYQTGDHVAMWPTNNEDEVLRLANILGLQDKLDNVISVKAIDPAAPKQHPFPVPTTYRAIFRHYIDICAPASRQSLMSFVEFAPTDSAKDLLKLLATDKDEYRLKVGEAVRNLGEVLELVSGNDKDTQPGSFTSVPFDLIVETIPRLQPRYYSISSSSKENSSIISATCVTLAYQPDPTPDRTVYGVNTNFLYRIHTQSSDNDIQGLPKYDLAGPRKAFLNEQGQSHKLPIHIRRSQFKLPRNTSCPVIMIGPGTGVAPFRGFVRERALQKKEGKSVGPTVLFFGNRHSEHDFLYSDEWPELFNTLGDDSKLITAFSRETEHKVYVQHRLEENGKDIWQLLEKGAYIYVCGDARNMARDVNQTFVNLAMEYGEKTEQKALDYVKSLRNTGRYQEDVWS

SEQ ID NO: 17 - DNA, 2133 bp, Cunninghamella elegans
atggctcaacaaactccagctgttattgatactttggatttgattttgttgggttctattggtttgggtactattgcttggtttactagaagacaattgtctgaaagattgtttggtactggtcaatctaatgctactccaaaaccaactactccacaagctccaaaaagagaaagaaattttgttaaagttatggaacaacaaggtagaaaagttatttttttttatggttctcaaactggtactgctgaagattttgcttctagattggctaaacaatgttctcaaaaatatggtgtttcttgtatgactgctgatattgaaatgtatgatttgtcttatttggatactttgtctgaagattctttggtttgttttgttatggctacttatggtgaaggtgaaccaactgataatgctgttgatttttgggaacaatttattactgatgaatctccagttttttctgaaggtggtgaaactttggaaaatttgagatatttgatgtttggtttgggtaataaaacttatgaacattataatgctgttgctagaattttggataaaaaattgactggtttgggtgctaaaagaattggtgaaagaggtgaaggtgatgatgatggttctttggaagaagattttttggcttggcaagaatctatgtggccaactttttgtgatgctttgggtgttgatgaaaataatgctcaacaaggtccaagacaagcatcttattctgttgatgaattgaaagaagaatataaaaatgatgatgtttattttggtgaattgggtactaaatctaaagattcttctagagttgtttatgatgctaaaagaccatataatgctccaattactactagagaattgtttaattcttctgaaagacattgtttgcatgttgatattgatatttctggtactaatttgtcttatcaaactggtgatcatgttgctatgtggccaactaataatgaagatgaagttttgagattggctaatattttgggtttgcaagataaattggataatgttatttctgttaaagctattgatccagctgctccaaaacaacatccatttccagttccaactacttatagagctatttttagacattatattgatatttgtgctccagcttctagacaatctttgatgtcttttgttgaatttgctccaactgattctgctaaagatttgttgaaattgttggctactgataaagatgaatatagattgaaagttggtgaagctgttagaaatttgggtgaagttttggaattggtttctggtaatgataaagatactcaaccaggttcttttacttctgttccatttgatttgattgttgaaactattccaagattgcaaccaagatattattctatttcttcttcttctaaagaaaattcttctattatttctgctacttgtgttactttggcttatcaaccagatccaactccagatagaactgtttatggtgttaatactaattttttgtatagaatccatactcaatcttctgataatgatattcaaggtttgccaaaatatgatttggctggtccaagaaaagcatttttgaatgaacaaggtcaatctcataaattgccaattcatattagaagatctcaatttaaattgccaagaaatacttcttgtccagttattatgattggtccaggtactggtgttgctccatttagaggttttgttagagaaagagctttgcaaaaaaaagaaggtaaatctgttggtccaactgttttgttttttggtaatagacattctgaacatgattttttgtattctgatgaatggccagaattgtttaatactttgggtgatgattctaaattgattactgctttttctagagaaactgaacataaagtttatgttcaacatagattggaagaaaatggtaaagatatttggcaattgttggaaaaaggtgcttatatttatgtttgtggtgatgctagaaatatggctagagatgttaatcaaacttttgttaatttggctatggaatatggtgaaaaaactgaacaaaaagcattggattatgttaaatctttgagaaatactggtagataccaagaagatgtttggtcttag

SEQ ID NO: 18 - protein, 713 aa, Gibberella fujikuroi
MAELDTLDIVVLGVIFLGTVAYFTKGKLWGVTKDPYANGFAAGGASKPGRTRNIVEAMEESGKNCVVFYGSQTGTAEDYASRLAKEGKSRFGLNTMIADLEDYDFDNLDTVPSDNIVMFVLATYGEGEPTDNAVDFYEFITGEDASFNEGNDPPLGNLNYVAFGLGNNTYEHYNSMVRNVNKALEKLGAHRIGEAGEGDDGAGTMEEDFLAWKDPMWEALAKKMGLEEREAVYEPIFAINERDDLTPEANEVYLGEPNKLHLEGTAKGPFNSHNPYIAPIAESYELFSAKDRNCLHMEIDISGSNLKYETGDHIAIWPTNPGEEVNKFLDILDLSGKQHSVVTVKALEPTAKVPFPNPTTYDAILRYHLEICAPVSRQFVSTLAAFAPNDDIKAEMNRLGSDKDYFHEKTGPHYYNIARFLASVSKGEKWTKIPFSAFIEGLTKLQPRYYSISSSSLVQPKKISITAVVESQQIPGRDDPFRGVATNYLFALKQKQNGDPNPAPFGQSYELTGPRNKYDGIHVPVHVRHSNFKLPSDPGKPIIMIGPGTGVAPFRGFVQERAKQARDGVEVGKTLLFFGCRKSTEDFMYQKEWQEYKEALGDKFEMITAFSREGSKKVYVQHRLKERSKEVSDLLSQKAYFYVCGDAAHMAREVNTVLAQIIAEGRGVSEAKGEEIVKNMRSANQYQVCSDFVTLHCKETTYANSELQEDVWS

SEQ ID NO: 19 - DNA, 2142 bp, Gibberella fujikuroi
atggcagaattagatacacttgatatagtagtattaggtgttatctttttgggtactgtggcatactttactaagggtaaattgtggggtgttaccaaggatccatacgctaacggattcgctgcaggtggtgcttccaagcctggcagaactagaaacatcgtcgaagctatggaggaatcaggtaaaaactgtgttgttttctacggcagtcaaacaggtacagcggaggattacgcatcaagacttgcaaaggaaggaaagtccagattcggtttgaacactatgatcgccgatctagaagattatgacttcgataacttagacactgttccatctgataacatcgttatgtttgtattggctacttacggtgaaggcgaaccaacagataacgccgtggatttctatgagttcattactggcgaagatgcctctttcaatgagggcaacgatcctccactaggtaacttgaattacgttgcgttcggtctgggcaacaatacctacgaacactacaactcaatggtcaggaacgttaacaaggctctagaaaagttaggagctcatagaattggagaagcaggtgagggtgacgacggagctggaactatggaagaggactttttagcttggaaagatccaatgtgggaagccttggctaaaaagatgggcttggaggaaagagaagctgtatatgaacctattttcgctatcaatgagagagatgatttgacccctgaagcgaatgaggtatacttgggagaacctaataagctacacttggaaggtacagcgaaaggtccattcaactcccacaacccatatatcgcaccaattgcagaatcatacgaacttttctcagctaaggatagaaattgtctgcatatggaaattgatatttctggtagtaatctaaagtatgaaacaggcgaccatatcgcgatctggcctaccaacccaggtgaagaggtcaacaaatttcttgacattctagatctgtctggtaagcaacattccgtcgtaacagtgaaagccttagaacctacagccaaagttccttttccaaatccaactacctacgatgctatattgagataccatctggaaatatgcgctccagtttctagacagtttgtctcaactttagcagcattcgcccctaatgatgatatcaaagctgagatgaaccgtttgggatcagacaaagattacttccacgaaaagacaggaccacattactacaatatcgctagatttttggcctcagtctctaaaggtgaaaaatggacaaagataccattttctgctttcatagaaggccttacaaaactacaaccaagatactattctatctcttcctctagtttagttcagcctaaaaagattagtattactgctgttgtcgaatctcagcaaattccaggtagagatgacccattcagaggtgtagcgactaactacttgttcgctttgaagcagaaacaaaacggtgatccaaatccagctccttttggccaatcatacgagttgacaggaccaaggaataagtatgatggtatacatgttccagtccatgtaagacattctaactttaagctaccatctgatccaggcaaacctattatcatgatcggtccaggtaccggtgttgccccttttagaggcttcgtccaagagagggcaaaacaagccagagatggtgtagaagttggtaaaacactgctgttctttggatgtagaaagagtacagaagatttcatgtatcaaaaagagtggcaagagtacaaggaagctcttggcgacaaattcgaaatgattacagctttttcaagagaaggatctaaaaaggtttatgttcaacacagactgaaggaaagatcaaaggaagtttctgatcttctatcccaaaaagcatacttctacgtttgcggagacgccgcacatatggcacgtgaagtgaacactgtgttagcacagatcatagcagaaggccgtggtgtatcagaagccaagggtgaggaaattgtcaaaaacatgagatcagcaaatcaataccaagtgtgttctgatttcgtaactttacactgtaaagagacaacatacgcgaattcagaattgcaagaggatgtctggagttaa

SEQ ID NO: 20 - protein, 691 aa, Saccharomyces cerevisiae
MPFGIDNTDFTVLAGLVLAVLLYVKRNSIKELLMSDDGDITAVSSGNRDIAQVVTENNKNYLVLYASQTGTAEDYAKKFSKELVAKFNLNVMCADVENYDFESLNDVPVIVSIFISTYGEGDFPDGAVNFEDFICNAEAGALSNLRYNMFGLGNSTYEFFNGAAKKAEKHLSAAGAIRLGKLGEADDGAGTTDEDYMAWKDSILEVLKDELHLDEQEAKFTSQFQYTVLNEITDSMSLGEPSAHYLPSHQLNRNADGIQLGPFDLSQPYIAPIVKSRELFSSNDRNCIHSEFDLSGSNIKYSTGDHLAVWPSNPLEKVEQFLSIFNLDPETIFDLKPLDPTVKVPFPTPTTIGAAIKHYLEITGPVSRQLFSSLIQFAPNADVKEKLTLLSKDKDQFAVEITSKYFNIADALKYLSDGAKWDTVPMQFLVESVPQMTPRYYSISSSSLSEKQTVHVTSIVENFPNPELPDAPPVVGVTTNLLRNIQLAQNNVNIAETNLPVHYDLNGPRKLFANYKLPVHVRRSNFRLPSNPSTPVIMIGPGTGVAPFRGFIRERVAFLESQKKGGNNVSLGKHILFYGSRNTDDFLYQDEWPEYAKKLDGSFEMVVAHSRLPNTKKVYVQDKLKDYEDQVFEMINNGAFIYVCGDAKGMAKGVSTALVGILSRGKSITTDEATELIKMLKTSGRYQEDVW

SEQ ID NO: 21 - DNA, 2076 bp, Saccharomyces cerevisiae
atgccgtttggaatagacaacaccgacttcactgtcctggcggggctagtgcttgccgtgctactgtacgtaaagagaaactccatcaaggaactgctgatgtccgatgacggagatatcacagctgtcagctcgggcaacagagacattgctcaggtggtgaccgaaaacaacaagaactacttggtgttgtatgcgtcgcagactgggactgccgaggattacgccaaaaagttttccaaggagctggtggccaagttcaacctaaacgtgatgtgcgcagatgttgagaactacgactttgagtcgctaaacgatgtgcccgtcatagtctcgatttttatctctacatatggtgaaggagacttccccgacggggcggtcaactttgaagactttatttgtaatgcggaagcgggtgcactatcgaacctgaggtataatatgtttggtctgggaaattctacttatgaattctttaatggtgccgccaagaaggccgagaagcatctctccgctgcgggcgctatcagactaggcaagctcggtgaagctgatgatggtgcaggaactacagacgaagattacatggcctggaaggactccatcctggaggttttgaaagacgaactgcatttggacgaacaggaagccaagttcacctctcaattccagtacactgtgttgaacgaaatcactgactccatgtcgcttggtgaaccctctgctcactatttgccctcgcatcagttgaaccgcaacgcagacggcatccaattgggtcccttcgatttgtctcaaccgtatattgcacccatcgtgaaatctcgcgaactgttctcttccaatgaccgtaattgcatccactctgaatttgacttgtccggctctaacatcaagtactccactggtgaccatcttgctgtttggccttccaacccattggaaaaggtcgaacagttcttatccatattcaacctggaccctgaaaccatttttgacttgaagcccctggatcccaccgtcaaagtgcccttcccaacgccaactactattggcgctgctattaaacactatttggaaattacaggacctgtctccagacaattgttttcatctttgattcagttcgcccccaacgctgacgtcaaggaaaaattgactctgctttcgaaagacaaggaccaattcgccgtcgagataacctccaaatatttcaacatcgcagatgctctgaaatatttgtctgatggcgccaaatgggacaccgtacccatgcaattcttggtcgaatcagttccccaaatgactcctcgttactactctatctcttcctcttctctgtctgaaaagcaaaccgtccatgtcacctccattgtggaaaactttcctaacccagaattgcctgatgctcctccagttgttggtgttacgactaacttgttaagaaacattcaattggctcaaaacaatgttaacattgccgaaactaacctacctgttcactacgatttaaatggcccacgtaaacttttcgccaattacaaattgcccgtccacgttcgtcgttctaacttcagattgccttccaacccttccaccccagttatcatgatcggtccaggtaccggtgttgccccattccgtgggtttatcagagagcgtgtcgcgttcctcgaatcacaaaagaagggcggtaacaacgtttcgctaggtaagcatatactgttttatggatcccgtaacactgatgatttcttgtaccaggacgaatggccagaatacgccaaaaaattggatggttcgttcgaaatggtcgtggcccattccaggttgccaaacaccaaaaaagtttatgttcaagataaattaaaggattacgaagaccaagtatttgaaatgattaacaacggtgcatttatctacgtctgtggtgatgcaaagggtatggccaagggtgtgtcaaccgcattggttggcatcttatcccgtggtaaatccattaccactgatgaagcaacagagctaatcaagatgctcaagacttcaggtagataccaagaagatgtctggtag

SEQ ID NO: 22 - protein, 503 aa, Homo sapiens
MALIPDLAMETWLLLAVSLVLLYLYGTHSHGLFKKLGIPGPTPLPFLGNILSYHKGFCMFDMECHKKYGKVWGFYDGQQPVLAITDPDMIKTVLVKECYSVFTNRRPFGPVGFMKSAISIAEDEEWKRLRSLLSPTFTSGKLKEMVPIIAQYGDVLVRNLRREAETGKPVTLKDVFGAYSMDVITSTSFGVNIDSLNNPQDPFVENTKKLLRFDFLDPFFLSITVFPFLIPILEVLNICVFPREVTNFLRKSVKRMKESRLEDTQKHRVDFLQLMIDSQNSKETESHKALSDLELVAQSIIFIFAGYETTSSVLSFIMYELATHPDVQQKLQEEIDAVLPNKAPPTYDTVLQMEYLDMVVNETLRLFPIAMRLERVCKKDVEINGMFIPKGVVVMIPSYALHRDPKYWTEPEKFLPERFSKKNKDNIDPYIYTPFGSGPRNCIGMRFALMNMKLALIRVLQNFSFKPCKETQIPLKLSLGGLLQPEKPVVLKVESRDGTVSGA

SEQ ID NO: 23 - DNA, 1533 bp, Homo sapiens
aagcttaaaatggcactgattcccgatttagcaatggagacttggttgttgcttgccgtaagtctcgtcttactgtatttgtacggaacgcactcgcacggattatttaagaaattgggcattcccgggcccactccactaccattcctaggtaatatacttagttatcacaagggtttctgcatgttcgacatggaatgtcacaagaagtatggtaaggtatggggattctacgacggccaacaacctgtgttggcgatcaccgacccagacatgatcaaaactgtcctcgtaaaagaatgttactctgttttcactaatagaagaccatttggacctgtaggattcatgaagagtgctatatccattgcagaggacgaagaatggaagaggcttagaagccttctgtcacctacattcacaagcggcaagttgaaggagatggtccctatcatcgcccagtatggcgatgtcttagtgagaaatttacgtagggaagctgaaactggtaagcctgtgacgctgaaggatgtctttggagcttatagcatggacgtgatcacttcgacttcctttggcgtaaatatcgattcgcttaacaacccacaggatccctttgttgagaacacgaagaaactgttgagatttgactttctcgatccgttcttcctttccattaccgtcttccctttcctcatacccattctggaagtcctgaatatatgcgtattcccaagagaggtgacgaacttcttaaggaaatcggtaaagaggatgaaggaatcccgtcttgaggacacccagaagcacagggtcgactttctacagttaatgatagattcacagaattcgaaagagacggagagccataaggctttaagtgatcttgagcttgtagcacagagtatcatcttcattttcgccggctacgagacgacgagcagtgtgttgtcgttcatcatgtacgagttggcgacacatcccgacgtgcagcagaagttacaggaagaaatcgatgctgttttaccaaataaagccccacccacttatgatacagttttgcagatggagtacttagacatggtggttaacgaaacactaagactgtttccgattgctatgcgattggaacgagtgtgtaagaaggacgtagaaattaacggcatgtttataccaaagggcgtagttgtcatgataccttcttatgctttgcatcgagaccctaagtactggaccgaacctgaaaagtttctcccagagcgctttagcaagaagaataaggataacatagacccctacatttatacgccattcggatccggtccacgtaactgtataggcatgcgtttcgctctgatgaacatgaagctggcgttaatcagggtattacagaacttttcattcaaaccatgcaaagagacacagataccgttgaagctctctttaggtggacttctgcagcccgagaagccagtggttctcaaagttgagagcagggacggtacagtttcaggcgcttagaagactccgcgg

SEQ ID NO: 24 - protein, 503 aa, Pongo abelii
MDLIPDLAMETWILLAVSLVLLYLYGTHSHGLFKKLGIPGPTPLPLLGNVFSYRKGFWRFDMECHKKYGKVWGFYDGRQPVLAITDPDMIKTVLVKECYSVFTNRRPFGPVGFMKSAISIAEDEEWKRIRSLLSPTFTSGKLKEMVPIIARYGDVLVRNLRREAETGKPVTLKDVFGAYSMDVITSTSFGVNIDSLNNPQDPFVENTKKLLRFDFLDPFFLSIIVFPFLTPILEILNISVFPREVTSFLRKSVKRMKESRLKDTQKHRVDFLQLMIDSQNSKETESHKALSDLELVAQSIIFIFAGYETTSSVLSFIMYELATHPDVQRKLQEEIDAVLPNKAPPTYDTVLQMEYLDMVVNETLRLFPIAMRLERVCKKDVEINGMFIPKGVVVMIPSYALHHDPKYWTEPGKFLPERFSKKNKDNIEPYVYTPFGTGPRNCIGMRFALMNMKLAVIRVLQNFSFKPCKETQIPLKLRLGGLLQTEKPIVLKVESRDGTLSGA

SEQ ID NO: 25 - DNA, 1533 bp, Pongo abelii
aagcttaaaatggaccttatccctgacctcgctatggagacttggatcttacttgcggtttctctagtgctgttatacttgtatggaacacactcccatggattgtttaagaaattaggtatcccaggaccaacaccgttgcctttgctaggaaacgtcttcagttatcgaaagggcttctggagatttgatatggaatgtcacaagaagtacggcaaggtgtggggcttctacgatggcaggcagcctgtcctcgcaataacagatccggatatgataaagacggttttagtaaaagaatgctactctgtatttactaacaggcgccctttcgggccagtggggttcatgaagagcgccatctctatcgccgaagatgaggagtggaagcgtatccgatccttattatctcctacgtttacaagcgggaagttaaaagagatggtgccaataatagccaggtatggagacgttctggttaggaatttgagaagagaggctgagacggggaagcctgttaccttaaaggacgtcttcggcgcctacagcatggacgtaataaccagtacttcatttggcgtcaacatcgacagtctaaacaaccctcaggatccatttgtcgagaataccaagaaactcttaaggttcgactttctagacccattcttcctgagcattattgtgttccctttccttacccctattctcgagatactaaatatctctgttttcccaagagaggtaacgtcgttcttacgcaaatctgtaaagagaatgaaagagagtagattgaaggatacacaaaagcacagagtagacttccttcagctaatgattgattctcagaattcaaaggagaccgagagccacaaggccctttctgacctggaattagtagcacagtcaattatcttcattttcgccggatacgaaacaactagttctgtgttatcatttattatgtacgagttagcaactcacccggacgtacagaggaaattacaggaagagatagatgcagttcttccaaacaaggccccaccaacttatgacaccgtcctacaaatggagtatttggatatggttgtgaacgagacactgagattgtttcctatagcaatgagacttgagcgtgtgtgtaagaaagatgtcgagataaatggaatgttcatccctaagggcgtagtcgtgatgattccgtcctacgcactccaccacgaccctaagtattggacggagccgggtaagttcttacctgagaggttcagtaagaagaacaaagacaacatagaaccttatgtatacacgccctttggaaccgggccacgtaactgcattgggatgcgtttcgcactcatgaacatgaaacttgcggtcatacgagtgcttcaaaacttttcctttaagccatgcaaggagacacaaataccgctaaagttgagattgggtggattgttgcagacagagaagccgattgtccttaaggtcgaatcgcgcgacggcacattatctggcgcctagaagactccgcgg

SEQ ID NO: 26 - protein, 503 aa, Papio anubis
MDLIPDLAVETWLLLAVTLVLLYLYGTHSHGLFKKLGIPGPTPLPLLGNVLSYRKGFWTFDMECYKKYGKVWGFYDGRQPVLAITDPNMIKTVLVKECYSVFTNRRPFGPVGFMKSAISIAEDEEWKRIRSLLSPTFTSGKLKEMVPIIAKYGDVLVRNLRRETETGKPVTLKDVFGAYSMDVITSTSFGVNIDSLNNPQDPFVENTKKLLRFDFLDPFFLSITIFPFLIPILEVLNISIFPREVTSFLRKSVKRIKESRLKDTQKHRVDFLQLMIDSQNSKETESHKALSDLELVAQSIIFIFAGYETTSSVLSFIMYELATHPDVQQKLQEEIDAVLPNKAPPTYDTVLQMEYLDMVVNETLRLFPIAMRLERVCKKDVEINGIFIPKGVVVMIPTYALHHDSKYWTEPEKFLPERFSKKNKDNIDPYIYTPFGSGPRNCIGMRFALMNMKLALIRVLQNFSFKPCKETQIPLKLRLGGLLQTEKPIVLKIESRDGTVSGA

SEQ ID NO: 27 - DNA, 1533 bp, Papio anubis
aagcttaaaatggatcttattcctgacctcgctgttgagacatggctgcttttggcagttacactagtactactttacctgtacggaacccactcccacggcctatttaagaagttgggaatcccaggacctactccgctacctctactagggaatgtattatcataccgtaaaggtttctggactttcgacatggagtgttataagaagtacggaaaggtctggggcttttatgatggacgccaaccggtcctagccattacagatccaaacatgataaagaccgttttggtaaaagagtgctactctgttttcacgaatagaagaccctttggaccagttggcttcatgaagagtgcgatctctatcgccgaggatgaggagtggaagagaatcagatccctgttatcgccaaccttcacttcaggcaagctcaaagagatggtgccaataattgcgaaatacggtgacgtacttgtccgtaatctgcgtagagagacagagaccggaaagccagttacattaaaggacgtctttggtgcatactctatggacgtgatcacaagtacttctttcggtgtgaatattgattctttgaataacccacaggatccttttgtggagaacactaagaaattgctgaggtttgacttcttggatcccttcttcctgagcataaccatctttccttttctaattccaatcttggaagttttaaatatcagtatctttcccagggaagtcacttctttcctacgaaagtcggtgaagcgtataaaagagagcagattgaaggatacgcaaaagcatcgcgtcgactttctccaactcatgatagacagccagaattcgaaagaaacagaatcacacaaggcgctctctgacttggagttggtggcccaatcgataatattcatattcgcaggatatgagacaacatcgtccgtgttgagctttattatgtacgagttggccacccaccccgacgtacagcagaagttgcaggaagagatcgacgccgttttgccgaacaaagctccgcccacttatgataccgtgctacagatggaatacctagacatggtagttaatgagacgttgaggttattcccaatagcaatgaggttggaaagagtttgtaagaaggatgtagagataaatggtatctttattccaaaaggggtcgtagtgatgatccccacatacgccttacaccacgattctaaatattggacagagccggagaaattcttgccggaacgcttctcaaagaagaacaaagataacatcgacccgtacatctacactccatttggatcgggcccgaggaactgtattggtatgaggttcgcgcttatgaacatgaagctagccttgattagggtattacagaacttcagctttaagccatgtaaagagacccagataccgctgaaactgaggttgggtgggctgttgcagaccgagaagcccatagttttgaagattgaatcgagggacgggaccgtatcaggtgcgtagaagactccgcgg

SEQ ID NO: 28 - protein, 504 aa, Gorilla gorilla gorilla
MALIPDLAMETWLLLAVSLVLLYLYGTHSHGLFKKLGIPGPTPLPFLGNIWSYRKGFCMFDMECHKKYGKVWGFYDGRQPVLAITDPDMIKTVLVKECYSVFTNRRPFGPVGFMKSAISIAEDEEWKRLRSLLSPTFTSGKLKEMVPLIAQYGDVLVRNLSREAETGKPVTMKDLFNTFSTTMEISTTDAGQNIDSLNNPQDPFVENTKKLLRFDFLDPFFLSIIVFPFLTPILEVLNISVFPRAVTSFLRKSVKRMKESRLEDTQKHRVDFLQLMIDSQNSKETESHKALSDLELVAQSIIFIFAGYETTSSVLSFITYELATHPDVQQKLQEEIDAVLPNKAPPTYDTVLQMEYLDMVVNETLRLFPIAMRLERVCKKDVEINGMFIPKGVVVMIPSYALHHDPKYWTEPEKFLPERFSKKNKDNIDPYIYTPFGSGPRNCIGMRFALMNMKLALIRVLQNFSFKPCKETQIPLKLRLGGLLQPEKPIVLKVESRDGTVSGA

SEQ ID NO: 29 - DNA, 1536 bp, Gorilla gorilla gorilla
aagcttaaaatggctttaattcccgacttggccatggagacctggttgttgttagctgttagcctagtcttgttgtacttgtacgggacccattctcacggcttatttaagaaactcggtataccagggcctactccattaccattcttagggaacatttggtcatatagaaagggattttgcatgttcgacatggagtgtcacaagaaatacgggaaggtatggggattctatgacggtcgtcaacccgtgttggccataaccgaccctgatatgattaagactgtcttagtcaaggagtgttattctgttttcacgaacaggcgtcctttcggtccagtcggcttcatgaaatcagcaatatccattgcagaggacgaggagtggaaacgattacgttctttgttgtctcctacttttacatcagggaaacttaaagagatggtcccgttaatcgctcagtacggcgacgtgttagttaggaacctgtccagagaggcagaaactggaaaacctgtcaccatgaaagacttattcaacaccttctcgaccacgatggagattagtaccactgatgcaggccagaacatcgattccctcaacaatccgcaagaccctttcgtagagaacaccaagaagttacttagatttgatttcctagacccgttctttctttcgataatcgtgttcccttttctaacaccaatcctagaggtattgaatatatcggtcttcccccgcgctgtaacatctttccttagaaaatcagtaaagcgtatgaaagaatctagattggaagatacacaaaagcaccgtgtcgacttcttacaattaatgatcgacagtcaaaactcgaaagagacggaatcacacaaagcactttcggacctggagttagttgcgcaaagcataattttcatctttgcggggtacgagactacatcctcagttttgtcattcataacctacgagctggccactcatccggatgtgcagcaaaagctgcaggaagaaattgacgcagtcttacccaacaaggctcccccaacctacgacactgttcttcagatggagtacctcgacatggtagtgaatgagacattgagattgtttcccatcgccatgaggttagaaagggtatgcaagaaggacgtcgagataaacggcatgttcatccctaagggcgtggttgtaatgatcccctcttacgcgctccaccatgatccaaaatactggacagagcccgaaaagttccttccggagagattcagcaagaagaacaaggacaacatagacccttacatatataccccattcggtagtggaccacgtaactgcatcggcatgaggtttgctttaatgaacatgaaacttgcattgatcagagttctgcaaaacttttccttcaagccctgtaaagagacgcagattccgttaaagctaaggttaggtggcctactgcaaccagagaagccgattgtactcaaagtcgagagtagggatggtactgtctctggcgcttagaagactccgcgg

SEQ ID NO: 30 - protein, 503 aa, Canis lupus familiaris
MDLIPSFSMETWLLLATSLVLLYLYGTYTHGVFKKLGIPGPTPLPFVGTALGYRKGFSVFDENCFRKYGRMWGFYDGRQPVLAITDPDMIKTVLVKECYSVFTNRRSFGPVGFMKSAISLSEDEEWKRIRTLLSPTFTSGKLKEMFPIIGQYGDVLVRNLRKEAEKGKSINLKDIFGAYSMDVITSTSFGVNIDSLNNPQDPFVENIKKLLKFDFLDPFFFSILLFPFLTPVFEVLNIWLFPKSVTDFFTKSVKRMKENRLKDKQKHRVDFLQLMINSQNSKETDTHKALSDLELVAQSIIFIFAGYETTSTSLSFLMYELATHPDVQQKLQEEIDATFPNKALPTYDALVQMEYLDMVLNETLRLYPIAGRLERVCKKDVEISGVFIPKGTVVMVPTFTLHRDQSLWPEPEEFRPERFSRKNKDSINPYTYLPFGTGPRNCIGMRFAIMNMKLALVRVLQNFSFKPCKETQIPLKLNAQGIIQPEKPIVLKVEPRDGSVNGA

SEQ ID NO: 31 - DNA, 1533 bp, Canis lupus familiaris
aagcttaaaatggacttgatccctagcttcagtatggaaacatggctactgctcgcgacatcccttgtattgctttatctctacggcacatacactcatggcgtgtttaagaagttgggtatcccaggacctacacctcttcctttcgtcggcactgcgttaggatataggaagggcttctcagtctttgacgagaattgcttccgtaagtacggaagaatgtggggtttctatgacggaaggcagcctgtgttggcgatcacggatccagacatgattaagaccgtattagtcaaagagtgctatagcgtattcacgaacagacgttcctttgggcccgtcggtttcatgaagtcagccatctcgttgagcgaagacgaggagtggaaaagaattaggacacttctgtctccaacatttacttcaggcaaactcaaggaaatgtttcctatcataggacagtacggggacgtccttgttcgtaacctcaggaaggaagccgagaaagggaagtccataaacttaaaggacatcttcggagcttattctatggacgtcatcacttccacgtccttcggcgttaatattgatagtttaaacaacccccaagacccgttcgtggagaacatcaagaaattattgaagttcgatttcctggaccctttcttcttctcaattctactgttccccttcttaacacctgttttcgaggttttgaatatatggttgtttccgaagagcgttacggatttctttacaaagtcggtaaagcgtatgaaagagaaccgcctaaaagacaagcagaaacatagagtagacttcttgcagcttatgataaactcacaaaattctaaagagactgacacccacaaagccctgtccgacttggagttggttgctcagtcgataatcttcatattcgccggctatgagacgaccagtacttcgctgtccttcttaatgtatgaattagcgacccaccccgatgtccagcagaagttacaagaggaaattgacgccacgttcccaaataaagcgttacccacttacgatgctctggtgcagatggagtacttggatatggttttaaacgaaactctccgtttatacccaatcgccgggagattggagagagtatgcaagaaagacgttgagattagtggagtattcatccccaagggaactgtcgtgatggttccaactttcaccctacatcgtgatcagagcttgtggccggagcctgaggaatttagacccgagaggttctcaagaaagaataaggattccatcaacccatatacttaccttccgttcggtactggacctagaaactgtattggaatgcgcttcgccataatgaacatgaagctagctctagttcgcgtattgcagaacttctcatttaagccgtgtaaagagacacaaatcccattaaagctgaatgctcagggtatcatacagccagagaagccaattgttttaaaggttgagcctagggacggtagtgtgaacggggcttagaagactccgcgg

SEQ ID NO: 32 - protein, 490 aa, Homo sapiens
MEPFVVLVLCLSFMLLFSLWRQSCRRRKLPPGPTPLPIIGNMLQIDVKDICKSFTNFSKVYGPVFTVYFGMNPIVVFHGYEAVKEALIDNGEEFSGRGNSPISQRITKGLGIISSNGKRWKEIRRFSLTTLRNFGMGKRSIEDRVQEEAHCLVEELRKTKASPCDPTFILGCAPCNVICSVVFQKRFDYKDQNFLTLMKRFNENFRILNSPWIQVCNNFPLLIDCFPGTHNKVLKNVALTRSYIREKVKEHQASLDVNNPRDFIDCFLIKMEQEKDNQKSEFNIENLVGTVADLFVAGTETTSTTLRYGLLLLLKHPEVTAKVQEEIDHVIGRHRSPCMQDRSHMPYTDAVVHEIQRYSDLVPTGVPHAVTTDTKFRNYLIPKGTTIMALLTSVLHDDKEFPNPNIFDPGHFLDKNGNFKKSDYFMPFSAGKRICAGEGLARMELFLFLTTILQNFNLKSVDDLKNLNTTAVTKGIVSLPPSYQICFIPV

SEQ ID NO: 33 - DNA, 1494 bp, Homo sapiens
aagcttaaaatggagccctttgtcgtgttggtactttgcttgagcttcatgttgttgttttccttatggagacagtcgtgtcgtaggagaaaactaccaccgggtcctactccactcccaataattggtaacatgctgcagatcgatgttaaagacatctgtaaatcattcacaaacttctcgaaggtatatggtcccgtctttactgtctacttcggtatgaacccgatcgtggtcttccacggttacgaggccgtgaaggaagcattgatagataatggggaagaattctcagggcgcggcaacagtcccattagtcagaggatcaccaaggggttgggaataatctcttcgaatggtaagagatggaaggagatccgaagattcagccttaccactctcagaaatttcggcatgggaaaacgcagtatagaggaccgtgtccaagaggaagctcactgcttagtagaggagttgaggaagacgaaagcatctccatgtgatcctaccttcatcttaggttgcgctccatgcaatgttatatgctcagtggtattccaaaagagattcgactataaagaccagaacttcctaactttgatgaagcgctttaatgagaatttccgtatccttaactcaccgtggatccaggtctgcaacaactttccacttctgattgattgtttcccgggcactcacaacaaagtgcttaagaacgttgctctcactcgtagttacatccgtgaaaaggttaaagagcaccaagctagtctggacgttaacaacccacgtgacttcatagactgcttcctaatcaagatggaacaagaaaaggataaccagaaatctgagtttaacatagaaaacctggtaggtacggtggctgatctgttcgtcgctggcactgagacaactagcactaccttgaggtacgggctacttctgttgttgaagcacccagaggtaactgctaaagtacaagaggaaattgatcatgtaatcggtcgtcaccgtagtccgtgcatgcaggatagatcccacatgccctacacagacgcagtggtccacgaaatccagagatactctgacctagtgccaactggcgtcccacacgcagtcacaaccgacacgaagtttagaaattaccttattccgaaaggtacgactatcatggctttgctaacatcagtgctacatgatgacaaggagttccccaaccctaatatctttgatcctggccattttcttgataagaacggcaacttcaagaaatcggactactttatgccgttttcggctgggaagaggatctgcgctggagaaggattagctagaatggagttgttcttatttctgacgactattctacagaacttcaatttaaagtcggttgacgatttgaagaacctgaacacaactgcagttacaaagggcatagttagtctaccgccatcttatcaaatatgctttatcccggtatagaagactccgcgg

SEQ ID NO: 34 - protein, 490 aa, Pan troglodytes
MEPFVVLVLCLSFMLLFSLWRQSSGRRKLPPGPTPLPIIGNMLQIDVKDICKSFSNFSKVYGPVFTVYFGMNPIVVLHGYEAVKEALIDNGEEFSGRGSSPISQRITKGLGIISSNGKRWKEIRRFSLTTLRNFGMGKRSIEDRVQEEAHCLVEELRKTKASPCDPTFILGCAPCNVICSVVFQKRFDYKDQNFLTLMKRFNENFRILNSPWIQVCNNFPLLIDCFPGTHNKVLTNVALTQSYIREKVKEHQASLDVNNPRDFIDCFLIKMEQEKDNQKSEFNIENLVGTVADLFVAGTETTSTTLRYGLLLLLMHPEVTAKVQEEIDHVIGRHRTPCMQDRSHMPYTDAVVHEIQRYSDLVPTGVPHAVTTDTKFRNYLIPKGTTIMTLLTSVLHDDKEFPNPNIFDPGHFLDKNGNFKKSDYFMPFSAGKRICAGEGLARMELFLFLTTILQNFNLKSVDDLKNLNTTAVTKGIVSLPPSYQICFIPV

SEQ ID NO: 35 - DNA, 1494 bp, Pan troglodytes
aagcttaaaatggagcccttcgtcgtattagttctctgcctttcttttatgttgctattctcattgtggcgccagagttccggacgacgtaaattaccacctggaccaacaccactcccaataataggtaacatgctacagatagacgtaaaagacatatgcaagtccttctcaaacttttctaaggtatatggacctgtattcacggtatattttgggatgaatcccatcgtggttctgcacggatacgaagccgttaaagaggctcttattgataatggcgaggaatttagtggcaggggctcgtcgccgatatctcagaggataactaaaggactaggaattattagctccaatggaaagcgctggaaggagatcagaaggttcagcctgacgacactacgtaacttcggaatgggtaagcgatcaatagaggatagggttcaggaagaggcacactgcctggtagaagaattacgcaagactaaagcatccccatgtgatccgacattcatcctcggctgcgcaccatgcaacgtaatctgctcggtcgttttccagaagcgatttgattacaaggaccagaactttcttacgttgatgaagcgctttaatgagaatttcaggattttgaatagcccttggatccaggtctgcaataacttcccgcttctaatagactgcttccctggtacccataataaggtgttaaccaacgtcgcactgacccaatcctacattcgagagaaagtcaaagagcatcaagcatcacttgacgtcaataaccctagagacttcattgactgcttcttgatcaaaatggagcaggagaaggacaatcagaagtcagaattcaacatcgaaaacttagtcggtactgtggctgatctgtttgtcgcagggacggaaactacttccacgaccttaagatacggattattgctgttgcttatgcaccccgaggttacagcgaaagtccaagaggagatcgaccatgtaattggccgtcaccgtacgccctgtatgcaagaccgttcgcacatgccctacacagatgcggttgtacacgagatccagcgatactcagacctggtgccaactggggtgccccacgctgtaactactgacacgaagtttcgtaattacttaattccaaaaggcacgaccattatgacgctattaacgtctgtcctgcacgacgacaaggagttccctaaccctaacatattcgacccaggccattttctagataagaacgggaacttcaagaaatcggattactttatgcctttctcagctgggaagaggatctgcgcaggtgagggcttggccaggatggagttattcttgttcttgactactatattacagaacttcaacttgaagtcagttgatgacttgaagaaccttaacactacagcagtcactaagggtatagtctcattaccccctagttatcaaatctgcttcattcctgtttagaagactccgcgg

SEQ ID NO: 36 - protein, 490 aa, Pongo abelii
MEPFVVLVLCLSFMLLFSLWRQSSGRRKLPPGPTPLPIIGNMLQIDIKDICKSFSNFSKVYGPVFTVYFGMNPMVVLHGYEAVKEALIDNGEEFSGRGSSPISQRITKGLGIISSNGNRWKEIRRFSLTTLRNFGMGKRSIEDRVQEEARCLVEELRKTKASPCDPTFILGCAPCNVICSVVFQKRFDYKDQNFLTLMKRFNENFRILNSPWIQVCNNFPLLIDCFPGTHNKLLKNVALTRSYIREKVKEHQTSLDVTSPRDFIDCFLIKMEQEKDNQKSEFNIENLVGTVADLFVAGTETTSTTLRYGLLLLLKHPEVTAKVQEEIDHVIGRHRSPCMQDRSHMPYTDAVVHEIQRYIDLVPTGVPHAVTTDIQFRNYLIPKGTTIMTLLTSVLHDDKEFPNPKIFDPGHFLDKNGNFKKSDYFMPFSAGKRICAGEGLARMELFLFLTTILQNFNLKSVDDLKNLNTTAVTKGIVSLPPSYQICFIPV

SEQ ID NO: 37 - DNA, 1494 bp, Pongo abelii
aagcttaaaatggagccatttgtggtacttgtactgtgtcttagcttcatgcttctgttctccctatggagacagtcatctggacgacgtaagttgccgccagggccaacccctttacccatcattgggaacatgcttcaaatagatattaaggacatatgcaagagcttttcgaacttctcaaaggtttatgggcctgtgtttaccgtatatttcggaatgaacccaatggtcgtgttgcatggttacgaggctgttaaggaagcactgatagacaacggcgaggagttctcaggccgtgggtcatctcctatctcacaaaggattaccaagggattgggaataatatcgtcaaacggtaaccgctggaaggagatcagaagattcagcctcactaccttgcgtaactttggtatggggaaaagaagtatcgaggaccgtgtacaggaagaggcaaggtgtcttgtcgaggagctacgtaagaccaaggcgtccccgtgcgacccaacctttatcttgggctgcgctccgtgtaacgtaatctgctcagtcgtgttccagaagaggtttgattacaaggaccagaacttcttgactttaatgaagcgttttaatgagaactttaggattctaaactccccgtggattcaggtttgtaacaatttcccgttacttatagactgttttccaggtactcacaataagctactcaagaatgtggcactaacccgtagctatattcgcgagaaagtcaaagagcaccagacgtccctagatgtgacttcacccagggacttcatagactgcttcttaataaagatggagcaggagaaggataaccagaagagtgaattcaatattgagaatttagtcggtacggttgccgatctattcgttgccggaacggagactacatcgactacactgcgttatggtttgttattgttgttaaagcaccctgaggtcacagctaaagtgcaggaagagattgatcacgtcatcggtagacacagaagtccatgcatgcaagacagaagccacatgccatatactgacgcagttgtccacgagatacagcgttacatcgatttggtcccaacaggggtgccacacgctgttaccacggatattcagtttagaaactatcttataccaaaaggaacgacaatcatgacccttctgacctctgttctacatgacgacaaagagttcccaaatcctaagatcttcgacccaggtcacttcttggacaagaatggaaacttcaagaagtccgattacttcatgcctttcagtgccggtaagagaatctgtgctggtgaaggactagcgaggatggagcttttcttattcctaacaaccatattgcagaactttaatcttaaatcagttgacgacctaaagaacctaaatacaactgccgtgacgaaaggcatagttagtctcccaccgtcctaccagatatgtttcattccagtatagaagactccgcgg

SEQ ID NO: 38 - protein, 490 aa, Chlorocebus aethiops
MEPFVVLVLCLSFVLLFSLWRQSSGRRNLPPGPTPFPIIGNMLQIDVKDICKSFSNFSKVYGPVFTVYLGMNPVVVLHGYEAVKEALIDNAEEFSGRGILPISERITKGLGIISSNGKRWKETRRFSLTTLRNFGMGKRSIEDRVQEEARCLVEELRKTKASPCDPTFILGCAPCNVICSVVFQKRFDYKDENFLTLMKRFTENFRILTSPWIQVCNNFPLLIDCFPGTHNKLLKNVALTKSYIREKVKEHQATLDINNPRDFIDCFLIKMEKEKDNQQSEFTIENLVGTVADLFVAGTETTSTTLRYGLLLLLKHPEVTAKVQEEIDHVIGRHRSPCMQDRSHMPYTDAVVHEIQRYIDLVPTGVPHAVTTDIKFRNYLIPKGTIIMTLLTSVLHDDKEFPNPKIFDPGHFLDENGNFKKSDYFMPFSAGKRICAGEGLARMELFLFLTTILQNFNLKSVADLKNLNTTSATRGIISLPPSYQICFIPV

SEQ ID NO: 39 - DNA, 1494 bp, Chlorocebus aethiops
aagcttaaaatggagccattcgttgttttagtcctgtgcttatcttttgttttactgttctctttatggcgacagtcgagcggtcgacgaaacctaccaccaggccccactccgttcccgatcataggtaatatgcttcaaatcgacgtaaaggatatctgcaagtccttctccaatttcagtaaagtctacggcccggtgtttacagtatatttgggtatgaacccggtagtcgtactacacggatacgaggcggttaaagaagcattaatcgataacgcagaggaattctcagggcgcgggatattacccatatctgagcgcatcacaaaggggcttggcattatttccagcaatggtaaaagatggaaggagacacgaagattttcactaacaactttgcgtaacttcggaatgggaaaacgttcgatcgaggaccgcgtacaagaggaagcacgatgtcttgtggaagagttgagaaagaccaaggcttcgccatgtgatcctacattcattcttggatgtgcaccctgcaacgtaatctgcagtgtggtattccagaagcgatttgactataaggacgagaacttcttaactttaatgaaaagattcacggagaactttaggatcttgacttcaccttggatccaggtatgcaataactttcctcttctaatcgactgcttcccaggaacacataacaagttgttgaagaacgtagcactaactaagtcatacatacgtgagaaggtgaaagaacaccaagcaacacttgatattaataatcctcgtgactttattgactgctttctaatcaagatggagaaagagaaggacaaccagcagtctgagttcactatagagaacctagttgggactgtagctgacttgtttgtcgccggtaccgagacaacatcaacaaccttgaggtatggtctattattgttactgaagcatcccgaagtgacggcaaaggtccaggaagagatagaccacgtaatcggccgacaccgttcaccgtgcatgcaggatagatcacatatgccatataccgatgcggtcgtacatgagatccaaaggtacattgacttggttcctacaggcgttccccacgccgtaacaactgacattaaattccgcaactatctaatacccaagggcactatcatcatgacgctactgacgtccgtcctgcatgatgacaaggagtttccaaaccctaagatcttcgacccgggacacttcctagacgagaatggtaacttcaagaaatcagattacttcatgcccttctcagctggtaaacgaatctgcgccggagaaggcctcgctcgtatggagcttttcttgttcttaacgaccatattgcagaacttcaacctaaagtcagttgcagaccttaagaatttaaatacaaccagcgccactcgtggcatcatctctttgccgccgtcatatcagatatgctttattcctgtatagaagactccgcgg

SEQ ID NO: 40 - protein, 502 aa, Homo sapiens
MDLIPNLAVETWLLLAVSLVLLYLYGTRTHGLFKRLGIPGPTPLPLLGNVLSYRQGLWKFDTECYKKYGKMWGTYEGQLPVLAITDPDVIRTVLVKECYSVFTNRRSLGPVGFMKSAISLAEDEEWKRIRSLLSPTFTSGKLKEMFPIIAQYGDVLVRNLRREAEKGKPVTLKDIFGAYSMDVITGTSFGVNIDSLNNPQDPFVESTKKFLKFGFLDPLFLSIILFPFLTPVFEALNVSLFPKDTINFLSKSVNRMKKSRLNDKQKHRLDFLQLMIDSQNSKETESHKALSDLELAAQSIIFIFAGYETTSSVLSFTLYELATHPDVQQKLQKEIDAVLPNKAPPTYDAVVQMEYLDMVVNETLRLFPVAIRLERTCKKDVEINGVFIPKGSMVVIPTYALHHDPKYWTEPEEFRPERFSKKKDSIDPYIYTPFGTGPRNCIGMRFALMNMKLALIRVLQNFSFKPCKETQIPLKLDTQGLLQPEKPIVLKVDSRDGTLSGE

SEQ ID NO: 41 - DNA, 1530 bp, Homo sapiens
aagcttaaaatggacttgatcccaaacttggctgttgaaacttggttgttattggccgtttctttggtcttgttgtacttgtatggtactagaacccatggtttgttcaagagattgggtattccaggtccaactccattgccattattgggtaatgttttgtcctacagacaaggcttgtggaagtttgatactgagtgctataagaaatacggtaagatgtggggtacttacgaaggtcaattgccagttttggctattactgatccagatgttatcagaaccgtcttggtcaaagaatgctactctgttttcaccaacagaagatctttgggtccagttggttttatgaagtccgctatttctttggccgaagatgaagaatggaagagaatcagatctttgttgtctccaactttcacctccggtaagttgaaagaaatgttcccaattattgcccaatacggtgatgttttggtcagaaacttgagaagagaagctgaaaaaggtaagccagttaccttgaaggatattttcggtgcttactccatggatgttattaccggtacttctttcggtgtcaacatcgattctttgaacaatccacaagatcccttcgttgaatctaccaagaagtttttgaagttcggtttcttggaccccttgttcttgtccattattttgttcccatttctgaccccagttttcgaagccttgaatgtttctttgtttccaaaggacaccatcaatttcttgagcaagtccgttaacaggatgaagaagtctagattgaacgacaagcaaaagcacaggttggatttcttgcaactgatgatcgattcccagaactctaaagaaactgaatcccataaggctttgtccgatttggaattggctgcccaatctatcattttcattttcgctggttacgaaaccacctcctctgttttgtcttttaccttgtatgaattggccactcatccagacgttcaacaaaagttgcaaaaagaaatcgatgccgtcttgccaaacaaagctccaccaacttatgatgctgttgtccaaatggaatacttggatatggttgtcaacgaaaccttgaggttgtttccagttgctatcagattggaaagaacctgcaaaaaggatgtcgaaatcaacggtgttttcatcccaaaaggttccatggttgtgattccaacttacgcattgcatcatgatccaaagtattggactgaaccagaagaattcagaccagaaagattctccaagaagaaggattccattgatccttacatctacactccatttggtactggtcctagaaactgtattggtatgagattcgctctgatgaacatgaagttggccttgattagagtgttgcagaacttctctttcaaaccctgtaaagaaacgcagatcccattgaagttggatacacaaggtttattgcaaccagaaaagcctatcgttttgaaggtcgattctagagatggtactttgtctggtgagtgaaagactccgcgg

SEQ ID NO: 42 - protein, 502 aa, Pan troglodytes
MDLIPNLAVETWLLLAVSLVLLYLYGTRTHGLFKRLGIPGPTPLPLLGNVLSYRQGLWKFDTECYKKYGKMWGMYDGQLPVLAITDPDMIRTVLVKECYSVFTNRRSLGPVGFMKSAISLAEDEEWKRIRSLLSPTFTSGKLKEMFPIIAQYGDVLVRNLRREAEKGKPVTLKDIFGAYSMDVITGTSFGVNIDSLNNPQDPFVESTKKFLKFGFLDPLFLSIILFPFLTPVFEALNVSLFPKDTINFLSKSVNRMKKSRLNDKQKHRLDFLQLMIDSQNSKETESHKALSDLELAAQSIIFIFAGYETTSSVLSFTLYELATHPDVQQKLQKEIDAVLPNKAPPTYDAVVQMEYLDMVVNETLRLFPVAIRLERTCKKDVEINGVFIPKGSMVVIPTYALHHDPKYWTEPEEFRPERFSKKKDSIDPYIYTPFGTGPRNCIGMRFALMNMKLALIRVLQNFSFKPCKETQIPLKLDTQGLLQPEKPIVLKVDSRDGTLSGE

SEQ ID NO: 43 - DNA, 1530 bp, Pan troglodytes
aagcttaaaatggacttgatcccaaacttggctgttgaaacttggttgttattggccgtttctttggtcttgttgtacttgtatggtactagaacccatggtttgttcaagagattgggtattccaggtccaactccattgccattattgggtaatgttttgtcctacagacaaggcttgtggaagtttgatactgagtgctataagaaatacggtaagatgtggggtatgtacgatggtcaattgccagttttggctattactgatccagatatgatcagaaccgtcttggtcaaagaatgctactctgttttcaccaacagaagatctttgggtccagttggttttatgaagtccgctatttctttggccgaagatgaagaatggaagagaatcagatctttgttgtctccaactttcacctccggtaagttgaaagaaatgttcccaattattgcccaatacggtgatgttttggtcagaaacttgagaagagaagctgaaaaaggtaagccagttaccttgaaggatattttcggtgcttactccatggatgttattaccggtacttctttcggtgtcaacatcgattctttgaacaatccacaagatcccttcgttgaatctaccaagaagtttttgaagttcggtttcttggaccccttgttcttgtccattattttgttcccatttctgaccccagttttcgaagccttgaatgtttctttgtttccaaaggacaccatcaatttcttgagcaagtccgttaacaggatgaagaagtctagattgaacgacaagcaaaagcacaggttggatttcttgcaactgatgatcgattcccagaactctaaagaaactgaatcccataaggctttgtccgatttggaattggctgcccaatctatcattttcattttcgctggttacgaaaccacctcctctgttttgtcttttaccttgtatgaattggccactcatccagatgttcaacagaagttgcaaaaagaaatcgatgccgttttgccaaacaaagctccaccaacttatgatgctgttgtccaaatggaatacttggatatggttgtcaacgaaaccttgaggttgtttccagttgctatcagattggaaagaacctgcaaaaaggatgtcgaaatcaacggtgttttcatcccaaaaggttccatggttgtgattccaacttacgcattgcatcatgatccaaagtattggactgaaccagaagaattcagaccagaaagattctccaagaagaaggattccattgatccttacatctacactccatttggtactggtcctagaaactgtattggtatgagattcgctctgatgaacatgaagttggccttgattagagtgttgcagaacttctctttcaaaccctgtaaagaaacgcagatcccattgaagttggatacacaaggtttattgcaaccagaaaagcctatcgttttgaaggtcgattctagagatggtactttgtctggtgagtgaaagactccgcgg

SEQ ID NO: 44 - protein, 503 aa, Macaca fascicularis
MDLIPNLAMETWLLLAVSLVLLYLYGTRSYGLFKRQGIPGPTPLPFLGNILSYRQGLWKFDTECYKKYGKMWRTQDGQLPVLTITDPDMIKTVLVKECYSVFTNRRPLGPVGLMKSAISIAEDEEWKRIRSLLSPTFTSGKLKEMFPIIAQYGDMLVRNLRREAEKGKPVTLKDIFGAYSMDVITSTSFGVNIDSLNNPKDPFVESVKKFLKFDFLDPLFLLTILFPFLIPAFEALNVSLFPKDAINFLNKSVNSMKKSRLNDKQKHRVDFLQLMIDSQNSKETESHKALSDQELVAQSIIFIFAGYETTSSVLSFIIYELATHPDVQQKLQKEIDAVLPNKAPATYDAMVQMEYLDMVVNETLRLFPIAIRLERACKKDVEINGVFIPKGAMVVIPTYALHHDPKYWTEPEEFRPERFSKKNKDSIDPYIYTPFGSGPRNCIGMRFALMNMKLAIIKVLQNFSFKPCKETQIPLKLGNQGLLQSEKPIVLKVESRDGTLSGE

SEQ ID NO: 45 - DNA, 1533 bp, Macaca fascicularis
aagcttaaaatggacttgatcccaaacttggctatggaaacttggttgttgttggctgtttctttggtcttgttgtacttgtacggtactagatcttacggtttgttcaagagacaaggtattccaggtccaactccattgccatttttgggtaacattttgtcctacagacaaggcttgtggaagttcgatactgaatgctataagaaatacggcaagatgtggcgtactcaagatggtcaattgccagttttgactattaccgatccagatatgatcaagaccgtcttggtcaaagaatgctactctgttttcactaacagaaggccattgggtccagttggtttgatgaagtctgctatttctattgccgaagatgaagaatggaagaggatcagatctttgttgtctccaactttcacttccggcaaattgaaagaaatgttcccaattattgcccagtacggtgatatgttggttagaaacttgagaagagaagccgaaaaaggtaagccagttaccttgaaggatattttcggtgcttactccatggacgttattacttctacttctttcggtgtcaacatcgacagtttgaacaatccaaaggatccattcgttgagagcgttaagaagtttttgaagttcgactttttggaccccttgttcttgttgactattctgttcccatttttgattccagctttcgaagccttgaacgtttctttgtttccaaaggacgctatcaacttcctgaacaagtctgttaactccatgaagaagtctaggttgaacgataagcaaaagcacagggttgatttcttgcagttgatgatcgattcccagaactctaaagaaaccgaatctcataaggctttgtccgatcaagaattggttgcccaatccatcattttcattttcgctggttacgaaaccacctcctctgttttgtctttcatcatctatgaattggctacccatccagatgtccaacaaaagttgcaaaaagaaatcgatgccgtcttgccaaacaaagctccagctacttatgatgctatggtccaaatggaatacttggatatggttgtcaacgaaaccttgaggttgttccctattgctatcagattggaaagggcttgcaaaaaagatgtcgaaatcaacggtgttttcattccaaaaggtgccatggttgttattccaacttacgcattgcatcacgatccaaagtattggactgaaccagaagaattcagaccagaaagattctccaagaaaaacaaggattccatcgatccttacatctacactccatttggttctggtccaagaaactgtatcggtatgagatttgctctgatgaacatgaagttggccattattaaggtcctgcagaacttctctttcaaaccatgcaaagaaacccagattccattgaagttgggtaatcaaggtctgttgcaatctgaaaagccaatcgttttgaaggttgaatccagagatggtactttgtctggtgagtaaaagactccgcgg

SEQ ID NO: 46 - protein, 503 aa, Callithrix jacchus
MDLIPNLAVETWLLLALSLVLLYLYGTRSHGIFKKLGIPGPAPLPFVGNILSYRQGIWKFDSECHKKYGKMWGSYDGQLPVLAITDPDIIKAVLVKECYSIFTNRRPLGPVGFMKSAITVAQDDEWKRIRSLLSPTFTSGKLKEMFPIIAQYGDVLVRNLRREAGKGKPVTMKDIFGAYSMDVITGTSFGVNIDSLNNPKDPFVESVKKFLKFDFLDPLFLSTIFFPFLTPVFEALNFSLFPKDAINFLKQSVNRMKKSRLNDKQKHRVDFLQLMIDSQNSNETASHKALSDLELLAQSIIFIFAGYETTSSVLSFTIYELATNPDVQQKLQEEIDVVLPNKAPATYDAVVQMEYLDMVVNETLRLYPIAVRLERVCKKDVEINGVFIPKGALVVIPTYALHHDPKYWTEPKEFRPERFSKKNKDSIDPYIYTPFGTGPRNCIGMRFALMNMKLALIRVLQNFSFKPCKETQIPLKLGVQGLLQAEKPIILKVESRDGTLSGE

SEQ ID NO: 47 - DNA, 1514 bp, Callithrix jacchus
aagcttaaaatggacttgatcccaaacttggctgttgaaacttggttgttattggccttgtctttggtcttgttgtacttgtatggtactagatcccatggcatctttaagaagttgggtattccaggtccagctccattgccatttgttggtaacattttgtcttacaggcaaggcatttggaagttcgattctgaatgccataagaaatacggtaagatgtggggttcttacgatggtcaattgccagttttggctattactgatccagatattatcaaggccgtcttggtcaaagaatgctactctgtttttaccaacagaaggccatttggtccagttggtttgatgaagtctgctatttctttggcccaagatgatgaatggaagagaatcagatctttgttgtctccaactttcacctccggtaagttgaaagaaatgttcccaattattgcccaatacggtgatgttttggtcagaaacttgagaagagaagctggtaaaggtaagccagttaccatgaaggatattttcggtgcttactccatggatgttattaccggtacttctttcggtgtcaacatcgattctttgaacaatccaaaggatcccttcgttgaatctgtcaagaagtttttgaagtttgacttcttggaccccttgttcttgtctactattttctttccattcttgacgccagttttcgaagccttgaattttagcttgttcccaaaggatgctatcaacttcctgaagcaatccgttaacaggatgaagaagtctagattgaacgacaagcaaaagcacagggttgatttcttgcaactgatgatcgattcccagaactctaacgaaactgcttctcataaggctttgtctgatttggaattgctggcccaatccattattttcattttcgctggttacgaaaccacctcctctgttttgtcttttaccatctatgaattggccaccaatccagatgttcaacagaaattgcaagaagaaatcgacgttgtcttgccaaacaaagctccagctacttatgatgctgttgtccaaatggaatacttggatatggttgtcaacgaaaccttgaggttgtatccaattgctgtcagattggaaagggtctgcaaaaaggatgttgaaatcaacggtgttttcattccaaagggtgctttagttgttattccaacttacgccttgcatcacgatcctaaatattggactgaacccaaagaattcagaccagaaagattctccaagaaaaacaaggattccatcgatccttacatctacactccatttggtactggtcctagaaactgtattggtatgagattcgctctgatgaacatgaagttggccttgattagagtgttgcagaacttctctttcaaaccctgtaaagaaacccagattccattgaaattgggtgtccaaggtttgttgcaagctgaaaaacctatcatcttgaaggttgaatccagagatggtactttgtctgg

SEQ ID NO: 48 - protein, 134 aa, Homo sapiens
MAEQSDEAVKYYTLEEIQKHNHSKSTWLILHHKVYDLTKFLEEHPGGEEVLREQAGGDATENFEDVGHSTDAREMSKTFIIGELHPDDRPKLNKPPETLITTIDSSSSWWTNWVIPAISAVAVALMYRLYMAED

SEQ ID NO: 49 - DNA, 419 bp, Homo sapiens
aagcttaaaatggccgagcaatctgatgaagcagtgaagtactacacattagaagagatacaaaaacacaaccattcaaaaagcacttggctcattctacaccataaagtttatgatttgactaagtttttggaggaacatccaggaggtgaagaggtccttagagaacaggcaggcggtgacgctactgaaaactttgaagatgttgggcattcaaccgacgctagagaaatgagtaaaactttcattattggtgaacttcacccagatgacagaccaaaactgaataagcctcctgaaacactaataacgacaatcgattcttcctcttcatggtggacaaattgggttatcccagcgatctctgccgtcgctgtagcattaatgtataggttgtacatggctgaagattaaccgcg

SEQ ID NO: 50 - protein, 677 aa, homo sapiens
MGDSHVDTSSTVSEAVAEEVSLFSMTDMILFSLIVGLLTYWFLFRKKKEEVPEFTKIQTLTSSVRESSFVEKMKKTGRNIIVFYGSQTGTAEEFANRLSKDAHRYGMRGMSADPEEYDLADLSSLPEIDNALVVFCMATYGEGDPTDNAQDFYDWLQETDVDLSGVKFAVFGLGNKTYEHFNAMGKYVDKRLEQLGAQRIFELGLGDDDGNLEEDFITWREQFWPAVCEHFGVEATGEESSIRQYELVVHTDIDAAKVYMGEMGRLKSYENQKPPFDAKNPFLAAVTTNRKLNQGTERHLMHLELDISDSKIRYESGDHVAVYPANDSALVNQLGKILGADLDVVMSLNNLDEESNKKHPFPCPTSYRTALTYYLDITNPPRTNVLYELAQYASEPSEQELLRKMASSSGEGKELYLSWVVEARRHILAILQDCPSLRPPIDHLCELLPRLQARYYSIASSSKVHPNSVHICAVVVEYETKAGRINKGVATNWLRAKEPAGENGGRALVPMFVRKSQFRLPFKATTPVIMVGPGTGVAPFIGFIQERAWLRQQGKEVGETLLYYGCRRSDEDYLYREELAQFHRDGALTQLNVAFSREQSHKVYVQHLLKQDREHLWKLIEGGAHIYVCGDARNMARDVQNTFYDIVAELGAMEHAQAVDYIKKLMTKGRYSLDVWS

SEQ ID NO: 51 - DNA, 2040 bp, homo sapiens
taaaatgggtgattcacatgttgatacatcttctacagtttcagaagctgttgctgaagaagtttctttattttcaatgactgatatgattttgttttcattaattgttggtttgttgacatattggttcttgtttagaaagaagaaggaagaagttccagaatttactaagattcaaaccttgacatcttcagttagagaatcatcttttgttgaaaagatgaagaagactggtagaaatattattgttttctacggttctcaaactggtactgctgaagaatttgctaacagattgtcaaaggatgcacatagatatggtatgagaggtatgtctgctgatcctgaagaatatgatttagcagatttatcttcattgcctgaaattgataatgctttagttgttttctgtatggctacttatggtgaaggtgatcctactgataacgctcaagatttttatgattggttgcaagaaactgatgttgatttatctggtgttaagttcgctgttttcggtttgggtaataagacttatgaacatttcaacgctatgggtaaatacgttgataaaagattggaacaattgggtgctcaaagaatttttgaattaggtttgggtgatgatgatggtaacttagaagaagattttattacatggagagaacaattttggcctgcagtttgtgaacatttcggtgttgaagctaccggtgaagaatcatctattagacaatatgaattggttgttcatacagatattgatgctgctaaagtttacatgggtgaaatgggtagattgaaatcatatgaaaatcaaaagccacctttcgatgctaagaatcctttcttagctgcagttacaacaaacagaaagttgaatcaaggtacagaaagacatttgatgcatttggaattggatatttctgattcaaaaattagatacgaatctggtgatcatgttgctgtttatccagctaatgattctgctttagttaaccaattaggtaaaattttgggtgctgatttagatgttgttatgtctttaaataacttagatgaagaatctaacaagaaacatccattcccatgtcctacttcatacagaacagctttaacttattatttagatattacaaaccctccaagaactaatgttttgtatgaattggctcaatatgcatctgaaccttctgaacaagaattgttaagaaaaatggcttcttcatctggtgaaggtaaagaattatacttgtcatgggttgttgaagctagaagacatattttagcaattttacaagattgtccatcattgagaccaccaattgatcatttgtgtgaattgttgcctagattacaagctagatattattctattgcatcatcttctaaagttcatccaaattcagttcatatttgtgctgttgttgttgaatatgaaactaaggctggtagaattaacaaaggtgttgcaactaattggttgagagctaaggaacctgctggtgaaaatggtggtagagcattagttccaatgttcgttagaaagtctcaatttagattgccatttaaagctactacaccagttattatggttggtcctggtacaggtgttgctccttttattggtttcattcaagaaagagcatggttaagacaacaaggtaaggaagttggtgaaacattattatattacggttgtagaagatcagatgaagattatttgtacagagaagaattagcacaattccatagagatggtgctttgacacaattgaatgttgctttttcaagagaacaatctcataaagtttatgttcaacatttgttgaaacaagatagagaacatttatggaagttgattgaaggtggtgcacatatttatgtttgtggtgatgctagaaacatggcaagagatgttcaaaatacattctatgatattgttgctgaattaggtgctatggaacatgcacaagcagttgattacattaagaaattgatgacaaaaggtagatattctttggatgtttggtcttaacc

SEQ ID NO: 52 - DNA, 1572 bp, Mucor circinelloides
atgactttgattgcttcttataatcaaactttgttggaaagagttatttctgttgttagaaaaaataaaacttcttatattggtatggctattttgtgtgttgttttgcaacaagtttatgcttcttttactgttccaccaaaatatttgagaagatacccaactgtttctttttttgaaatgatgaaatctttttatagaaaagaatctgttttgaatagaaataaaagattggttactccattgactaatgctggtcatggtttttatgtttgtagaataccattggattggactatttatgttactgatccaattgctgctaaaactttgttgttgaaaactgataattttccaaaatctcatgctatttttggtgctttgggtgaatcttctccagcagttaaatttatgggttctgaaaatgttgctgtttctaatggtgaaatgtggaaaaaacaaagaaaaattatgaatccagcttttcatagatctcaaccagttaaattgtttggtggtgttatgccagatttgtttgctttgattgatcaagatccagaacatgtttttgttgctccaagaatgaaatcttttgctttggatgctttgggtttgtctgcttttggttttgattttcaatctttgaaaggtgatccagaaggttggacttctaaatataatactgttatttctactttgtttaatccatttattaatttgtttgctaaatatgattttttgattaaatatatttctccagaaagaagaagagttattaaagctactgatgaatttaatgttatgttgtctaatttggctgataaaagaagacaagaaattttggatggtgaaaaaaaagatatggctgaaaatgaaaaagatttgttgactttgatgattgaagctgatattagagaaggtgttgaaactactactactgaattgagacataatatggctattttttttttggctggtcatgatactactgctaatactttggctttgtgtttgtatcaattggctaaacataaacatgttcaaaaaaaagctagacaagaagttttggatattttgggtgatgatccatgtgatgttactccaactttggaagatttgaaaaaattgaattatgttaatatggttattaaagaaaatttgagaagaaattctccagttgataatttgatggctagagatactcatcaagatattgatttgaatggtacttttattccaaaaggttctaaagttactgttaatgttgcttctattcatttgaatccaaaaatttggcatgatccagaatcttttattccagaaagatttgaaccaggtggtgaatatgatggtcatgatggttttacttggattccattttctaatggttctagacaatgtttgggtttgaatttttctttgactgaacaaagagttgttttgtgtatgttgttgaaaagatatgaaattgaaattccaaaagattctattcattataatgaaattgtttttgataaaccatttacttttgctccacaatctttggaattgtcttttaaaaaaagatattag

SEQ ID NO: 53 - protein, 523 aa, Mucor Circinellloides
MTLIASYNQTLLERVISVVRKNKTSYIGMAILCVVLQQVYASFTVPPKYLRRYPTVSFFEMMKSFYRKESVLNRNKRLVTPLTNAGHGFYVCRIPLDWTIYVTDPIAAKTLLLKTDNFPKSHAIFGALGESSPAVKFMGSENVAVSNGEMWKKQRKIMNPAFHRSQPVKLFGGVMPDLFALIDQDPEHVFVAPRMKSFALDALGLSAFGFDFQSLKGDPEGWTSKYNTVISTLFNPFINLFAKYDFLIKYISPERRRVIKATDEFNVMLSNLADKRRQEILDGEKKDMAENEKDLLTLMIEADIREGVETTTTELRHNMAIFFLAGHDTTANTLALCLYQLAKHKHVQKKARQEVLDILGDDPCDVTPTLEDLKKLNYVNMVIKENLRRNSPVDNLMARDTHQDIDLNGTFIPKGSKVTVNVASIHLNPKIWHDPESFIPERFEPGGEYDGHDGFTWIPFSNGSRQCLGLNFSLTEQRVVLCMLLKRYEIEIPKDSIHYNEIVFDKPFTFAPQSLELSFKKRY

SEQ ID NO: 54 - DNA, 1542 bp, Lichtheimia corymbifera
atgactgaaattaaagatcatatttatagatatagacattatattggtgttgctgctgctgttttgttggtttgtcaacaagtttatcatagaatttttagaataccaaaaaatttgagacatttgccagctattccatacggtaaacaattgaaagcattgcaatctcaagaaaatttgatttctagaactcaaagattggtttttccattgttgccaaaagctcatggtgtttatttgaatagaatgccatttcaatggactatttatgttgctgatccagaaattgctagaattgttttttttaaaccagaatttgctaataaaacttcttctgttttggattctattgatcaaaatactactttgattgaatttgttggtaatgataatgtttctattgttaatggtcatcattggaaagatcaaagaaaaattatgaatccagcttttcatagagctactccagttggtatgtttggttctttgatgccaaaagtttttagattggttgaagaacaaccaactgttccagttttggaattgatgcaaaaattgactttggatgctttgggtaaatctgtttttggttttgattttggtggtttggatgatccagattctgtttgggttaaaacttatagattgttgtttgatggttttactaatgttattccattggtttttccaagattggatggtttgtatagatatttttctgctaaaagaagagcacaacatgatgctgtttataaattgattgatttgttggatggtgttgctgataaaaaaagatctatgttgcaagatgattctaattctcataatgatgttccagaacatgaaaaagatttgttgcaattgatgttggaagctgaattgagaggtgaaggtaattggactaaaaaagaattgagacataatatggctattttttttgttgctggtcatgatactacttctcatgctttgactttttgtttgtatttgttggctatgaatcaagatattcaaaaaaaagctagagaagaaattttgagagttttgggtgatgaaccaaaagatgtttttccaactttggaagattgtaaaaaattggattatttggatatggttattaaagaatctatgagaatttatccaccagctaatgatattttggctagagatgttcatgaagatttgaatgttaaaggtatttttattccaaaaggtgctatggtttctgttgatattcaagcattgcatcatagaccagatttgtggcatgaaccagaaaaatttaatccagatagatttttgccaggtggtgaacatgattctcatgaaggtattgcttatgctccattttcttctggtgctagacaatgtattgctttgaaattttctattatgcaacaaagagttgttttggctatgttgttgagaaaatttgaatgggaattgccaaaagaatctaaacataaagatggtattcaatttgaaattccatttaatttggctccaaaagatttggaattgatttttcataaaagatattag

SEQ ID NO: 55 - protein, 513 aa, Lichtheimia corymbifera
MTEIKDHIYRYRHYIGVAAAVLLVCQQVYHRIFRIPKNLRHLPAIPYGKQLKALQSQENLISRTQRLVFPLLPKAHGVYLNRMPFQWTIYVADPEIARIVFFKPEFANKTSSVLDSIDQNTTLIEFVGNDNVSIVNGHHWKDQRKIMNPAFHRATPVGMFGSLMPKVFRLVEEQPTVPVLELMQKLTLDALGKSVFGFDFGGLDDPDSVWVKTYRLLFDGFTNVIPLVFPRLDGLYRYFSAKRRAQHDAVYKLIDLLDGVADKKRSMLQDDSNSHNDVPEHEKDLLQLMLEAELRGEGNWTKKELRHNMAIFFVAGHDTTSHALTFCLYLLAMNQDIQKKAREEILRVLGDEPKDVFPTLEDCKKLDYLDMVIKESMRIYPPANDILARDVHEDLNVKGIFIPKGAMVSVDIQALHHRPDLWHEPEKFNPDRFLPGGEHDSHEGIAYAPFSSGARQCIALKFSIMQQRVVLAMLLRKFEWELPKESKHKDGIQFEIPFNLAPKDLELIFHKRY

SEQ ID NO: 56 - DNA, 1593 bp, Lichtheimia corymbifera
atgtcttctttgaatattttgtctttgttggataataaacatattaatgctttttttgataatccatctagagcacaatctggtattattgctggttctgttgctattgtttctttgtgtgctgcttattctttgggttctagattgagaggttctaataatggtgttccattggttccatatacttttccaattattggttctactaaagaatatcaagctgatccacaagcatttattgaaaaatggactgctaaattgggtccagtttttagagttcatttgtttggtagaatacatactgttgtttctgatagatatgttagagaagtttttttgaataatgattttgattttttgaaaggtactggtaaaagatttgatactttgttgttgactgatactactttggaagatgttgatattgaagtttttagaactgttgttatgaaacatttgactaaagaaatgaaacattatactccaagagttgttgaacatttgactgctggtggtgatgaaaaattgggtgatgctactgaaccaaaagaattggttcatttgtttccattgttgcaacacatggttgctaaagcatctgcttctatttttgttggtactgaattggctgctgatgatgctgttgttgaaacttgtaaaaatattgctattgatattggttctgaattgggtccatcttcttatattatggatgcttttccatctttggctagattgagaatgtggtatattggtaaatatggtaaagctattaataaacatagacaacatttgttgcacgctttgggtccagttattgataaaagattggctgctgctgaaaaaggtggtgattgggatagaccacaagatattttgcaagatattattgaaactattaatttgactttggataatccaaaaagacatattttgccagttaaatggttgttggctttgttttttgcttctattcatactacttctgaaaattctactattgttttgtatagaattatgcaaaatccagaaattattgatgttttgttggaagaacaaaatgaaattttggaaaaacattatggtactaatattgattattctgatactactaaattgtttactggtgaagttattaaagaaatggttaaattggattctgtttgtagagaagctatgagatctagaaattcttatttggaattgccacatacttatgttggtaaatctagaattactttgtcttgtggtgctgttattgaaccaggtcatgatgttttgattaatatgtggggtaatcatagagatgctaaaattcaaagagatactattggtgatcatcatgattttaaaccatttagatttgttggtttggatagacaatctactaaaattggtgatgattttttgatgtttggtcaaggtagacatgcttgtccaggtagatggtttgctattcaagaaattaaaactattgtttctgttttgattagatattataaattgactccaaaaggtccaattacttttccaactcatccaagaatgccaatgccaactggtgaagttattattcaaagaagacaagaatag

SEQ ID NO: 57 - protein, 530 aa, Lichtheimia corymbifera
MSSLNILSLLDNKHINAFFDNPSRAQSGIIAGSVAIVSLCAAYSLGSRLRGSNNGVPLVPYTFPIIGSTKEYQADPQAFIEKWTAKLGPVFRVHLFGRIHTVVSDRYVREVFLNNDFDFLKGTGKRFDTLLLTDTTLEDVDIEVFRTVVMKHLTKEMKHYTPRVVEHLTAGGDEKLGDATEPKELVHLFPLLQHMVAKASASIFVGTELAADDAVVETCKNIAIDIGSELGPSSYIMDAFPSLARLRMWYIGKYGKAINKHRQHLLHALGPVIDKRLAAAEKGGDWDRPQDILQDIIETINLTLDNPKRHILPVKWLLALFFASIHTTSENSTIVLYRIMQNPEIIDVLLEEQNEILEKHYGTNIDYSDTTKLFTGEVIKEMVKLDSVCREAMRSRNSYLELPHTYVGKSRITLSCGAVIEPGHDVLINMWGNHRDAKIQRDTIGDHHDFKPFRFVGLDRQSTKIGDDFLMFGQGRHACPGRWFAIQEIKTIVSVLIRYYKLTPKGPITFPTHPRMPMPTGEVIIQRRQE

SEQ ID NO: 58 - DNA, 1548 bp, Absidia repens
atgaataaattgtttccagttggtacttctaataaaaaaaaagctgttttgttgtctttgggtgctactgttgctttgatttgtagagctatttatagaatttattatgttccaagatctttgagacatattccatctgttggttattttagattgattagatctattttgagaagagaagatgctactactagagctagaactgtttatggtccagctattaaaaaaggtaatggtatttatttggctaattttccaattacttggtctgtttttgtttcttctccaattgctgctaaatctgttttgatgaaaactgataattttccaaaatctatggaaatttttcatgctttgggtaaagaaaatccagttgttagattttttggtattgataatgttgctattgttaatggtgaaaaatggaaaaaacaaagaaaagttatgaatccagcttttcatagagctatgccagttcaaatgtttggtagattgatgttgaaaggttttaaaaatattgaaaaacaagattatcaagttccaattttggatttttttcaaagattgactttggatgctttgggtattgctggttttggttttgattttcattctgttgatgatccagaatctatttggactaaaacttatgaaaatgttagattgggtttgagatctccattttcttttttgtttccatctatggattggttgttgaaatatattattccaggtagaaaagaattggataaatctgttgataaattgaatgctttgttgatgtctatggctcaagaaagaagattgcaagttagagcttctattgatgataatgttccagattctgaaaaagatttgttgactttgatgttggaagctgaattgagaggtgaaggtactgcttctgatgaacaattgagatctaatttggctgttttttttttggctggtcatgaaactactgctaatactatgtctttttgtttgtataatttggctatgaataaagaagttcaatctaaagctagacaagaagttttgactgttttgggtgatgaaccagttgatattttgccacaaattgatgaattgagacaaatgccatatattgatatggttttgaaagaaaatttgagaagatttggtccagcttctatgttgattgctagaaaatctcaagaagattttgatttgaatggtgtttttattccaaaaaatactccagttgttgttgaaactcatgctttgcatcataatccagatgtttggaaaaatccagaacaatttgatccagaaagatttgctccaggtggtgaacatgaaacttgtcatgaaggtatggcttggttgccattttcttctggttctagaggttgtttgggtatgaatttttctttggctgaacaaagaacttttttggttatgttgttgagaaaatatgaatgggaattgccagaagattctattcatagaaatggtgttaaaattcaaaattttcaaaatgctgctccagaatctttggaaattaaattttcttctagatattag

SEQ ID NO: 59 - protein, 515 aa, Absidia repens
MNKLFPVGTSNKKKAVLLSLGATVALICRAIYRIYYVPRSLRHIPSVGYFRLIRSILRREDATTRARTVYGPAIKKGNGIYLANFPITWSVFVSSPIAAKSVLMKTDNFPKSMEIFHALGKENPVVRFFGIDNVAIVNGEKWKKQRKVMNPAFHRAMPVQMFGRLMLKGFKNIEKQDYQVPILDFFQRLTLDALGIAGFGFDFHSVDDPESIWTKTYENVRLGLRSPFSFLFPSMDWLLKYIIPGRKELDKSVDKLNALLMSMAQERRLQVRASIDDNVPDSEKDLLTLMLEAELRGEGTASDEQLRSNLAVFFLAGHETTANTMSFCLYNLAMNKEVQSKARQEVLTVLGDEPVDILPQIDELRQMPYIDMVLKENLRRFGPASMLIARKSQEDFDLNGVFIPKNTPVVVETHALHHNPDVWKNPEQFDPERFAPGGEHETCHEGMAWLPFSSGSRGCLGMNFSLAEQRTFLVMLLRKYEWELPEDSIHRNGVKIQNFQNAAPESLEIKFSSRY

SEQ ID NO: 60 - DNA, 1560 bp, Thamnostylum piriforme
atgatttcttatccagttgttagagatagattgtctagatataaatattatattgttattggtgctttgttttctattgcttggcaacaaatttattatagattttttagagttccaagaaatttgagacatattccatctattgcttatgctcaacaattgttggctttgttgagaggtgaaccaattactttgagaactcaaagattggtttttccattgttgtctaaagctaatggtatttatttgaatagagcaccatttttgtggactatttttgttgctaatccagttttggctaaagaagttttgtttaaatctgaattggctaataaaaatactattttggatgcttttccaaaagattctgcttttgttgaatttgttggtaaagataatgttgctttttctaatggtgaaaaatggaaaagacaaagaaaaattatgaatccaatttttcatagagctactactgctgctgcttttgcttctgttactttgaaattgtttagagttattgatgatactcaagctgctggttctcatgttgctgttccaattttgatgaaaagattggctttggaagcattgggtagaactatgtttggttttgattttggtggtttggaagatgaaggttctgaatgggttgctgcttgtaatgaagtttttacttctttttctgattttacttctttgtctgctagagctgatgctatgttgagagttttttctagatctagacaagaaaaatataaagctagatttagattgattaatatgtttgatgatatgattgaacaaagaagagttactttgttggatactaaagaaacttcttctactaatgttccagataatgaaaaagatttgttgactttgttgttggaagctgaaatgagaggtgaaggtacttggagaaaaaatgaattgagatataatattgctactttgttttttgctggtcatgatactactgcttctactttgtcttttgctttgtattctttggctgttaataaagaagttcaatctaaagctagagaagaagttaatgatttgttgggtaataatcataatgatgttgctccaactttggaacaatgtaaacaattgccatatattgatatgattattaaagaaactttgagaatgtattctccatctgatcatttgtttgctagagttgcttctgatgatttggaattgggtggtgttttgattccaaaaggtgctaaagtttctgttgattttcatgctttgcattatcatccagatttgtgggaagctccagaaagatttattccagaaagattttctgattctggtgaacattctaaacatgaaggtattacttgggctccattttctggtggttctagacaatgtattggtttgaatttttctatgactgaacaaagagttgctttgtctatgttgttgagaaaatatgaatgggaattgccagcaggttctattcatgaaaaaggtttggttatggatcaaccatataattttgctccaatgtctttggaattgagatttaaaaaaatttattag

SEQ ID NO: 61 - protein, 519 aa, Thamnostylum piriforme
MISYPVVRDRLSRYKYYIVIGALFSIAWQQIYYRFFRVPRNLRHIPSIAYAQQLLALLRGEPITLRTQRLVFPLLSKANGIYLNRAPFLWTIFVANPVLAKEVLFKSELANKNTILDAFPKDSAFVEFVGKDNVAFSNGEKWKRQRKIMNPIFHRATTAAAFASVTLKLFRVIDDTQAAGSHVAVPILMKRLALEALGRTMFGFDFGGLEDEGSEWVAACNEVFTSFSDFTSLSARADAMLRVFSRSRQEKYKARFRLINMFDDMIEQRRVTLLDTKETSSTNVPDNEKDLLTLLLEAEMRGEGTWRKNELRYNIATLFFAGHDTTASTLSFALYSLAVNKEVQSKAREEVNDLLGNNHNDVAPTLEQCKQLPYIDMIIKETLRMYSPSDHLFARVASDDLELGGVLIPKGAKVSVDFHALHYHPDLWEAPERFIPERFSDSGEHSKHEGITWAPFSGGSRQCIGLNFSMTEQRVALSMLLRKYEWELPAGSIHEKGLVMDQPYNFAPMSLELRFKKIY

SEQ ID NO: 62 - DNA, 1650 bp, Cunninghamella echinulata
atgtctcaatttatttctactatttctcaatattgggatgttaataattttattgatcaacaagcatggtctagattttatgaaacttatttgttgaaatatactgattctaaagctaaaagattgactattggtgtttctgtttctttgttgttgttgggttatggtattaaaagattgttgactccaccaaaacatttgagacatattaaacatgcttcttttttgagatttacttataattttgttattaaaggtgttactccaaaagaaatgcatactactgtttctaaaaaaattgttgaagaaaataatggtttttatttgcaattggaaagaactggttgggttgtttatgttgctaatccagaagctgttaaacaagttttgttgaaatctgatatttttccaaaaatggatttttctaaattggcttctgaagaaggttcttattttgaaaaatttattggttttaaaaatattttgatgactactggttctgaatggttgaaacatagaaaattgactaatccagcttttcatagatctttgccagctaaattgtttggtgaaactgctcaaggtttgtttaaaatttgggataatgaatataatgataaaccatttgaagttaatattcataatatgaatgaaagaattactttggatattattggtaaagctggttttgcttttgattttaatgctgttgctgatgaaaaatctccttggaaaaaaacttatgatattattaatactgctgcttctgatccattgttttttatgtttccaattttggaaaataaattgttgtggttgtttccaaaaagacaagaatcttttaaaaaattggatgaatggaaagctatgttgacttctgttattgaaaataaaagaagattgttgaaagataatattgatcaaggtgttgaagaagctgaaaaagatttgttgactttgatgattgaatctgaatttagaggtgaaggtgttttgactaaagaagaattgattggtaatttgactgttttttttttggctggtcatgatactacttcttttgctttgacttctgctatttattatatggctagatacccagaaattcaagaaaaagctagacaagaagttaattctattttgtgtccaaatggtgaaccaaatgaaggtattttgccaactattgaagatactaaaaaattggtttatttgaatcaaattatgaaagaatctatgagaattggtaatccagttttgtttttgttgtctccaagacaagctactaaagattttaatttgaatggtacttttattccaaaaggtactcaagttaatattaatattcatgatttgcatcattcttctaatgtttgggatgatccagatacttttaatccagatagatttgctccaggtggtgaagctgataaaaaaactggtattgcttgggttccattttctaatggttctagacaatgtttgggtatgaatttttctttgttggaacaaagagttattttgtcttgtttgttgagaaaatatgaatggactttgccagaaaattctattcataaaaatgatatgatttctaaatttgatttgattccatctccaattgatatgaaaattagatttgaaagaagatattaa

SEQ ID NO: 63 - protein, 549 aa, Cunninghamella echinulata
MSQFISTISQYWDVNNFIDQQAWSRFYETYLLKYTDSKAKRLTIGVSVSLLLLGYGIKRLLTPPKHLRHIKHASFLRFTYNFVIKGVTPKEMHTTVSKKIVEENNGFYLQLERTGWVVYVANPEAVKQVLLKSDIFPKMDFSKLASEEGSYFEKFIGFKNILMTTGSEWLKHRKLTNPAFHRSLPAKLFGETAQGLFKIWDNEYNDKPFEVNIHNMNERITLDIIGKAGFAFDFNAVADEKSPWKKTYDIINTAASDPLFFMFPILENKLLWLFPKRQESFKKLDEWKAMLTSVIENKRRLLKDNIDQGVEEAEKDLLTLMIESEFRGEGVLTKEELIGNLTVFFLAGHDTTSFALTSAIYYMARYPEIQEKARQEVNSILCPNGEPNEGILPTIEDTKKLVYLNQIMKESMRIGNPVLFLLSPRQATKDFNLNGTFIPKGTQVNINIHDLHHSSNVWDDPDTFNPDRFAPGGEADKKTGIAWVPFSNGSRQCLGMNFSLLEQRVILSCLLRKYEWTLPENSIHKNDMISKFDLIPSPIDMKIRFERRY

SEQ ID NO: 64 - DNA, 1392 bp, Rhizopus delemar
atggtcaagtccttcttgaaggctgaatctccaactgatagatacaagagaatcattcatccagtcgcctctaaaggtaatggtttctacgtttctaaggtcccatttttgtgggctgtttacgttactaatccagttgttgctaagcaggtcttgttgaagtctgatattttcccaaagaaccatgccgttttccatcaaattggtaaggattctccattcactcagttcttgggtttagataacgttgctttgtctaacggtgatgtctggaaaaagcaaagaaaggttatgaacccagccttccatagatctttgccaatcaaaactatggcctctgttgttaacaccttgttctccgttattgataactctgatggtccagttttgatcacttctgctatgcaaaacttcaccttggatgttttaggtttggccattttcggtttcgaattcaaggctttacaaggtgatccagataactggactaagacttacaagaccgttatcgaatctttgttcgatccagtcatgaacgttttcgctactttcgatactttgttgacatgggtttaccccaagagaagagaatgttctgttgccatttctaagatgaacttgaagttcgatgaactggccaaacaaaaaagagccgaagttaagtctggtgcttatgctaatgttccagatcacgataaggatctgttgaccttgatgttggaagctatggaaaaaggtgaagccttgacttctcaagacgaattgagacataacattgccgtttttttcttggctggtcatggtactactgctcatactttgtctttctgcttttaccatctggctaagaacaagcacatccagagaaaattgagggaagaaatcatctccgttttgggtgatgaaccagttgatatagttccatccttggaacaaatgaagcacatgaagtatatgaacctggtcatcaaagaaaacctgagaatgaatactccagccgataccttgtttactagagatactgttgaggatattaacttggccggtcatatcattccaaaggataccgctatttccatcgatattaacgccattcatcacgatccaaagtactggcataatccagaacatttcatcccagaaagatttgctgaaggtggtgaacaagaatctcatgaaggtttgacttggttgccattctcaaatggttctagacaatgtatcggcatgaacttctcattggctgaacagagattggttttggctatgttggttaggaagtacgaaatcgatatcccaaaggattccatccactacgaaagaatcttgtttgacagaccaggtaacattgctccattgtctttgggtttgaccttcaccaagagatattaa

SEQ ID NO: 65 - protein, 463 aa, Rhizopus delemar
MVKSFLKAESPTDRYKRIIHPVASKGNGFYVSKVPFLWAVYVTNPVVAKQVLLKSDIFPKNHAVFHQIGKDSPFTQFLGLDNVALSNGDVWKKQRKVMNPAFHRSLPIKTMASVVNTLFSVIDNSDGPVLITSAMQNFTLDVLGLAIFGFEFKALQGDPDNWTKTYKTVIESLFDPVMNVFATFDTLLTWVYPKRRECSVAISKMNLKFDELAKQKRAEVKSGAYANVPDHDKDLLTLMLEAMEKGEALTSQDELRHNIAVFFLAGHGTTAHTLSFCFYHLAKNKHIQRKLREEIISVLGDEPVDIVPSLEQMKHMKYMNLVIKENLRMNTPADTLFTRDTVEDINLAGHIIPKDTAISIDINAIHHDPKYWHNPEHFIPERFAEGGEQESHEGLTWLPFSNGSRQCIGMNFSLAEQRLVLAMLVRKYEIDIPKDSIHYERILFDRPGNIAPLSLGLTFTKRY

SEQ ID NO: 66 - DNA, 1584 bp, Rhizopus microsporus
atggaattgaccgaaatcgccatcgaaacttatcatagagctttggataagctggtcccaatcttgcaaaaaagatccaagagatcctacattggtgttgctgttgctttggttgttttggaaagaatctacagcttcttcagagtcccaaagtccattagacatattccagctgttccatactttgctatggctaagtctttcttgacttctgaagctccatcttccagacatcaaagaatagttttgccagtcatcgagaaaggtaatggtatctacgttaacaagttgccattggaatggactgttaatgttgctactccaacctctgctaaacacgttttgttgaagtctgaaatctaccccaagtccgaatcctttttgaaattattgggtccacaatctccagccgttttgtttttaggtggtaagaatgttggtttcgttaacggtgatgcttggagaaagcaaagaaagattatgaacccagccttccatagatccatgccaattcaaactatggcttctgttatgccagatttcttctcagccattgataagtatggtgatgaaggtattccaatctccaccatcatgagagatttcaccttggatgttttgggtcatactgcttttggtttcgatttcaaggctttgaaaggtgatccagataactggactagaacctaccatatcattaacaacgctttgttcaacccaaccgctaatatgttgacttctttgaaccctatcctgtccattatctctccagaaagaagaagaattttggaggccatcaaaaagttgaacggtatgttggaagccatgatcaagcaaaagagacaagaagttcaatccaacgctcaagctcatgctccagaaaacgaaaaagatttgttgaccttgatgttggaggctcaacaaagaggtgaaggtttggctactgatgaagaattgaagcacaatgtctctggttttttcttggctggtcatgatacaacctctgaaactttgtctttctacttctacaacattgccaagaacaaggacgtccaaagaaagttgagagaagagttgaatgctgtcttgggtgataagccagttgatgttattccaaccttggagcaattgaagtccatggaatatttgaactgcaccatcaaagaaaacttgaggttgaatggtccagccgataatgttttgccaagagttgctactgaagatatggttgttgatggtactccaattccaaagggtactgttgtgaacgttgatattcatgccattcatcacgataccagatactggaaagatccatacaagtttgtcccagaaagatttttgccaggtggtgaacatgattctcattctggtatgacttggttgccttttggtaatggtgctagacaatgtttgggtatgaatttctcattggccgaacagagattggttattgctatgactgttaggaagtacgatatcgaagttccaaaggattccatccattacgatcatccaatcctggaatcttctaaaacaaaagctccagcctccttgaagttgatcttcagaaagagatactga

SEQ ID NO: 67 - protein, 527 aa, Rhizopus microsporus
MELTEIAIETYHRALDKLVPILQKRSKRSYIGVAVALVVLERIYSFFRVPKSIRHIPAVPYFAMAKSFLTSEAPSSRHQRIVLPVIEKGNGIYVNKLPLEWTVNVATPTSAKHVLLKSEIYPKSESFLKLLGPQSPAVLFLGGKNVGFVNGDAWRKQRKIMNPAFHRSMPIQTMASVMPDFFSAIDKYGDEGIPISTIMRDFTLDVLGHTAFGFDFKALKGDPDNWTRTYHIINNALFNPTANMLTSLNPILSIISPERRRILEAIKKLNGMLEAMIKQKRQEVQSNAQAHAPENEKDLLTLMLEAQQRGEGLATDEELKHNVSGFFLAGHDTTSETLSFYFYNIAKNKDVQRKLREELNAVLGDKPVDVIPTLEQLKSMEYLNCTIKENLRLNGPADNVLPRVATEDMVVDGTPIPKGTVVNVDIHAIHHDTRYWKDPYKFVPERFLPGGEHDSHSGMTWLPFGNGARQCLGMNFSLAEQRLVIAMTVRKYDIEVPKDSIHYDHPILESSKTKAPASLKLIFRKRY

SEQ ID NO: 68 - DNA, 1488 bp, Parasitella parasitica
atggccgttttgtgcttggtcttggaaagaatctatgcttcttatgctgttccaccatcctacttgagacattacccaaaggtttctttgttcgacatgctgaagtccttctacatcaaagaatctgttgcctccagaaacaagagattgattgctccattgactaatgctggtcatggtttttacgtctgcagaattccattgaactggactatctatgttaccgatccattggctgctaagactttgttgttgaagtctgaaaacttcccaaagaacaaggctattttcactgctttgggtgattcttcaccagtcattaagttcatgggtaaagaaaacgttgccatgtctaatggtgaagagtggaaaaagcaacgtaagattatgaacccagccttccatagatctcaaccagttaagacttttggtaacgttatgccagatttgttcgccttgattgatcaagatccagaaagagttttcatcacgccaaagatgaagtcttttgctttggatgctttaggtttgtctgctttcggtttcgatttccaatctttgaaaggtgatccagaaggttggactagaaagtacaatgttgttatctccaccttgttcaaccccttcgttaatatctttgcctccttggatttcctggtcaagtatatttcaccagaaagaagaagagttatcaaggccactgatgagttcaattctatgttgggtgaattggcagataagagaaggcaagaaattttggacggtgagaaaaagaacatcccagaaaacgaaaaggacctgttgaccttgatgattgaagccgatattagagacaacattaagactactaccaccgaattgagacataacatggccattttctttttggccggtcatgattctacagctaacactttgtctctgtgcttgtacaatttggctaaacacaagcacgttcaaaagaaggctagacaagaagttttggctatcttgggtgatgaaccattggatgttattccaactgctgaggacttgaagaagttggattacgttaacatggtcatcaaagaaaacctgagaagaaatggtccagccgataatttgatgtctagagatactcaacaggacatgaacttgaacggtactattattccaaagggctccaaggtttctgttaacgttgctgctattcatctgaacccaaagatttggcatgacccagaaaatttcattccagaacgttttgagcaaggtggtgaattcgaacaacatgatggttttacttggatcccattctctaacggttctagacaatgtttgggtctgaacttctcattgactgaacaaagggttgttctgtgcatgatcttgaagagatacgaaatcgatatccccaaggattccatccattacaacgaaatcgttttcgatggtgcttttactttcgctccacaatctttggaactgtccttcaagagaagatactga

SEQ ID NO: 69 - protein, 495 aa, Parasitella parasitica
MAVLCLVLERIYASYAVPPSYLRHYPKVSLFDMLKSFYIKESVASRNKRLIAPLTNAGHGFYVCRIPLNWTIYVTDPLAAKTLLLKSENFPKNKAIFTALGDSSPVIKFMGKENVAMSNGEEWKKQRKIMNPAFHRSQPVKTFGNVMPDLFALIDQDPERVFITPKMKSFALDALGLSAFGFDFQSLKGDPEGWTRKYNVVISTLFNPFVNIFASLDFLVKYISPERRRVIKATDEFNSMLGELADKRRQEILDGEKKNIPENEKDLLTLMIEADIRDNIKTTTTELRHNMAIFFLAGHDSTANTLSLCLYNLAKHKHVQKKARQEVLAILGDEPLDVIPTAEDLKKLDYVNMVIKENLRRNGPADNLMSRDTQQDMNLNGTIIPKGSKVSVNVAAIHLNPKIWHDPENFIPERFEQGGEFEQHDGFTWIPFSNGSRQCLGLNFSLTEQRVVLCMILKRYEIDIPKDSIHYNEIVFDGAFTFAPQSLELSFKRRY

SEQ ID NO: 70 - DNA, 1545 bp, Rhizopus delemar
atggctttggaaggtgctttgcctttgttccaaaagagatccaaatcctcttatatcgttgccgccattttgttgattaccgtcaaacaaatctacagcttcttcagagttcctaccaacttgagacatttgccatgtgtttcttttttcgccatggccaaatctttgttgacttgtgaaccaccatacaacagattcaagagaattactttcccagccatccaagaaggtaacggtttttacgtttctaagattccaactggttggaccgtttatgttgctaatccagttgctgctaaacagctgctattgaagtctaacaatttccccaaatctcactacggtttggataccattggtgaaaaatctaccgctgttcaattcgttggtagagataacgttgttttgtccaacggtgaaatctggaaaaagcagagaaagatcatgaacccagttttccatagatccatgccaatcaaaactgttgcttctttggttcccttgttgttctctgcaattgaagaagcaaacggcagaattatgattacgccaaagatgaaggatttcactttggatgctttgggtttgaccatcttcgattttgattttaaagccttgcagggtgatccagataattggacttctatctacagattgatcaccaggtctatcttcgatccaatctcttacgttttctgtgctttggaacctttgttggtttacgtttacccaaagcgtagaagatctgttgatgctgttgctaagattaacgccaagttcgatcaagtcatctccaaaaaaagggaagaattgcagaacggcatcttctctaacaaaccagataacgaaaaggacttggtcaccttgatgttggaagctggtatgcaagaagatgtttctatcaccaacgaagaattgagacataacatggccgttttgtttttggctggtcatgattctacttccaacactttgtctttctgcttgtaccatttggctaaaaacaagagagcccaacagaagttgagagaggaaattatcaacatcttgggtgatgatgatatcgacatcgttccatccttggaagagttgaaacaaatgaagtacatgaacatggtcatcaaagaaaccttgagattgggtatgccattggatttgttgaccccaagaaaaacagttgaagatacctttgtcgccgatacctttattccaaaggataccgttattgctgttgacgctggtgcattgcatagagatcctagatcttggaaagatccagacgaatttgtcccagaaagattcgaagatgatggtgaacaaaactcccatgaaggtttgacttgggttccattttctaacggtactagacaatgtatcggcatgaacttctcattgatggaacagagattgaccctgactatgttgttgagaaagtacgaagttgatctgccaaaggattccatccattacgatcatatcatctacgaacaaccatcctacgtttgtccagaatctttggaattgatcttcaccaagaggtactaa

SEQ ID NO: 71 - protein, 514 aa, Rhizopus delemar
MALEGALPLFQKRSKSSYIVAAILLITVKQIYSFFRVPTNLRHLPCVSFFAMAKSLLTCEPPYNRFKRITFPAIQEGNGFYVSKIPTGWTVYVANPVAAKQLLLKSNNFPKSHYGLDTIGEKSTAVQFVGRDNVVLSNGEIWKKQRKIMNPVFHRSMPIKTVASLVPLLFSAIEEANGRIMITPKMKDFTLDALGLTIFDFDFKALQGDPDNWTSIYRLITRSIFDPISYVFCALEPLLVYVYPKRRRSVDAVAKINAKFDQVISKKREELQNGIFSNKPDNEKDLVTLMLEAGMQEDVSITNEELRHNMAVLFLAGHDSTSNTLSFCLYHLAKNKRAQQKLREEIINILGDDDIDIVPSLEELKQMKYMNMVIKETLRLGMPLDLLTPRKTVEDTFVADTFIPKDTVIAVDAGALHRDPRSWKDPDEFVPERFEDDGEQNSHEGLTWVPFSNGTRQCIGMNFSLMEQRLTLTMLLRKYEVDLPKDSIHYDHIIYEQPSYVCPESLELIFTKRY

SEQ ID NO: 72 - DNA, 1569 bp, Rhizopus microsporus
atggaccacttgatccaggtctacaactcttctactcaagttttgattccagtcttgcagaagagatctaaggcttcttatattaccgctgccattgctttgattattgcccaaagactgtactcctacttcagagttccaaaacatttgagaggtttcccaaagttgccatactttggtattgctaagtcattcttcgccaaagaatctccaagagaaagagtcaagaagtacatcttgccaatcatcaacgaaagagatggcttctacattagcaacattccatttggttggatgctgtacgttaccaatccaattgctgctaagcaaatcctgttgaagtctaacggttttccaaaaaaccacggtttgctagaagatatgggtgagaatttgttcatcgagttcatcggtaaggataacgttgttttgactaacggtgatacctggaagagacaaagaaaggttatgaatccagccttccatcattccttgcctattaagactatgtccaacgtcgttttctccttgatctccgttattgatcaagctaatggtactgttccagttgcttctactatgcaaaacttcaccttggatactttgggtttagccattttcggttttgactttaaggcattgcaaggtgatggtgatgaatggactaagacttacagattggtttccgattgcttgttcgacccaattatcaacgttttcagctcctactccttcatcttcgatagaatctacccaagacgtagaagaggtgctatggctactagaaaattgggtgaaaagttcttggaaatcgcccagcaaaaaaggatggaaatcaaatctggtgctttcgctgatgttccagataacgaaaaagatctgttgaccttgatgttggaagctgaagaaaaaggtgatgtctggacttctgaagatgaattgagacataacattgccgttttgttcttggctggtcatgatacaactgctcatgctttgtctttctgcttttaccatttggctaagaacaaggacatccagcagaagttgagaaaagaagttttggatttgttgggtgatgaaccagttgatgttgttccaactgttgaacaattgaaggacatgcagtacttgaacatggtcatcaaagaaaacctgaggatgaattctccagccgatatgttgttttccagagatgttcaagaggatatcgttttggctaacacctttattccaaagggtactgtcatctccattaacattgaagccttgcattgcaatccaaagttgtggcataatccagatcaattcgatccagaaagatttgctccaggtggtgaacatgaacaacatgaaggtatgacttggttgccattttctaacggtactagacaatgtctgggtatgaacttcagcttgtttgaacagagattggttatcgccatgatcttgaagaagtacgaaatctccattccagaggattccatccatagaaaccacatcattaacgacatgccattcaatgttgctcccaagtctttggaattgactttcactaagaggtactaa

SEQ ID NO: 73 - protein, 522 aa, Rhizopus microsporus
MDHLIQVYNSSTQVLIPVLQKRSKASYITAAIALIIAQRLYSYFRVPKHLRGFPKLPYFGIAKSFFAKESPRERVKKYILPIINERDGFYISNIPFGWMLYVTNPIAAKQILLKSNGFPKNHGLLEDMGENLFIEFIGKDNVVLTNGDTWKRQRKVMNPAFHHSLPIKTMSNVVFSLISVIDQANGTVPVASTMQNFTLDTLGLAIFGFDFKALQGDGDEWTKTYRLVSDCLFDPIINVFSSYSFIFDRIYPRRRRGAMATRKLGEKFLEIAQQKRMEIKSGAFADVPDNEKDLLTLMLEAEEKGDVWTSEDELRHNIAVLFLAGHDTTAHALSFCFYHLAKNKDIQQKLRKEVLDLLGDEPVDVVPTVEQLKDMQYLNMVIKENLRMNSPADMLFSRDVQEDIVLANTFIPKGTVISINIEALHCNPKLWHNPDQFDPERFAPGGEHEQHEGMTWLPFSNGTRQCLGMNFSLFEQRLVIAMILKKYEISIPEDSIHRNHIINDMPFNVAPKSLELTFTKRY

SEQ ID NO: 74 - DNA, 1452 bp, Syncephalastrum racemosum
atgttcagaccaccagcaggtttgccaaaattgccaattatcaattacttcaggttgctgtgggccttgtacagaaaagaatctccaactagaagatcccagagattgattttgccagccttgcaaaaacataacgctaaagcttacttggctaaggttccatatacttggactgtttacttggttgatccagttgctgttaagaccttcttgatgagaaatggtactttcccaaagaccatggaatccattgatgctttcgatcaatctcacccaaatgttcaattttggggtagagaaaacttgggtttctctgttggtgattcttggaagagacaacgtaagattatctttccagcttttagaagggctatgccagttcaattattcggtgaattggttccaaagatgttcgacttgatcgacaaagaacattccaccattgccatcgatttgatgcaaagattcaccttggatgctttgggtttagctgctttttctttcgatttccatgccttggataaccacaacaatgaatgggaagttgcctacgagatgatcagaaaagagttggtttctccactgactaacatgttggctagatacgattacatcctgaagtacattattccaggtagagctgaaaaacaagctgccgtttctaagatcaaccacttgttgtctgatattgccaacgagagaagaaagatgattaagaggaatcccgatatgttgaaggttccagattctgaaaaggacttgttgaccttgatgttggaatccgatttggaaaactctgatgatccagcttccgaagaattgattagagctaatttggctaccttcttcttggctggtcatgatacaactgctaacactttgtctttctggttgtaccatttggccatgtacaaggatattcaaaagaaggctagagaagaggtcattgaaactatgggtggtgctccagaagatatagttccaactgctgaacagctgaagaaaatgaagtacatggactgcatcatcaaagaaaacctgagattcatgggtccagctttggaattatttccaaggattgccaaagaggactacaacttgaacggtattttcatcccaaagggtactagagtttctgttgacttgcataccttacatcatcatccagatgtttggaaagaaccagagagatttgatccattgagattcgttgaaaacggcgaacattctaaacacgaaggtttgtcttggattgctttttcatctggtgctagagtatgcatcggtcaaaatttctcattggttgaacaaagggtcgtcatgtctatgttgttgagaagatacgaatgggacatcccagaagattccattcatagagaaggcttgcaattgaaggacaccaacaatcaagctccaagatcattggaaatcgtgttcaagaagaggtactaa

SEQ ID NO: 75 - protein, 483 aa, Syncephalastrum racemosum
MFRPPAGLPKLPIINYFRLLWALYRKESPTRRSQRLILPALQKHNAKAYLAKVPYTWTVYLVDPVAVKTFLMRNGTFPKTMESIDAFDQSHPNVQFWGRENLGFSVGDSWKRQRKIIFPAFRRAMPVQLFGELVPKMFDLIDKEHSTIAIDLMQRFTLDALGLAAFSFDFHALDNHNNEWEVAYEMIRKELVSPLTNMLARYDYILKYIIPGRAEKQAAVSKINHLLSDIANERRKMIKRNPDMLKVPDSEKDLLTLMLESDLENSDDPASEELIRANLATFFLAGHDTTANTLSFWLYHLAMYKDIQKKAREEVIETMGGAPEDIVPTAEQLKKMKYMDCIIKENLRFMGPALELFPRIAKEDYNLNGIFIPKGTRVSVDLHTLHHHPDVWKEPERFDPLRFVENGEHSKHEGLSWIAFSSGARVCIGQNFSLVEQRVVMSMLLRRYEWDIPEDSIHREGLQLKDTNNQAPRSLEIVFKKRY

SEQ ID NO: 76 - DNA, 1485 bp, Parasitella parasitica
atggccatcgaaaacttcatgcagtcttacaacagagccattgaaaacgtcttgccaatcttgagaaaaaggtctaaggcttcctatattggtatggccattatgtgcatcgttatcaagcaagtttactccgcttactctgttccaaaacacttgcaaagattccccaaggtttcattcttgtccatgatcagatcctacttgatcaaagaagccgttgtcgaaagaactaagagattggttactccattgactgatgctggtcatggtttttacgtctgtaaaattccattgacctggaccgtttttgttaccgatccaattgctgctaagaccttgttgttgaaaactgagtttttcccaaagtctcacgctttctttgatgctttgggtgataattctccagccgttcaatttttgggtagagaaaatgttgctgcctccaatggtgaaatctggaaaaagcaacgtaaattcatgaaccccgctttcttgagatcttctccagttaagactttctcctctgttacccacaacttgattaaggttatcgaaacccaatctgatgctgttccaattgcaaactgtatgaaggctttcactattgacgctttaggtttgtctgctttcggtttcgatttccaatctttgaatggtgatccagaaggttggactgaaacttacaatattgctattgccggtttgttcgacccattcattaacatctttgttaaggtcgacttcatgatgaactacatctcttctaagaggaagagaatcaacaaggccattaccagattcaactccatgttggaagatttggctaacaagagaaggcaagaaatcttgaacggtgaaactttgggtgttccagaaaacgaaaaggatttgttgaccttgatgatcgaagccgatattagagaaggttccagaactacttctaccgaattgagacataacattgccttgtttttcttggccggtcatgatacaactgctcatactttggctttttgcttgtacaacctggctaaaaacaaacacgttcaagctaaagctagagccgaagttttggatattttaggtgatgaacctaaggatgttgacccaactatggaagatctgaagagaatggattacctgaacatggttatcaaagaaaacttgagaagatgcggtccagttgacaagttgttgtctagagatactgccgaagatatcgatttgaacggtactttgattccaaagggccaaaagatctccatcgatttcaactctatccacatgaatccaaagttgtggcataacccagaagaatttgtcccagaaagatttgaaccaggtggtgaatttgatcaacatactggttttacttggctgccattttctcatggttctagacaatgtatcggcatgaacttttcattgaccgagcaaaaagtcctgttgtctatgatctgtaagagagccatcgaagagatctga

SEQ ID NO: 77 - protein, 494 aa, Parasitella parasitica
MAIENFMQSYNRAIENVLPILRKRSKASYIGMAIMCIVIKQVYSAYSVPKHLQRFPKVSFLSMIRSYLIKEAVVERTKRLVTPLTDAGHGFYVCKIPLTWTVFVTDPIAAKTLLLKTEFFPKSHAFFDALGDNSPAVQFLGRENVAASNGEIWKKQRKFMNPAFLRSSPVKTFSSVTHNLIKVIETQSDAVPIANCMKAFTIDALGLSAFGFDFQSLNGDPEGWTETYNIAIAGLFDPFINIFVKVDFMMNYISSKRKRINKAITRFNSMLEDLANKRRQEILNGETLGVPENEKDLLTLMIEADIREGSRTTSTELRHNIALFFLAGHDTTAHTLAFCLYNLAKNKHVQAKARAEVLDILGDEPKDVDPTMEDLKRMDYLNMVIKENLRRCGPVDKLLSRDTAEDIDLNGTLIPKGQKISIDFNSIHMNPKLWHNPEEFVPERFEPGGEFDQHTGFTWLPFSHGSRQCIGMNFSLTEQKVLLSMICKRAIEEI

SEQ ID NO: 78 - DNA, 1626 bp, Lichtheimia corymbifera
atggctgttgcttctccacagatcaagaacatggttactatggatagattgcaggacatctactctaccgtttctcaacacgttgttgctcatgcttcagctgttacttctagacaaagaaagatttccatttccgctgctgttgcattggttgctttttacactgtttacaaggttgttactccaccagctaacttgagacatattccatctatgggtttcttctcttacttgaacgctttcttgagaggtaagcaattgcacgatatctccaagaatgttgttttgccacatgccgttaatgttgataacggtgtttacttgagattcgacattttaggttggaccgttcatattgctagaccagaagctgctaagagattcttgttgaagtctgatattttcccaaaggccgacatgatttctgaaagaggtaatactttgttcggcaagttcgtgttcaacagaaacatcgttatgttgaacggtgatgattggaaggctcaaagaaaagttgctaatccagctttccatagagctatgccagttgaattattcggtagattgactcaaaagaccctgaaaaagatggaagaagaaatggacggcggtactttgaacttccatgatattacagaaaggtacaccttggaagttattggtttggctggttttgaatttgaattcggtgctatcgaaaacccaaagtctgaatgggttgatagataccagagattgattgaagctactttcaacccatggttcattgcttttccaaacttggacatgagatacaggtttttgttcccatctaggaagagattgcacagagaaatggatgctttcttggacaagatgtcccaagttattactcacaagagagagttgttgaaccaccaaaaaactaccgttccagaatccgaaagagatatcttgaccttgatgatcgaagctgaaaagaatggtgaaggttctatgaccaatgaagagttgcagaacaacctgctggtttttttcattgctggtcatgatacaacatccttggctttgtcttatgctgcttattacttggctgttaacccagatgttcaaagaaaggctagagaagaagccattagagttttgggtgatgctcctgaagatgttatgccaacagttgaacaaactagacagttgacctacatcaacatggtcatcaaagaaaccttgagaatgtctccaccattggctactattccagttagagaagctagtgaagataccgaattgtgtggtacttttatcccaaagggtacaagaaccttcttggatatctacgaaatccaacataacccaaccgtttggaaagatccagaaacttttaagcccgaaagattcaaaccaggtggtgaagctgaagaattagctggttctggtatgtcttggttgccattttctaatggttccagacaatgtatcggcctgaatttctcattggtagaacaaagggttttcctgccaatgttgctgagaaagtatgaatggcatttgccagaagattccatccacaaagaacgtattcaaacaatgggtttagccgtcattaagccaaaggatttgaagttgactttcaagaagaggtactaa

SEQ ID NO: 79 - protein, 541 aa, Lichtheimia corymbifera
MAVASPQIKNMVTMDRLQDIYSTVSQHVVAHASAVTSRQRKISISAAVALVAFYTVYKVVTPPANLRHIPSMGFFSYLNAFLRGKQLHDISKNVVLPHAVNVDNGVYLRFDILGWTVHIARPEAAKRFLLKSDIFPKADMISERGNTLFGKFVFNRNIVMLNGDDWKAQRKVANPAFHRAMPVELFGRLTQKTLKKMEEEMDGGTLNFHDITERYTLEVIGLAGFEFEFGAIENPKSEWVDRYQRLIEATFNPWFIAFPNLDMRYRFLFPSRKRLHREMDAFLDKMSQVITHKRELLNHQKTTVPESERDILTLMIEAEKNGEGSMTNEELQNNLLVFFIAGHDTTSLALSYAAYYLAVNPDVQRKAREEAIRVLGDAPEDVMPTVEQTRQLTYINMVIKETLRMSPPLATIPVREASEDTELCGTFIPKGTRTFLDIYEIQHNPTVWKDPETFKPERFKPGGEAEELAGSGMSWLPFSNGSRQCIGLNFSLVEQRVFLPMLLRKYEWHLPEDSIHKERIQTMGLAVIKPKDLKLTFKKRY

SEQ ID NO: 80 - DNA, 1578 bp, Choanephora cucurbitarum
atgttcactgaaaccgccttgcaaatctaccatcaaatggctgaaaaggtcttgccaattttgaagagacagccaaagtcatcttatattggtgctgctttggttttcttgttggttgctgaaattagaaggcaactgtccgttccaaaacacttgaaaaagttcccaaccattggtgtgttcaccttgatgaagtctttcatgagaaacgactccgttatcgaaagacacaatagattggttgctccaatcgttaagcaaggtcataagttttacgctgccaagattccatttgactggtctttgtctatagtcgatccagaaattgccaagatcatgttgatgaagagtgatgcttttccaaagtctcaaggtttcactagaaagttgggtgactcttcattgatcgttagattcactggtagagacaacgtgtctatttctaatggtcatgtctggaagaggcagagaaagtttatgaatccagctttcagaagaagcactccaatcaagacttttggtgaattgaccttgaagttcttcgattgcgttgatgaacaaccacaagattttccagctgccattaagttgaagaactacactttggatgctttgggtattgctgcttttgatttcgacttcaagtctttgtcaggtgatccagaaggttggactgaaatctacaacgttattatgaagggtatgttcgacccttgggtttttttgtttggtaagatggaattcatcctgcagtacatcattccatctaagagagaatgcattaagtccgtcgttaagttcaacaagatgttggttgaaatggccgataagagaaggcaagaaattcaaaacggtaagaagttgaacaccccaaactctgaaaaggatctgttgactttgatgatcgaagctgaaatggaagagggtattatgactaccaacgaagaactgagagaaaacattgccttgtttttcttggctggtcaagattctacaggcaactctttgtctttttgcttgtaccatttggccaagaacaagcacgttcaagataagttgagaagggaaatcatgtccgttatgggtgatagagatttggatgcaattccaaccgtcgaagattttaaggatatgccctacttgaacatggtcatcaaagaaaacttgaggttgtctggtccagctgatagatttttggatagagttgttgccgaagatatcgtcttaggtggtgaactaattccaaagggtactttgattaccgttgatgttgcctccattcattacaatccagaatattggcatgaccccgaagttttcattccagaaagatttgaacctaacggtgaattcgatcaacatgctggtgttgcttggttgccattttcaaatggtgctagacaatgtatcggcatgaatttctcattggctgaacaaagggtctttctgactatgttgttgagaagatacgaagtcggtatctccaaggattctatccattacgattccatcgtctacgaacaatcttttactttcgctccatctagcctgactttgaactttactaagctgaactaa

SEQ ID NO: 81 - protein, 525 aa, Choanephora cucurbitarum
MFTETALQIYHQMAEKVLPILKRQPKSSYIGAALVFLLVAEIRRQLSVPKHLKKFPTIGVFTLMKSFMRNDSVIERHNRLVAPIVKQGHKFYAAKIPFDWSLSIVDPEIAKIMLMKSDAFPKSQGFTRKLGDSSLIVRFTGRDNVSISNGHVWKRQRKFMNPAFRRSTPIKTFGELTLKFFDCVDEQPQDFPAAIKLKNYTLDALGIAAFDFDFKSLSGDPEGWTEIYNVIMKGMFDPWVFLFGKMEFILQYIIPSKRECIKSVVKFNKMLVEMADKRRQEIQNGKKLNTPNSEKDLLTLMIEAEMEEGIMTTNEELRENIALFFLAGQDSTGNSLSFCLYHLAKNKHVQDKLRREIMSVMGDRDLDAIPTVEDFKDMPYLNMVIKENLRLSGPADRFLDRVVAEDIVLGGELIPKGTLITVDVASIHYNPEYWHDPEVFIPERFEPNGEFDQHAGVAWLPFSNGARQCIGMNFSLAEQRVFLTMLLRRYEVGISKDSIHYDSIVYEQSFTFAPSSLTLNFTKLN

SEQ ID NO: 82 - DNA, 1530 bp, Absidia repens
atgggcacctcttacaaaagaaaggctgcttatgttactattggtgctgctgttgttttgctgttcagatctatctacggtttctactacgttccaaagtccttgagacatttgccatgtgttggttatagagaattggcctactctatcatgaagagggaagatgctgctactagagctagatctgttttgggtcaagctatcaaagaaaagaacggtgcttttgttgctaagttcccaatggaatggactgtttttttgacttccccaagaaccattcaagccgttttgttgaagtctgacaagtttccaaagacctacgatatgtttcatgccttgggtgaatcttctccattcgttaagtttttgggtatcaagaacgtcggtttctctaatggtgatgattggaagagacaacgtaaggttatgaatccagccttccaaagatctgttccagttgaaatgttcggtaagttgatgcaaaagggtattttggccattgaaaagcaaggttacgaagttagagctttggacttcttcgaaagaatcaccttggattccatcggtattttcttgttctctttcgacttcggttctttggataacccaaattctgtttggtctttgacctacgacactattagaaggggtattaagaatccagctttgaccgtttttccacaattggattgcttgttgaaatacgttactccaggtagaaggcatttggatcaatgtgttactaagctgaacaacctgttgatggaagtcgctaaagaaaaaagaaggcaagtccaatctccatccgataagttgattccagattccgaaaaggatctgttgaccttgattttggaagctgaattgagaggtgatggttctgcttctgatgaagaactaagaggtaatttggccttgttttttttggctggtcacgaaactactgcttccgctatgtgtttttgcttgtacaatttggccatgaacaaggacattcaagagaaggctagaaaagaagtgttggaagttttgggtgatgaaccagttgatgttagaccagatatccaagacttgaagcaattcaggtacatggatatgatcttgcacgaaaacttgagaagatttggtccagctgctatgttgttgccaagaaaatctgaagaggatttcgttgccgatggtattttgattccaaagaataccccagttgtcatcgatttgaacaccatgcatcataatccacaagtttggaaggatccagaaatctttgacccagaaagatttgctcctggtggtgaatatgaagctaacggtgaaaaaatggcttggttgccattttcttcaggttctagagtctgcatcggtaagtctttttctatggctgaacaaagggtgttcctgtcaatgttgttgaaaaagtacgaatgggatttcccagatgactccattcatagagatggcattaagatggaaaacttcgaaaacaacgctcccgaatctttgtcttttagatttcatccaaggtactaa

SEQ ID NO: 83 - protein, 509 aa, Absidia repens
MGTSYKRKAAYVTIGAAVVLLFRSIYGFYYVPKSLRHLPCVGYRELAYSIMKREDAATRARSVLGQAIKEKNGAFVAKFPMEWTVFLTSPRTIQAVLLKSDKFPKTYDMFHALGESSPFVKFLGIKNVGFSNGDDWKRQRKVMNPAFQRSVPVEMFGKLMQKGILAIEKQGYEVRALDFFERITLDSIGIFLFSFDFGSLDNPNSVWSLTYDTIRRGIKNPALTVFPQLDCLLKYVTPGRRHLDQCVTKLNNLLMEVAKEKRRQVQSPSDKLIPDSEKDLLTLILEAELRGDGSASDEELRGNLALFFLAGHETTASAMCFCLYNLAMNKDIQEKARKEVLEVLGDEPVDVRPDIQDLKQFRYMDMILHENLRRFGPAAMLLPRKSEEDFVADGILIPKNTPVVIDLNTMHHNPQVWKDPEIFDPERFAPGGEYEANGEKMAWLPFSSGSRVCIGKSFSMAEQRVFLSMLLKKYEWDFPDDSIHRDGIKMENFENNAPESLSFRFHPRY

SEQ ID NO: 84 - DNA, 1620 bp, Absidia glauca
atgccaatcgttaacgccttgcaaacctattcttatgaagaacctatcaacttcttgaaggacgtttggttgaacagattatttccagctggtacgtctaacagaaaaaaggctgctttgttgactttgggtgctactattgctttggtatgtagaactgtttacaggttgtacagagtcccaagatccttgagacatattccagctgttggttatgttgccatgttgagatctattttgaagagggaagatgctactactagagccatgactatttttcaaccagccatgaagaaaggtaacggtgtttttttggttaacttcccattggagtggtctatctatgttgctgaaccattggctgctaaagctgttttgatgaagtctgacaatttccccaagtccatcgatttcattcatgccttgggtaaagaaaacccagttgttaagtttttcggtactgataacgttgccttggttaatggtgaacaatggaagagacaacgtaaggttatgaatccagctttccatagagctatgccagttcaaatgttcggtaggttgttgcaaaagggtttcaagaacattgaagaacaaggtcatcaagttgctgccttggattttttccaaagattgacattggatgctttgggtcatgctgtttttggttttgattttggtgccttgaacgatagagaagctgtttggactgttacctacgaatccattagattgaacttgagaaacccattggctttcgcttttccatctatggattggttgttgaagtacgttattccaggtagattgcaaatggctgcttcagttgataagttgaacggtttgatgatggacatgatcaaagagaagaggatcaagttgttggaatcccaagctcaagatgatactccagaaaacgaaaaggatctgttgaccttgatgttggaagctgaacaaagaggtgaaggtactaccaatgatgaagaattgagatccaatatggccgtttttttcttggctggtcacgaaactactgctaacactatgtctttttgcttgtacaacttggccatggataagtccgttcaagaaaaagctagacaagaggttatcaaggttttgggtgatgaaccagaagatgttttgccaagaaacgaagagttgagacaaatcccatacctggatatgatcctgaaagaaaacttgcgtagatttggtccagcttctatgttgaatgctagaaagactgttgaggacttcgatatgaacggtacttttatcccaaagaacacctccgttatcgttgaaactaatgccttgcatcataacccagaagtttggaagaatccagaacaattcgatccagaaagatttgctccaggtggtgaacacgaaacttctcatgaaggtatggcttggttgccattttcttcaggttctagaggttgtttgggcatgaatttttcaatggcagaacagagggttttcctggctatgttgttgagaaagtatgaatgggacttgccaaaggattccatccataagaacggtattcaaatcggtaacttccaaaacgcttgtccagattctttgaagattcaattcaccccaaggtactaa

SEQ ID NO: 85 - protein, 539 aa, Absidia glauca
MPIVNALQTYSYEEPINFLKDVWLNRLFPAGTSNRKKAALLTLGATIALVCRTVYRLYRVPRSLRHIPAVGYVAMLRSILKREDATTRAMTIFQPAMKKGNGVFLVNFPLEWSIYVAEPLAAKAVLMKSDNFPKSIDFIHALGKENPVVKFFGTDNVALVNGEQWKRQRKVMNPAFHRAMPVQMFGRLLQKGFKNIEEQGHQVAALDFFQRLTLDALGHAVFGFDFGALNDREAVWTVTYESIRLNLRNPLAFAFPSMDWLLKYVIPGRLQMAASVDKLNGLMMDMIKEKRIKLLESQAQDDTPENEKDLLTLMLEAEQRGEGTTNDEELRSNMAVFFLAGHETTANTMSFCLYNLAMDKSVQEKARQEVIKVLGDEPEDVLPRNEELRQIPYLDMILKENLRRFGPASMLNARKTVEDFDMNGTFIPKNTSVIVETNALHHNPEVWKNPEQFDPERFAPGGEHETSHEGMAWLPFSSGSRGCLGMNFSMAEQRVFLAMLLRKYEWDLPKDSIHKNGIQIGNFQNACPDSLKIQFTPRY

SEQ ID NO: 86 - DNA, 1584 bp, Rhizopus microsporus
atggccttgaccgaaattgccattgaaacttatcatagagccttggataagctggttccaatcttgcaaaagagatctaagcactcctatattggtgttgctgttgttttggttgtcttggaaagaatctacagcttcttcagagttccaaagtccattagacatattccagccgtttcttactttgctatggctaagtctttgttgactgctgaagctccatcttctagatacaagagaatagttttgcccgtcgtcaaaaaaggtaatggcttgtacgtttctaagttgccattggaatggactgttcatgttgctactccaatgtctgctaaacacgttttgttgaagtctgagatctacccaaagtccgaatctttcttgaaattgctaggtccacaatctccagctgttttgtttttgggtgcttctaatgttggtttcgttaacggtcatatttggaagaaccagcgtaagattatgaacccagcttttcatagatccatgccaattcaaactatggcctctgttatgccagatttcttttccgctattgacaaacatggtactgatggtacaccaatttctgccgttatgagagatttcaccttggatgttttgggtcatactgcttttggtttcgatttcaaggctttgaaaggtgatccagatcattggactagaacctaccatattatcaacaacgctttgttcaacccaaccgctaatatgttgacttctttgaacccaatcctgtccattatctctccagaaagaagaagaattttggaggccatcaaaaagttgaacggtatgttggaagccatgatcaaacagaaaagacaagaagttcaaaacaacgcccaagccaatattccagaaaacgaaaaagatctgctgaccttgatgttagaagcccaacaaagaggtgaaggtttggctactgatgaagaattgaagcacaatgtctctggttttttcttggctggtcatgatacaacctctgaaactttgtctttctacttctacaacattgccaagaacaaggatgcccaaagaaagttgagagaagaattgtctactatcttgggtgataagccagttgatgttattccaaccttggagcaattgaagtccatggaatatttgaactgcaccatcaaagaaaacttgagattgaatggtccagccgataacattttgcctagaattgctactgaagatatggttgttgacggtactccaattccaaaaggtactgttgttaacgttgatatccacgccattcatcatgataccagatattggcaagatccctacaagtttgtccctgaaagatttttgccaggtggtgaacatgaatctcattctggtatgacttggttgccttttggtaatggtgctagacaatgtttgggtatgaatttctcattggccgaacagagattggttattgctatgactgttaggaagtacgacatcgaaattccaaaggattccatccattacgatcacccaattctggaatcttcatctacaaaagctccagcctctttgaagttggtttttagaaagaggtactaa

SEQ ID NO: 87 - protein, 527 aa, Rhizopus microsporus
MALTEIAIETYHRALDKLVPILQKRSKHSYIGVAVVLVVLERIYSFFRVPKSIRHIPAVSYFAMAKSLLTAEAPSSRYKRIVLPVVKKGNGLYVSKLPLEWTVHVATPMSAKHVLLKSEIYPKSESFLKLLGPQSPAVLFLGASNVGFVNGHIWKNQRKIMNPAFHRSMPIQTMASVMPDFFSAIDKHGTDGTPISAVMRDFTLDVLGHTAFGFDFKALKGDPDHWTRTYHIINNALFNPTANMLTSLNPILSIISPERRRILEAIKKLNGMLEAMIKQKRQEVQNNAQANIPENEKDLLTLMLEAQQRGEGLATDEELKHNVSGFFLAGHDTTSETLSFYFYNIAKNKDAQRKLREELSTILGDKPVDVIPTLEQLKSMEYLNCTIKENLRLNGPADNILPRIATEDMVVDGTPIPKGTVVNVDIHAIHHDTRYWQDPYKFVPERFLPGGEHESHSGMTWLPFGNGARQCLGMNFSLAEQRLVIAMTVRKYDIEIPKDSIHYDHPILESSSTKAPASLKLVFRKRY

SEQ ID NO: 88 - DNA, 1590 bp, Syncephalastrum racemosum
atgacccaattgactaccccagataccttaggtaagttgttggctatctatagacaaactccagcttcaagaagggcttcttggattggttgggctgttgctgctactgttattgcttctcaactgtacaaaactttggtcccaccatctaatttgccaaacttgccaactattaactacttcaggctgctgtcatctttcttgagaagagattctccaaccatcagatcccaagaaattttgattccagctttggaaaagcacgaacaaaagaaagcttacttggctaagttgccattgacttggactgtttttttggttgatccaattgccgccaagatcttcttgatgaagatggatattttccccaagatcaaagaaaccatcgatgccttggattctcaacatccaatcgttgaatttttcggtagagaaaacgttgccatctctgttggtgaagcttggagaaatcagagaaaggttatgaatccagctttcagacgtgctatgccaatttctattttcggcaacttgatgttcaaggtgttcaagaacatcgaagaaaacaagccagttatcgccatcgatttgatgcaagcttttactttggatgctttgggtagagctgctttctcttttgattttcacgctttggatgaccaacactccatttgggttgaaacctacgaaatcatcagacagtctttgagaaatccagctaatgctgttttggccagatacaacttcatcacgaaatatttgatgccaggtagagctaaacaaaaggctgctactcataagctgaacagcttgttgttggaaatggcttctagaaagagagccgaattggaaaaacatccagaattgagagaattgccagactccgaaaaagatttgttgaccttgatggttgaagccgatatggaatctggtgatgatccaacttctgccgaattattgagagctaacttgtccgtttttttcttggctggtcatgataccactgctaacactttgtcattttggttgtaccatatggccgttaacaaagatgtacaagctaaggctagagaagaggtcatcaagattttaggtgatggtcctgaagatgttatgccaactgctgatcaatgtaagcaaatgacttacctggactgcatcatcaaagagaatttgagattattgggtccagcctctcaattgattccaagaatggctaccgaagatgttgatttgaacggtattttcatcccaaagggtactagagttactgttgatatgcataccatgcactactctccaatgttgtggaaagatccaggtgtttttaagccagatagattcttggatgaaggtgaacactctcaacatagaggtttggcttggttgccattttcttcaggtggtagacaatgtttgggtatgaacttctcattgaccgaacaaagggttgtcatgtctatgatgttaagaaagtacacctgggaattgcctgccgattctattcatagagatggtgttaagttgaacgaagttaacactgttgctccaagaaccttgtccattatcttccaacaaagataccactaa

SEQ ID NO: 89 - protein, 529 aa, Syncephalastrum racemosum
MTQLTTPDTLGKLLAIYRQTPASRRASWIGWAVAATVIASQLYKTLVPPSNLPNLPTINYFRLLSSFLRRDSPTIRSQEILIPALEKHEQKKAYLAKLPLTWTVFLVDPIAAKIFLMKMDIFPKIKETIDALDSQHPIVEFFGRENVAISVGEAWRNQRKVMNPAFRRAMPISIFGNLMFKVFKNIEENKPVIAIDLMQAFTLDALGRAAFSFDFHALDDQHSIWVETYEIIRQSLRNPANAVLARYNFITKYLMPGRAKQKAATHKLNSLLLEMASRKRAELEKHPELRELPDSEKDLLTLMVEADMESGDDPTSAELLRANLSVFFLAGHDTTANTLSFWLYHMAVNKDVQAKAREEVIKILGDGPEDVMPTADQCKQMTYLDCIIKENLRLLGPASQLIPRMATEDVDLNGIFIPKGTRVTVDMHTMHYSPMLWKDPGVFKPDRFLDEGEHSQHRGLAWLPFSSGGRQCLGMNFSLTEQRVVMSMMLRKYTWELPADSIHRDGVKLNEVNTVAPRTLSIIFQQRYH

SEQ ID NO: 90 - DNA, 1569 bp, Rhizopus microsporus
atggaccacttgatccaggtctacaactcttctactcaagttttgattccagtcttgcagaagagatctaaggcttcttatattaccgctgccattgctttgattattgcccaaagactgtactcctacttcagagttccaaaacatttgagaggtttcccaaagttgccatactttggtattgctaagtctttgttgaccagagaatctccaagagaaagagttaagaagtacgtcttgccaatcatcgacgaaaatgatggtttctacatcagcaagattccattcggttggatgttgtacattgctaatccagttgctgctaagcagttgttgttgaaatcttctggttttccaaagaaccacggtttgttggataatatgggtgaaaacttgttcgtcgagttcatcggtaaagataacgttgctttgtctaacggtgatacctggaaaagacaaagaaaggttatgaacccagccttccatcattctttgcctattaagactatgtccaaggtcgtgttctctttgatttccgctattgaacaagccaacggtactattccagttgcatctgctatgcaaaacttcaccttggatactttgggtttagccattttcggttttgactttaaggcattgcaaggtgatccagatgaatggactaagacttacagattcgtttccgattgcatcttcgatccagttatcaacgttttctcctcctactccttcatcatcgatagaatctatccaagacgtagaagaggtgctattgctaccaaaaagttgtccgaaaagttcttgaagatcgcccaacaaaagcgtaaagaaatcaaatctggtgcttacgctgatgttccagataacgaaaaagacttgttgaccttgatgttggaagctgaagaaaaaggtgatacttggacctcagaagatgaattgagacataacattgccatcttgttcgttgctggtcatgatacaactgctcatgctttgtccttttgcttttaccatttggccaagaacaaggatgtgcaacagaagttgagaaaagaggtcttgtctatcttgggtgataagccagttgatgttgttccaactgttgagcaattgaagaacatgcagtacttgaacatggtcatcaaagaaaacctgaggattaactctccagccgatatgttgttttccagggatgtaaaagaagataccatcttggctaacaccttgattccaaaaggtactgttgttaccattaacatcgaagccttgcattacaatccaagattgtggcataatccagatcaattcgacccagaaagatttgctccaggtggtgaacacgaaaaacatgaaggtatgacttggttgccattctctaatggtactagacaatgtctgggtatgaacttcagcttgtttgaacagagattggttatcgccatgatcctgaaaaagtacgaaatctccattccagaggattccatccatagagatcatatcgtttctgacattccattcaatggtgctccaaagtctttgaagttgactttcactaagaggcactaa

SEQ ID NO: 91 - protein, 522 aa, Rhizopus microsporus
MDHLIQVYNSSTQVLIPVLQKRSKASYITAAIALIIAQRLYSYFRVPKHLRGFPKLPYFGIAKSLLTRESPRERVKKYVLPIIDENDGFYISKIPFGWMLYIANPVAAKQLLLKSSGFPKNHGLLDNMGENLFVEFIGKDNVALSNGDTWKRQRKVMNPAFHHSLPIKTMSKVVFSLISAIEQANGTIPVASAMQNFTLDTLGLAIFGFDFKALQGDPDEWTKTYRFVSDCIFDPVINVFSSYSFIIDRIYPRRRRGAIATKKLSEKFLKIAQQKRKEIKSGAYADVPDNEKDLLTLMLEAEEKGDTWTSEDELRHNIAILFVAGHDTTAHALSFCFYHLAKNKDVQQKLRKEVLSILGDKPVDVVPTVEQLKNMQYLNMVIKENLRINSPADMLFSRDVKEDTILANTLIPKGTVVTINIEALHYNPRLWHNPDQFDPERFAPGGEHEKHEGMTWLPFSNGTRQCLGMNFSLFEQRLVIAMILKKYEISIPEDSIHRDHIVSDIPFNGAPKSLKLTFTKRH

SEQ ID NO: 92 - DNA, 1569 bp, Mucor ambiguus
atgtactccaccgcctcttacaatcaaaccttggaaagagttgtttccgtcgtcagaaaaaacaagacctcttatattggtatggccatcttgtgtgttgtcttgcaacaaatctactcctcttttgctgttccaccaaaacacttgagaagattcccaaaggtttccttcatggaactgatgaagtccttctacaagaaagaatccgtcatgaacagaaacaagagattggttactccattgactaatgctggtcatggtttctacatttccagaattccattggattggaccatctacgttactgatccaattgctgctaagaccttgttgttgaaaactgacaatttcccaaagtctcatgctatttttggtgccttgggtgaatcttcaccagttgttaagtttatgggtaacgaaaacgttgccgtttccaacgatattctttggagaaagcaacgtaagattatgaacccagctttccatagatctcaaccagttaaggtttttggtggtgttatgccagatttgttcgccttgattgatcaagatccagaacatgttttcatcacgccaaagattaagtcctttgctttggatgctttgggtttgtctgcttttggtttcgatttccagtctttgaagaatgatccagaaggttggacttctaagtacaataccgttgtctcttctctgttcaacccattcgttaacttgttcgctaagtgcgacttcctgattaagtacatttctgccgaaagaagaagagtcatcaaggttactgatgaattcaacgccatgttgtctaacttggctgataagagaaggcaagaaatcatgaacggtgagaaaaagaacattgccgaaaacgaaaaggacctgttgactttgatgattgaagctgatacaagagaaggtgttgaaactactactaccgaattgagacataacatggccatttttttcttggccggtcatgatacaactgctaatactttggctttgtgcttgtaccaattggccaaacataagcacgttcaaaagaaggctagacaagaagttttggatatcttgggtgatgatccatgggatgttgctccatctttggaagatttgaagaagctgaactacctgaacatggtcatcaaagaaaacctgagaagaaacggtccagttgacaatttgatgtctagagatacccaacaggacatcaatttgaacggtacttttatcccaaagggttctaaggttgttatcaacgttgcctccattcatttgaacccaaagatttggcataaccccgaatctttcattccagaaaggtttgaacaaggtggtgaattcgattctcatgatggttttacttggctgccattttctaacggttctagacaatgtttgggcctgaatttctcattgactgaacaaagggttgctctgtgcatgttattgaagagatacgaaattgacatccccaaggattctatccattacgacgaaatcgttttcgataaggcttttactttcgccccacaatcattggaattgtccttcaaaaagaggtactaa

SEQ ID NO: 93 - protein, 522 aa, Mucor ambiguus
MYSTASYNQTLERVVSVVRKNKTSYIGMAILCVVLQQIYSSFAVPPKHLRRFPKVSFMELMKSFYKKESVMNRNKRLVTPLTNAGHGFYISRIPLDWTIYVTDPIAAKTLLLKTDNFPKSHAIFGALGESSPVVKFMGNENVAVSNDILWRKQRKIMNPAFHRSQPVKVFGGVMPDLFALIDQDPEHVFITPKIKSFALDALGLSAFGFDFQSLKNDPEGWTSKYNTVVSSLFNPFVNLFAKCDFLIKYISAERRRVIKVTDEFNAMLSNLADKRRQEIMNGEKKNIAENEKDLLTLMIEADTREGVETTTTELRHNMAIFFLAGHDTTANTLALCLYQLAKHKHVQKKARQEVLDILGDDPWDVAPSLEDLKKLNYLNMVIKENLRRNGPVDNLMSRDTQQDINLNGTFIPKGSKVVINVASIHLNPKIWHNPESFIPERFEQGGEFDSHDGFTWLPFSNGSRQCLGLNFSLTEQRVALCMLLKRYEIDIPKDSIHYDEIVFDKAFTFAPQSLELSFKKRY

SEQ ID NO: 94 - DNA, 1572 bp, Phycomyces biakesleeanus
atggacaccatcaaccacatctctccatctttcgaatcttacattaccgttttcgctaagatcgttccaaagggtttttatgttgttgctgctgttgctttgttcctgtgtaaaaaggtttacgattttaccgctgctccatacaagttgagacattttccaaaggtttctttcttcgccttctccaaatctattttctccgctgaatctgttgaacacagaactaagagattgatctctccactgttgcataagtacaagggtttctacattgctaagttcccattatactggactgttttcgttactgaaccacatgctgttcaatacgttttgatgaagggtgaaatcttcccaaaaaagaccagattcatgaacaccttgaacaaggactcattgatgattaggttgttcggctcctctaatattgcttttgcttctggtgaaatttggaagcaccaacgtaagattatgaacccagcttttcatagaactgccccaattgaattattcggtagaatgatcccagacatgttcagattgatcgataagtccaacggtaacattatgttggccgatttgttgcatagaattacctttgatgctatgggcaaagccttgtttggtttcgatttcaaaactgccagagaagaaaactctgaatggacttctgcttacaacgatgctatgtctggtatttctgctccaattttgaacatcaccccatccttggaacatatcactagatacttgtatccagattacgctaaggccaaaaagggtattgataagttgactgaattgaccttggaaatggtcaacgagaggaaagaaaagattcaagaagctatcggtcaaccagatgatggtagagaaaaggatttcttgaccttgattatcgaagccgaaatgaaggaagataaggcttctggttctggtggtttgagagaaaatttgaaggcttttttggttgctggtcatgcttctactgctagctctatttctttctgcatctaccatttggccatgaacaaagatgtccaaaacaaggcaagaaaagaagccttggatatcttgggtgatgatgctaatatttctaccccaaccgttaacgaatgtaagcacattacctacatcaacatgatcatcaaagaaacgttgagattgaacgctccattcggtactttgttcgaaagaattgctactgaagatgtcaccttgtccggtgtttttattccaaaaggtactatcatctccgtcgacattgaaaccattcataagaatccagccatttggaagtctccaactgtttttgatccagagagattttctaaaggcggtgaacatgaccaacatgaaggtattacttgggctccattttctgatggtaacagaaaatgcttgggcatcaatttctctatggctgaacaacaagtcatcctgctgatgttgttgaaacattacgaatgggacttgtccgaaaactccattcacaaaaatggtatcgtttacgacggcatctctttgtttactccaagatccttgtacatcaagttcaacaagagacactaa

SEQ ID NO: 95 - protein, 523 aa, Phycomyces biakesleeanus
MDTINHISPSFESYITVFAKIVPKGFYVVAAVALFLCKKVYDFTAAPYKLRHFPKVSFFAFSKSIFSAESVEHRTKRLISPLLHKYKGFYIAKFPLYWTVFVTEPHAVQYVLMKGEIFPKKTRFMNTLNKDSLMIRLFGSSNIAFASGEIWKHQRKIMNPAFHRTAPIELFGRMIPDMFRLIDKSNGNIMLADLLHRITFDAMGKALFGFDFKTAREENSEWTSAYNDAMSGISAPILNITPSLEHITRYLYPDYAKAKKGIDKLTELTLEMVNERKEKIQEAIGQPDDGREKDFLTLIIEAEMKEDKASGSGGLRENLKAFLVAGHASTASSISFCIYHLAMNKDVQNKARKEALDILGDDANISTPTVNECKHITYINMIIKETLRLNAPFGTLFERIATEDVTLSGVFIPKGTIISVDIETIHKNPAIWKSPTVFDPERFSKGGEHDQHEGITWAPFSDGNRKCLGINFSMAEQQVILLMLLKHYEWDLSENSIHKNGIVYDGISLFTPRSLYIKFNKRH

SEQ ID NO: 96 - DNA, 1515 bp, Phycomyces biakesleeanus
atgtgcctgttcttctgcaagaaggtttacgattttactgccgttccatacgagttgaagaagtttccaaatatccccttcttctacttcgtcaaatccatcttgtctgttgaatccgtcgaaaacagaactaagagattggttttgcctctgttgcataagaacaacggtttctacgtttctaggtttccattctactggactgttttcactactgatccagatgctgttcagtacttgttgatgaagggtgaaattttcccaaaggataccagattcacttccgctgtttctaaggattccttgattattaggctgttcggttcttctaacgttgcctttatttctggtgaaccattgaagcaccaatgcagaactatgaatccagctttcagaagaactgccccagttaacattttcggtagattgattccagacatgttcaggttgatcgataagtccgatggtgatatcttgatcgtcaacttgttgcaaagaatgacctttgatgctttgggtaaagctttgttcggtttcgatttcaagaccatgaaggaagataattctgcttggatgactgcttactctgatgctatgtctggtgttactgctccagttttgaacattattccatccttggagtacatcctgagatacttctatccaaactacaccaaggctaagaacggtgttgataagttgaacagattgatcttggagctggtcaacaagaagaagcaagaattggaagaatccatgccacaatcttgctctaacaacaacaatggtgatactgatggtgatgcttacgaccaagaaaaggatttgttgaccttgattttggaagccgaaatgaaggacaacaagtcatctggttctgatgatttgagagctaacatggctactttcattatggctggtcacgaaactactgcttcatctgtttctttctgcatctaccacatggttatcaacaaggatgttagagataaggctagaagagaagccttggatattttgggttacgatgatttcatttccccaccaactttcgatgaatgcaagagagttaactacatcaacatggttgtcaaagaggctttgagattgtgtactccaggtggtttgttgttcgaaagaattgctactgaggacgttttcttgtccggtgtttttattccaaagggcaccagaatttccgttgatattgaagccttgcacaagaatccagcaatttggaaaaacccatccgttttcgatccagagagattttctaaaggcggtgaacatgaacaacatagaggtattacttgggctccattttctgatggtaacagaaaatgcttgggcatcaacttctctatgactgaacaacaggtcatcctgctgatgttgttgaaacattatgaatgggacctgtccgaaaactccatccataacaatggtatggtttacgacaacgttttctccttcgctccaaaaaccttgtctatcaagttccataagaggcactga

SEQ ID NO: 97 - protein, 504 aa, Phycomyces biakesleeanus
MCLFFCKKVYDFTAVPYELKKFPNIPFFYFVKSILSVESVENRTKRLVLPLLHKNNGFYVSRFPFYWTVFTTDPDAVQYLLMKGEIFPKDTRFTSAVSKDSLIIRLFGSSNVAFISGEPLKHQCRTMNPAFRRTAPVNIFGRLIPDMFRLIDKSDGDILIVNLLQRMTFDALGKALFGFDFKTMKEDNSAWMTAYSDAMSGVTAPVLNIIPSLEYILRYFYPNYTKAKNGVDKLNRLILELVNKKKQELEESMPQSCSNNNNGDTDGDAYDQEKDLLTLILEAEMKDNKSSGSDDLRANMATFIMAGHETTASSVSFCIYHMVINKDVRDKARREALDILGYDDFISPPTFDECKRVNYINMVVKEALRLCTPGGLLFERIATEDVFLSGVFIPKGTRISVDIEALHKNPAIWKNPSVFDPERFSKGGEHEQHRGITWAPFSDGNRKCLGINFSMTEQQVILLMLLKHYEWDLSENSIHNNGMVYDNVFSFAPKTLSIKFHKRH

SEQ ID NO: 98 - DNA, 1536 bp, Phycomyces biakesleeanus
atgctggccaaaaaggttaatggttacgctggttttaccttggatgctattcaaaccatctacttcaacagagccatcaagttggttagaccaccaaaagctttgtcccatattccacatgttccatacttcagctacatgtcctcattgatcaagaaagagaacaccatctccagaaacaagagattcgctaacaagttgttcgaagatccagaatctaacggcttgtacttaagaccaaatgtcaaaggttgggaagttgttgttactagaccagaagatgccaagaagctgttgttcaagtctgatatttttccaaaggccgatttcacctctggtattgatggtactattctgtccaagttttctaggggtccaaacttgttgtttactactggtgctcattggaaggctcaaagaatggttgctaatccagcttttcatagatctgctccagttaagttgtttggtgaattgacccaaaagctgttcagagttatggataacagagctaacaagaccgttgatatcaccagattgatggaagcttgggctttagatgctattggtttggctggttttgatttcgatttcaacgctatcgaaaaccccaattcttcttgggttagaatctacgaaagagtcgataaggctttggttcatccattctactcatttttcccaaaagcagacaagtacctgttgtgggttttgccaaatagaaagcaagctcataccgatttggacatcttcttgaagatgatcgacaacgttattatcgccaagaaaaaagccttgcacgagaacaagtctaacaagcacttggaaaactccgaaaaggatttgttgaccttgatgttggaatctgaagctaagggttctactttgtccgctaaagaattgagatctaacatgtgcgtttttttcgctgctggtcacgaaactactgctaattctttggcttacgccatctatttcatggctgttaatccagatgttcaatgcaaggctagagaagaagcttttaaggttttgggtgatgcccaagaggatattatgccaactattgaacagaccaagagcatggattacattaacgccgttatcaaagaaaccttgagatcacattctccagctttgggtacttttgctagaaaagctactaaggacactgaattaggtggtgttttgattccaaaggacaccatgatttccatggatatcttcaacttgcatcacaatccaaacgtctggaacaacccagatgaatttgatccatctagatttttgccaggtggtgaagctgaaaagcaaatcaacaatggtttctcctggattccatttggtacaggtgctagacaatgtatcggcatgaatttcagcttgatcgaacaaagggttatgctgtctatgatgttgagaaagtttgcttggtctttgccagaagattccatccataaggattacttgcataccaccaacttggttatttcttccgctaaggatctgaacatcaacttcgaaaagctgtactaa

SEQ ID NO: 99 - protein, 511 aa, Phycomyces blakesleeanus
MLAKKVNGYAGFTLDAIQTIYFNRAIKLVRPPKALSHIPHVPYFSYMSSLIKKENTISRNKRFANKLFEDPESNGLYLRPNVKGWEVVVTRPEDAKKLLFKSDIFPKADFTSGIDGTILSKFSRGPNLLFTTGAHWKAQRMVANPAFHRSAPVKLFGELTQKLFRVMDNRANKTVDITRLMEAWALDAIGLAGFDFDFNAIENPNSSWVRIYERVDKALVHPFYSFFPKADKYLLWVLPNRKQAHTDLDIFLKMIDNVIIAKKKALHENKSNKHLENSEKDLLTLMLESEAKGSTLSAKELRSNMCVFFAAGHETTANSLAYAIYFMAVNPDVQCKAREEAFKVLGDAQEDIMPTIEQTKSMDYINAVIKETLRSHSPALGTFARKATKDTELGGVLIPKDTMISMDIFNLHHNPNVWNNPDEFDPSRFLPGGEAEKQINNGFSWIPFGTGARQCIGMNFSLIEQRVMLSMMLRKFAWSLPEDSIHKDYLHTTNLVISSAKDLNINFEKLY

SEQ ID NO: 100 - DNA, 1380 bp, Rhizopus microsporus
atggccatctcgttcttgtatagagaaggtccagctgaaagattgaagaggttgaaattgccagctatgagaaaaggtaacggcttctatttgtctagagttccattttgttggaccgtttacgttgctaatccaattgctgctaaacagttgttgttgaaggctgaaaatttccccaagtctcactttttgatggttggtaaggattccccattcgttcaatttttgggtccagataacgttgtcaactctaatggtgaaaactggaaaaagcagcgtaaggttatgaatccagctttccatagatcaatgccagttaagactattgccggtgttgttttgactttgttcgccgttattgataagtacaaaggtaaggttccagtcacctctactatgcaagaattcaccttggatgttttgggtttagccatcttcaatttcgacttcggttctttgaaaggtgatgctaaaaaatggcgtgctgagtacaaattggttatgttgtttgatccagtgaccaacgttttcactggtttcgattttttgctgaggtacatctaccctaagagaatcaaaggtgctaacgctgttaacaacctgaacaagttgttcgatcaattggtcaagcagaagagattggaagttcaatctggtgttcatgctaacaagccacaaaacgaaaaggatttgttgaccttgatgttggaagctgaacaaaggggtgaagctatgactactgatatggaaatgagacataacgtcgccgtttttttcttggctggtcatgaatctactgcccatgttttgtctttcaccttgtactttttggccaagaacaagtacgtgcaacagaagttgagagaagaggtttctagagttatgggtagaaagtctgttgatgttgctccaactttggaagaattgagacagatggaatacttgtacgccgtcatcaaagaatccttgagattgtgctctatcttcgacgttttgattttgagagatgccgtggaagatatgtacttggatgatacttttattcccaagggcaccagaattaccattgatgtttctgccattcagagagatccaaaggtttggaacaatccagatgatttcatcccagaaagattcatggaaggtggtgaagccgaaggtcatgaaggtatgacttggttgccatttggtggtggtgctagacaatgtattggtatgaatttctccctgaccgaacaaaaagttgctttggctatgttggttcagagatacgatattgatgttcccaaggactccatccattacgaagatattgcttacgaaaggccattttacttggctccacaatctttggaattgaccttcactaagttgcactaa

SEQ ID NO: 101 - protein, 459 aa, Rhizopus microsporus
MAISFLYREGPAERLKRLKLPAMRKGNGFYLSRVPFCWTVYVANPIAAKQLLLKAENFPKSHFLMVGKDSPFVQFLGPDNVVNSNGENWKKQRKVMNPAFHRSMPVKTIAGVVLTLFAVIDKYKGKVPVTSTMQEFTLDVLGLAIFNFDFGSLKGDAKKWRAEYKLVMLFDPVTNVFTGFDFLLRYIYPKRIKGANAVNNLNKLFDQLVKQKRLEVQSGVHANKPQNEKDLLTLMLEAEQRGEAMTTDMEMRHNVAVFFLAGHESTAHVLSFTLYFLAKNKYVQQKLREEVSRVMGRKSVDVAPTLEELRQMEYLYAVIKESLRLCSIFDVLILRDAVEDMYLDDTFIPKGTRITIDVSAIQRDPKVWNNPDDFIPERFMEGGEAEGHEGMTWLPFGGGARQCIGMNFSLTEQKVALAMLVQRYDIDVPKDSIHYEDIAYERPFYLAPQSLELTFTKLH

SEQ ID NO: 102 - DNA, 1581 bp, Phycomyces blakesleenanus
atggccaactcctctttcgaaaacctgcaatctttgttcgttgatttcgtccaaccacaattggtccaaagaaaaaaacaagccggtgttattttctccgccgttgttttggttttgtgttacaacaccatcaacaagatcatctacccaccaaagtccttgagacatattccacacgttaactacattgcctacaccagatcacaattgagaaaacaaccagcttctgaacaagctagagaactgttgttgccattattggctgaaaacaatggtttctacgccattccatttctaggtaagtggtctgttcaagttgctaacccaattgccattaagaccatcctgttgaagtttgacatgttcccaaaggctaactccttgtctaaatctcaaggtacattggcccatagattcattggtggtccaaatgtttttttgttggagggtaaaaagtggcgtaagcagagaatgatttctaacccagctttctctagatccatgccagttgatatgtttggtaggattaccatcaacctgtttaagtacttggataacatcgatccaaccatcgatgttttggataccatgaagaaatggaccttggatactttgggttctgctgtttttgatttcgacttcgaatctttgaccaagccaaacaatgaatggacctctatctactacgagattaacgcctctttgtttgtcccaatcttcaacattttgccagtcttggaaaagtccttcttgtggatgtttcctaagagaaaaagggttcacgataagatgaccaagttgaaggatatgatgagacaagtcatcatccaaaagcaggctaggttgaaagaaaacaaacccaatccaaacttgaaggacaccgaaaaggatttgttgaccttgttgttggaatccgaaaatgaaggtcatgagccaatgtctgaagatgagttgatgtctaatttgtgcgcttttttcttcgctggtcatgatacaactgctaacgctttatcttctgccttgtatcatttggctgttcaacaagacgttcaaaagaaagcaagagaagaagtcatcaacgttttgggtgatgaaccagaagatgtcattccatctattgaagataccagacagttggactacctgaacttgatcatcaaagaaaacatgaggatcaacccaccagttggtggaccattagatagattggttactgaagatatcgttttggacggtgttttgttgccaaaaggtacttctgttaaggttgccgtttactccttgcatagaaatccattattgtgggattccccagaagaattcagaccagaaagatttttgccaggtggtgaagctgataagattgaaggtatgggttacatcccattttctgatggtggtagacaatgtatcggtatgaacttctcattggttgaacaaagggttttgttggctatgatgttgagaaagtacacctggaagttgtctgagaacactattaacaaggacgaattgcaagtttacgcctttaacattatggccccattcgatttgaagatcactttggaaaagaggtactaa

SEQ ID NO: 103 - protein, 526 aa, Phycomyces blakesleeanus
MANSSFENLQSLFVDFVQPQLVQRKKQAGVIFSAVVLVLCYNTINKIIYPPKSLRHIPHVNYIAYTRSQLRKQPASEQARELLLPLLAENNGFYAIPFLGKWSVQVANPIAIKTILLKFDMFPKANSLSKSQGTLAHRFIGGPNVFLLEGKKWRKQRMISNPAFSRSMPVDMFGRITINLFKYLDNIDPTIDVLDTMKKWTLDTLGSAVFDFDFESLTKPNNEWTSIYYEINASLFVPIFNILPVLEKSFLWMFPKRKRVHDKMTKLKDMMRQVIIQKQARLKENKPNPNLKDTEKDLLTLLLESENEGHEPMSEDELMSNLCAFFFAGHDTTANALSSALYHLAVQQDVQKKAREEVINVLGDEPEDVIPSIEDTRQLDYLNLIIKENMRINPPVGGPLDRLVTEDIVLDGVLLPKGTSVKVAVYSLHRNPLLWDSPEEFRPERFLPGGEADKIEGMGYIPFSDGGRQCIGMNFSLVEQRVLLAMMLRKYTWKLSENTINKDELQVYAFNIMAPFDLKITLEKRY

SEQ ID NO: 104 - DNA, 1341 bp, Lichtheimia ramosa
atggataaccagacctggtctagtgttccaggtgcttcattttggaaaggcaaattggtttctggtcactacgttagggaagtgtttttgaacaacgatttcgacttcttgaaaggcactggtaagagattcgatactttgttgttgactgataccaccactcaagatgttgacatcgaagttttcagaaccgttgttatgaagcacttgaccaaagaaatgaaggcttacactccaagagttgttcaacatttgactgctggtggtgacgaaaaattgggtgatgctaaagaaccacaagaattggttcatctgttccctttgttacaacatatggttgctaaagcctccgcctctatttttgttggtactgaattggcttccgatgatgatgttgttgaaacctgtaagaacattgccatcgacattggttctgaattaggtccaggttcctatatcatggatgcttttccatctttggccagattgagaatgtggtacattggtaaatttggcaaggccattaacaagcacagacaacatttgttgagagctttgggtccagttattgataagagattggctgctgctgaaaaaggtggtgattgggatagaccacaagatatattgcaagacatcatcgaaaccatcaacttgactttggataacccaaagagacatatcttgccagttaagtggttgttggctttgttctttgcttctattcataccacctccgaaaactctactatcgtcttgtacagaatcatgcagaacccagaaatcatcgatgtcttgttggaagaacaaaaccaggtcttggaaaaacactacggttccaacattgattactccgataccactaagttgttcactggtgaagtcatcaaagagttggttaagttggattccttgtgcagagaagctatgagagctagaaattcctatttggaattgccacatacttacgtcggtaagtccagaattactttgtcatgcggtgctattattgaaccaggtcatgatgttttgatcaacatgtggggtaatcatagagatgccaaaattcaaagggataccatcggtgatcatcacgattttaagccattcagattcgttggtttggacagacaatctaccaagattggtgatgactttttgatgttcggtcaaggtagacatgcttgtccaggtagatggtttgctattcaagaaatcaagaccatcgtgtccgttttgattaggtactacaagttgactccaaacggtccaattacttttccaactcatccaagaatgccaatgcctatgggtcaagttataattcagagaaggcagtaa

SEQ ID NO: 105 - protein, 446 aa, Lichtheimia ramosa
MDNQTWSSVPGASFWKGKLVSGHYVREVFLNNDFDFLKGTGKRFDTLLLTDTTTQDVDIEVFRTVVMKHLTKEMKAYTPRVVQHLTAGGDEKLGDAKEPQELVHLFPLLQHMVAKASASIFVGTELASDDDVVETCKNIAIDIGSELGPGSYIMDAFPSLARLRMWYIGKFGKAINKHRQHLLRALGPVIDKRLAAAEKGGDWDRPQDILQDIIETINLTLDNPKRHILPVKWLLALFFASIHTTSENSTIVLYRIMQNPEIIDVLLEEQNQVLEKHYGSNIDYSDTTKLFTGEVIKELVKLDSLCREAMRARNSYLELPHTYVGKSRITLSCGAIIEPGHDVLINMWGNHRDAKIQRDTIGDHHDFKPFRFVGLDRQSTKIGDDFLMFGQGRHACPGRWFAIQEIKTIVSVLIRYYKLTPNGPITFPTHPRMPMPMGQVIIQRRQ

SEQ ID NO: 106 - DNA, 1593 bp, Hesseltinella vesiculosa
atgctgttccagtacatccatcatttggccgaaagattcgatcacaaaaagaccttggatcaattgcaaactttcgcttctactccagaaggtgctgttggtattactgctgctgttgctttggttgctggtgcttcttatttgaagaacaagaacaacgatagaggttgcccaaaagttccaggttcttctgtttggggtacttctactgaagagtatagagctgatccaaaggcttttatcgttaagtggcaaaatgaattgggtccagtttaccatgctgagttgtttggtcatactgctacagttgtttctggttcttacgtcagagaaatcttcttgaacgataagttcgatttcatggctggcttgcatagaactttcgataacatgttgttgaccaactgtggtccatacgaagatttgtctgctgctcatacttctgaagttgtcaagaagtttttgtcgccacatttgaaacatttcaccccaagagttatcgaacacttgcaacaaggtttgaaagctcaaaccggtgaaatttctgctgaaggtaaacaattcccacacgtttatggtttggttcaacatccagttgctttagcttcagcttctgtttttgttggtccagagttgtctaagaacgagttgttgattgactccttcaagaacatggttattgatgtcggttccgagttgttaccaaatccatggttggaaccatttccaagattgaacagattgagaatgtggtgggttggtaagacttcttctactgttaagagacacagaggtcaattggctactgctttgaaaccagaattggatagaagattgaaggctatggcttccaatgattctaattgggaaagaccagatgacatcttgcagaacttgttggaacattacactccaccaaaaggtatggataccttgaactacatggttaattggatgactcaattgactttcgctgctattcatacaacctctgaaggttctacttgggtcttgtacagattattacaaactccaggtttgtgggaagagttgtaccaagaacaaaacgaagttttggaagcctccggtattgattcttcagctggtgctgaagttttcaccagagaaattttgaacaagttcgttaagatggactccgtcattagagaaactatgagagctagaactgcctacattactttgccacatatcaacaagtccaacgaagtcgttactttgtctaatggtgctaaaatctacccaggtgaatccgcttatatcaacgtttggtctaatcacaatgacccctcattgcaaaattccatgaaggacttacaacagttcaagccattgagatttttggacgctgaaaagaactctaccaagatcggtgaagatttcctgtttttcggtatgggtaaacatgcttgtccaggtagatggtttgctgttcaagaaatcaaaaccatcgttgccttgttgttgagagagtacaaattggaagctgttggcgatttgtttttcccagaagttgaatccattccttttccaatgggtgaattcaagatctacccaagaaagcaagttgcctga

SEQ ID NO: 107 - protein, 530 aa, Hesseltinella vesiculosa
MLFQYIHHLAERFDHKKTLDQLQTFASTPEGAVGITAAVALVAGASYLKNKNNDRGCPKVPGSSVWGTSTEEYRADPKAFIVKWQNELGPVYHAELFGHTATVVSGSYVREIFLNDKFDFMAGLHRTFDNMLLTNCGPYEDLSAAHTSEVVKKFLSPHLKHFTPRVIEHLQQGLKAQTGEISAEGKQFPHVYGLVQHPVALASASVFVGPELSKNELLIDSFKNMVIDVGSELLPNPWLEPFPRLNRLRMWWVGKTSSTVKRHRGQLATALKPELDRRLKAMASNDSNWERPDDILQNLLEHYTPPKGMDTLNYMVNWMTQLTFAAIHTTSEGSTWVLYRLLQTPGLWEELYQEQNEVLEASGIDSSAGAEVFTREILNKFVKMDSVIRETMRARTAYITLPHINKSNEVVTLSNGAKIYPGESAYINVWSNHNDPSLQNSMKDLQQFKPLRFLDAEKNSTKIGEDFLFFGMGKHACPGRWFAVQEIKTIVALLLREYKLEAVGDLFFPEVESIPFPMGEFKIYPRKQVA

SEQ ID NO: 108 - DNA, 1572 bp, Phycomyces blakesleeanus
atgatcgagtacctgaaagaattcgtcgacaggattgattctaagaccttggaaaacgttaagtccttggccttttctaaagaaggtgccattggtatttctaccgccattattttgtcctccgcttacaattatcacaagtggtcctctagaaccatttctaatggttgtccaagagttccacataccttgccatttgttggtttgactagagtttaccgtaaggactctaaggctttttgtgaagaatggcatgctaaattgggtccagtttttagagcacacttgttcggtaaagaagttaccgttgtttctggtcactacgtcagagaagtttttttgaacaagcacttcgatttcgttaagggtgttgctaaggtttttgataccaggttgttgactgattccggttccagagaagattttactccagaagatttgagggaaatcatcacgaaatacttgaccccaaagttgaacttctacaccaagagagttatcaagagattgaagcaaggtgtcgaatcttctttgggtgataaggattccatcgaattggataacttgtacccattcgttcaacacttggttgttaatgcctctgcctctatttttgtcggtgaagaattgtcccaaaacaagttgttgatcgactccttcaagaacatggttagagatgtgggtaaagagatcaagcaaaatccatggtttgaaccctttccaaccatcaacaagtttaggatgtggttgattggtaagacctctccagttattaagaaccacaaagagcaactgttgaacgccattaagccagaagttgagtatagattgtctcaggctagatctaatccagactggaaaaaacctaccgatatgttgcaagacttgttggaaaattctaagccaccagctcatttggatttgatggatcatttggttcacatcatcacgttcttgatttttgttgccttgcataccacctctgaaaacactactgttttgttgtacaggatgttggagaatccagctatcgttgatgaattggtcatcgaacaacaagaagtcttggaacaagaaggtttggacgctaattgtggttccgaagttttcaccagagatatcttgaagaagttcgtcaagttggattctgtctgtagagaaaccttcagaatgaagaaccagtacatctctttgccacatgaatacgatggtaaggttccattgactttgtctaatggtgctgttattaacccaggtgaagatgttttgattgatgtttggactaaccaccagtacactgaagatgctaatgatgttgaagatgccgatcaattcaaggcctttagatttgttgatcaggacaagcaatctaccaaggttggtgaagattacttgttttttggtatgggtagacgtgcttgtccaggtagatggtttgctattcaagaagtccaaaccattttggccatgttggttcgtgagtataagtttatgccaaagggtccaatcgttttcccaactgaagaaagatctccaattccaaccggtaagtgtattatccagagaaagtga

SEQ ID NO: 109 - protein, 523 aa, Phycomyces blakesleeanus
MIEYLKEFVDRIDSKTLENVKSLAFSKEGAIGISTAIILSSAYNYHKWSSRTISNGCPRVPHTLPFVGLTRVYRKDSKAFCEEWHAKLGPVFRAHLFGKEVTVVSGHYVREVFLNKHFDFVKGVAKVFDTRLLTDSGSREDFTPEDLREIITKYLTPKLNFYTKRVIKRLKQGVESSLGDKDSIELDNLYPFVQHLVVNASASIFVGEELSQNKLLIDSFKNMVRDVGKEIKQNPWFEPFPTINKFRMWLIGKTSPVIKNHKEQLLNAIKPEVEYRLSQARSNPDWKKPTDMLQDLLENSKPPAHLDLMDHLVHIITFLIFVALHTTSENTTVLLYRMLENPAIVDELVIEQQEVLEQEGLDANCGSEVFTRDILKKFVKLDSVCRETFRMKNQYISLPHEYDGKVPLTLSNGAVINPGEDVLIDVWTNHQYTEDANDVEDADQFKAFRFVDQDKQSTKVGEDYLFFGMGRRACPGRWFAIQEVQTILAMLVREYKFMPKGPIVFPTEERSPIPTGKCIIQRK

SEQ ID NO: 110 - DNA, 1587 bp, Licthheimia ramosa
atgccaagcttgattccaaagaacgcttccgatgctattgaacagtacatctctagactgaaaaccatggatagaaggcacatgggtattattgctggttctgttgctgttgtttccttgtacactttctacagacatttgaccagatccagagatgatattccattggttccatatacctggccattgattggttctactccatcttttaacagagatccagttgcctttgttgagaagtggtcacaagaatatggtccagtttttagagcacacttgcaaggtagaatccaaactattattgccgccgaatacgttagagacatcttcatgaattccgacttcgattttttgttcgccgtcaacaaaagattcgatccacatttgttggccgatatcgatgataacactttcactaccgaaatgttgagaaaggtcgttatgaagttgactacccagttgaaatcttacactccaagagctgttgaattcttggatgttggtagaaacgaattcttgtctcattttccagctggtcctgttcatttgccacacttgtatccattgatccaacatatggttggtaaagcctctgctgctatttttgctggtacaaagttggcttctaacccagaagttgttgagtccttcaagaacattactttggaagttggtgctgaaatcgccgttgattctgtttttttggaaagatactggggcttgaacagattcagaatgtggttgatgggtaaattctccaagtccatgaagagacatcacagagttttgaaagatgccctaagaccagaaatcaaggatagaattgaagcctcttctgacccatctagagaaagaccagatgatatgttgcagatcatcatcgagtcttactacactgaaagaagaggtgaatccgttgatgatttgactgaagatttggtcaagtggctgatctctttgattttcgctgctattcataccacctctgaaaactctactgttgtcttgtacaggatcttgtctaagcctgatgttgttgaagagttgttggaagaacaaagagaagttttggttaggcatggtatttctccagacgaaaaagatccatctaagatgtttactggtgccgttattaaggacttggttaagttggattctgcttgcagagaaggtatgagaatgagaaacgattacttgactttgggtcatacctacttgggtaaaaagccaattacattgtcttgcggtgctgttatcaaaccaggtgaagatgttattatcaacacctggtacaaccaccgtaacaacaagatccaaaaaatccaaggtgacgactactctaactacaacccattcagatttgttggttccgatagacaagctgctagaattggtgatgatttcttgatcttcggtgaaggtaaacatgcttgtccaggtagatggtttgctctgcaagaaatgaagaccatcatctcgtttttgatcagggattacaaaatggctccagaaggtccaattactttcccaaagaatcctaagatgactttgccaatgggtcaagtgattttggaatccagacattaa

SEQ ID NO: 111 - protein, 528 aa, Lichtheimia ramosa
MPSLIPKNASDAIEQYISRLKTMDRRHMGIIAGSVAVVSLYTFYRHLTRSRDDIPLVPYTWPLIGSTPSFNRDPVAFVEKWSQEYGPVFRAHLQGRIQTIIAAEYVRDIFMNSDFDFLFAVNKRFDPHLLADIDDNTFTTEMLRKVVMKLTTQLKSYTPRAVEFLDVGRNEFLSHFPAGPVHLPHLYPLIQHMVGKASAAIFAGTKLASNPEVVESFKNITLEVGAEIAVDSVFLERYWGLNRFRMWLMGKFSKSMKRHHRVLKDALRPEIKDRIEASSDPSRERPDDMLQIIIESYYTERRGESVDDLTEDLVKWLISLIFAAIHTTSENSTVVLYRILSKPDVVEELLEEQREVLVRHGISPDEKDPSKMFTGAVIKDLVKLDSACREGMRMRNDYLTLGHTYLGKKPITLSCGAVIKPGEDVIINTWYNHRNNKIQKIQGDDYSNYNPFRFVGSDRQAARIGDDFLIFGEGKHACPGRWFALQEMKTIISFLIRDYKMAPEGPITFPKNPKMTLPMGQVILESRH

SEQ ID NO: 112 - DNA, 1584 bp, Absidia repens
atgctgacccagtacatccaccaattcttcaacaatttcgaccagaaaaagaccatggaccaattgcaatctgttgcctcttctaaggatggtgttattggtattgctaccgccttgattttgatttctggtgttgctgcttacaagtcctctactgttgaaagaggttgtccacaagttccatgtggtactttttctttcggttctacttctgagtacagagaaaatccagttgcctttgttaagaagtgggaagaaaaattgggtccagttttcggtgctcaattatttggtcaatacgctactatagtctctggtcctcaagttagagaaatcttctccaacgaaaacttctctttcatggccggtattcaaagagatttcgatacttacttgttggctaacggtggttccattcatgatttgccaccacatgttgtttctggtggtattaagaagaacctgtctccaaagttgccattctacacctctagagttatcgaacatttgaagatcggcttgtacgaacaatgtggtgttgttccagatgagggtaaagaattcgatcatgtttacccattcgttcaacatatggttgctaaagcttccgcttctgtttttgttggtccagaattggctaaggatttgaacttggttgactccttcaagaacatggttttggaagttggttctgatatgggtccaaagccatacttggaacattttccacatttgatgagactgaggatgtggtacattggtaagacttctacaaacgtcaagagacacagagatcaattattcgctgctttggttccacaaatcgactctagattgaaagccatgaaggaaaaggattccaattgggatagaccaaacgatttcttgcaggatattttggaaaccgatgattgtccacctcacatggatatctattcttactgtgttgattggatgacccaaattatctttgctgccttgcataccacatctgaaaatggtactattgtcctgtaccgtttgttggataatccaaaagtcttggaagagttgtacgaagaacaaaacgctgtattggaagaagctggttacgacgatactgttggtcctgaagttttcaccagagagattttgaacaagttcgtcaagatggactccgtcattagagaatcttgtagattgagaaacgactacattggtttgccacataccaatgttggtaagaaaaccatcgttttgtctggtggtgctatgattagaccaggtgaaaatgctttcgtcaacttctactcaaaccatagggatgagaagttgcaaaagtctggtatgaatgccaacaacttcgaaccatacagattcgttgatcagggtaagaactctaccaagattggtgatgatttcatgttcttcggtatgttcaaacatgcttgtccaggtagatggtttgctatccaagaaatcaagaccattttggccatgctgatcagatcttacaagatgtctgctatcgattccgttgttttcccaacttctgattacactagaattccaaccggtagattcaaaatcgtcccaagaaagtga

SEQ ID NO: 113 - protein, 527 aa, Absidia repens
MLTQYIHQFFNNFDQKKTMDQLQSVASSKDGVIGIATALILISGVAAYKSSTVERGCPQVPCGTFSFGSTSEYRENPVAFVKKWEEKLGPVFGAQLFGQYATIVSGPQVREIFSNENFSFMAGIQRDFDTYLLANGGSIHDLPPHVVSGGIKKNLSPKLPFYTSRVIEHLKIGLYEQCGVVPDEGKEFDHVYPFVQHMVAKASASVFVGPELAKDLNLVDSFKNMVLEVGSDMGPKPYLEHFPHLMRLRMWYIGKTSTNVKRHRDQLFAALVPQIDSRLKAMKEKDSNWDRPNDFLQDILETDDCPPHMDIYSYCVDWMTQIIFAALHTTSENGTIVLYRLLDNPKVLEELYEEQNAVLEEAGYDDTVGPEVFTREILNKFVKMDSVIRESCRLRNDYIGLPHTNVGKKTIVLSGGAMIRPGENAFVNFYSNHRDEKLQKSGMNANNFEPYRFVDQGKNSTKIGDDFMFFGMFKHACPGRWFAIQEIKTILAMLIRSYKMSAIDSVVFPTSDYTRIPTGRFKIVPRK

SEQ ID NO: 114 - DNA, 1605 bp, Lichtheimia corymbifera
atgtacaccctggtgtctttcttgaaggaccaaaacattattgccgttttgaagaacgctattcacgctcaacaacaaggtactactgcttcctctattaccattttgtctttggctgttgctattaccactttcgccgttcatagaattaggctgtattccgtaaaagaacacggtgttccattggttccatatgttttgcctttcattggttcttcaccagagtacagaaaagatccaaaggcttttttggaaaagtggactgctaaattcggtccagtttttagagcccatattttcggtagagtttacaccattatctccggtcattacgtcagagaagttttcttgaacgaggacttctcattcgaagttggtatgggtaaaactttcgatggttggttgattaccgataccaaaaagtctgagttgttctctacaccattggtcagatctatggttatgaagcacttagccgttgatgttaagaactatactccaagagctgttgagcatttgactattgctgctagagaaatgttgggtgatatcggtgaatctaaagaattgccacacttgtacccattgatccaacatatggtttctaccgctattgcctctattttggttggtttgaaaatctgcaaggacaaggatttgttggagacttttaagaacgttgccgtcgatattggttctgaattgaatccagattcctacttgtacgaagctttcccaactatctctagattgagacaatggtacttgggtaaatacggtaaggctattaacaagcaccaagagcatatgttgagagttttgggtccagaaattgacgaaagattggctgctatggaacgtggtgatggtggatgggaaagaccagaagatattttacaaggtattctggaaaccgccaagttgacttctgatcatccacaaagatatatggtcccaatcaagtggttcctgattttggtttttgcttccattcataccacctctcaaaacactacagttgctatgtataggttgttgcagcatccagaagttattgacgaactgttggaagaacaaaaccaggtctttgaaaaacaccacggttctaactacgatgatcatgatattaccaagttgttgaccggtgaagttattaaggatttggtcaagttggattccgtctgtagagaagctatgagaatctcttctttctacgctgaattgcctcatacttacatcggtaaatctccattgactatgtccaacggtactattatcaatccaggtgatgatgtcttgatcaacggttacactaaccatcatgatccagatatccaaattgatggtggtggtgattatgctgaattcaagccattcagattcgtcgaaaaaggtagacaatctaccagaatcggtgatgactacttgattttcggtcaaggtaaacatgcttgtccaggtagatggtttgctatgcaagaaatgaagaccaccatctcgtttttgatcagacagtacattattaccgccaagggtgacattatgtttttgaagggtcatagacaaaagatccctatgggtcaagttatcttccagaagagatga

SEQ ID NO: 115 - protein, 534 aa, Lichtheimia corymbifera
MYTLVSFLKDQNIIAVLKNAIHAQQQGTTASSITILSLAVAITTFAVHRIRLYSVKEHGVPLVPYVLPFIGSSPEYRKDPKAFLEKWTAKFGPVFRAHIFGRVYTIISGHYVREVFLNEDFSFEVGMGKTFDGWLITDTKKSELFSTPLVRSMVMKHLAVDVKNYTPRAVEHLTIAAREMLGDIGESKELPHLYPLIQHMVSTAIASILVGLKICKDKDLLETFKNVAVDIGSELNPDSYLYEAFPTISRLRQWYLGKYGKAINKHQEHMLRVLGPEIDERLAAMERGDGGWERPEDILQGILETAKLTSDHPQRYMVPIKWFLILVFASIHTTSQNTTVAMYRLLQHPEVIDELLEEQNQVFEKHHGSNYDDHDITKLLTGEVIKDLVKLDSVCREAMRISSFYAELPHTYIGKSPLTMSNGTIINPGDDVLINGYTNHHDPDIQIDGGGDYAEFKPFRFVEKGRQSTRIGDDYLIFGQGKHACPGRWFAMQEMKTTISFLIRQYIITAKGDIMFLKGHRQKIPMGQVIFQKR

SEQ ID NO: 116 - DNA, 1563 bp, Syncephalastrum racemosum
atgaacgccttgttgcaaagacaggataagatgagagatttcctgaacactagagaaggtgtttacggtattactgctgctgttgctgttgttttgatttccgcttattctttgagaagaaccgtctacacctctagaagaaaagacgaaattgctaccgttccatacaagttgccattgaaaggttctactgaagagtatagagctgatccaagagctttcgttgaaaagtacgctaaaatgtacggtccagtttacagagcttacttgtttggtgaaatgatgaccatcgtttccgattcttacgtcagagaaatcttcttgaacgacaacttcaacttcttccaagccgttaaggatagattcgatatggttaagttgtgcaactgcgctaatgatgaaggtcatggtattgctgatatcgtcaagagatgtttgaacccaagattggatatgtacaccgaaagagtcaacgaacaattagaggaagcctccaaagaaatcttgactgaagttgataccaagggctctcaagaattgatgcacatgtacattttggtccaacatatggttgctagagcttccgctactgtttttgttggtccagaattggctaagaactccgaattgattgactccttcaagaacatggttatccaagtcggttctcaactaagaccaaatccatggttggaaccatttccaagattgaactcattgaggatgtggtacattggtaagacttctccagttgttagaaagcacagattgcaattgagatctgctgttaagccatccatcgatgatagattggctagacaaaagtctcaaggtaacgcttttcaaagaccagacgatttgttgcaggatatcattgaaagacatccagaagccaagaccaagtctgatatctatgattacgttgttgataccttgaccgctttgatttttgctgcattgcataccacctctgaaaactctactgttgtcttgtataggttgttgcagcatcctgaattgatggaagaattggttgctgaacaagatgccgttttgttggaacacggtttgccaaaagattcttctgctagagttatgaccagacagatgatcaagaagttcgaaaagttggattctgtctgcagggaatctttcagattgagaaatgattacttgggtttgccacatacctacgaaggtaaaaaggatatcgttttgtctaacggtgccattattaagccaggtgaaaaggctattatcaacttgtggggtaatcatcattctggtaacactccacaatctacctctcaagattatttcggtttcgacccatacagattcgttaagcaagataagcaagctaccaagatctctgaggattttttgtttttcggtttgggtaaacatgcttgcccaggtagattttttgctgtccaagaagctaaggttctgatctctgttttgttgaggaactacaagttgtcaccagttgatccaccatactttgctactgatgataccatgaagattccagccggtagaattagaatcgaaagaaggtaa

SEQ ID NO: 117 - protein, 520 aa, Syncephalastrum racemosum
MNALLQRQDKMRDFLNTREGVYGITAAVAVVLISAYSLRRTVYTSRRKDEIATVPYKLPLKGSTEEYRADPRAFVEKYAKMYGPVYRAYLFGEMMTIVSDSYVREIFLNDNFNFFQAVKDRFDMVKLCNCANDEGHGIADIVKRCLNPRLDMYTERVNEQLEEASKEILTEVDTKGSQELMHMYILVQHMVARASATVFVGPELAKNSELIDSFKNMVIQVGSQLRPNPWLEPFPRLNSLRMWYIGKTSPVVRKHRLQLRSAVKPSIDDRLARQKSQGNAFQRPDDLLQDIIERHPEAKTKSDIYDYVVDTLTALIFAALHTTSENSTVVLYRLLQHPELMEELVAEQDAVLLEHGLPKDSSARVMTRQMIKKFEKLDSVCRESFRLRNDYLGLPHTYEGKKDIVLSNGAIIKPGEKAIINLWGNHHSGNTPQSTSQDYFGFDPYRFVKQDKQATKISEDFLFFGLGKHACPGRFFAVQEAKVLISVLLRNYKLSPVDPPYFATDDTMKIPAGRIRIERR

SEQ ID NO: 118 - DNA, 1584 bp, Absidia caerulea
atgctgaccgagtacatccatcacttcatcaacaatttcgaccagaaaaagaccatggaccaattgcaaactatggtgtcatctaaagaaggtatgattggtttggctactgctgctgttttgatgtctggtgctgcagtttacaagtctaccagaattgaaagaggttgtccacaagtcccaaatcagtcttactttatgggttctaccaaagagtacagaaacaatccagctgcctttatcgaaaagtgggaaaaagaattgggtccagtttatggtgcttacttgtttggtcagtacactactgttgtttctggtcctcaagttagggaagttttcttgaacgatgacttcgatttcattgccggtatcagaagagatttcgataccaacttgttgtctaacggtggtgatttgagagatttgccagttcataagtttgccggttccattaagaagaacttgtctccaaaattgcccttctacacctccagagttattgaacatttgaagatcggcctgaaagaattctgtggtgttgttccagatgagggtaaagaattcgatcatgtttacccattggttcaacatatggttgctaaagcttccgcttctgtttttgttggtccagaattggctaagaacgaacaattgattgactccttcaagaacatggttttggaagtcggttctgaattggctccaaaaccttacttggaattcttcccaaatttgatgagactgaggatgtggttcattggtaagacttctcaaaaggtcaagagacacagagatcaattgagagctgctttggctccacaagttgagtatagattgaaagccatgaaggaaaacgattccaattgggatagaccaaacgatttcttgcaggacattttggaatctggtgatattccagctcatgttgatgttactgatcattgctgtgattggatgacccaaattatctttgctgccttgcataccacatctgaaaatggtactttgtccttctacaggttgttggataatccaaaggtcttggaagatttgttggaagaacaaaaccaggtgttagaagatgctggttacgattcttctgttggtcctgaagttttcaccagagaaatcttgaacaagttcgtcaagatggactccgttattagagaaacctctagattgagaaacgactacattggtttgccacacaagaacatttcttctaagaccattactttgtctggtggtgctatgattagaccaggtgaaagagcttacgttaacgcttattctaaccacagagatggtactatccaaaaggttaccgataacttgaagtccttcgaaccatacagattcgttaaccaggatagaaactctaccaagatcggtgaagatttcatctttttcggtatgggtaagcacgcttgtccaggtagatggtttgctattcaagaaatcaagaccatcattgccatgatgatcagatcctatcaattgtctgctttgggtcctgttactttcccaactgatgattactctagaattcccatgggtagattcaaaatcgtgccaagaaagtaa

SEQ ID NO: 119 - protein, 527 aa, Absidia caerulea
MLTEYIHHFINNFDQKKTMDQLQTMVSSKEGMIGLATAAVLMSGAAVYKSTRIERGCPQVPNQSYFMGSTKEYRNNPAAFIEKWEKELGPVYGAYLFGQYTTVVSGPQVREVFLNDDFDFIAGIRRDFDTNLLSNGGDLRDLPVHKFAGSIKKNLSPKLPFYTSRVIEHLKIGLKEFCGVVPDEGKEFDHVYPLVQHMVAKASASVFVGPELAKNEQLIDSFKNMVLEVGSELAPKPYLEFFPNLMRLRMWFIGKTSQKVKRHRDQLRAALAPQVEYRLKAMKENDSNWDRPNDFLQDILESGDIPAHVDVTDHCCDWMTQIIFAALHTTSENGTLSFYRLLDNPKVLEDLLEEQNQVLEDAGYDSSVGPEVFTREILNKFVKMDSVIRETSRLRNDYIGLPHKNISSKTITLSGGAMIRPGERAYVNAYSNHRDGTIQKVTDNLKSFEPYRFVNQDRNSTKIGEDFIFFGMGKHACPGRWFAIQEIKTIIAMMIRSYQLSALGPVTFPTDDYSRIPMGRFKIVPRK

SEQ ID NO: 120 - DNA, 1584 bp, Absidia caerulea
atgttcacccaatacctgcatcagttgttcactaacttcgaccaaaaaaagaccatggaccacttgcattctctggtttcttctaaagaaggtgctattggtttggctactgctgctgttttgatgtctggtgctgcagtttacagatcttctatgatggatagaggttgtccagttgttccatctggtttgtttactttgtcatctactgctgagtacagacaagatccagcttctttcattaagaagtggcagaaagaattgggtccagtttatggtgcttacttgtttggtcaatacgttaccgttgtttccggttctcaagttagagaaattttcctgaacgagaacttctccttcatcgatggtatttccagagatttcgatacctacttgttggctaatgctggtacttatcatgatttgccaacttccactattgccgacatgattaagaagaacttgtctccaaagttgcagttctacaccggtagagttattgaacatttgaagatggccttgcatgaacaatgtggtgttgttccagctgaaggtaaagaattcaatcacgtttacccattcgttcaacatatggttgctaaagcttccgcttctgtttttgttggtgttgaattggctaagaacgaagccttggttgattctttcactaacatggttttagaagttggtggtgctttgggtccaaaaccttatatggaatacttccccaacttgatgaagttgcatatgtggtacattggcaagacttccaagaacgttaagagacaccaagaccaattgagatctgctttgaaaccagaaatcgacactagattgaaggccatgaaggaaaaagattcctcttgggttagaccaaacgatttcttacaagacttgttggaaaccgatgaatgcccagatcatattgacatctactccagagttatctactggatcacccaaattatctttgctgccttgcataccacatctgaaaatggtactttggccttgtataggttgttggataatccagaattattcgaggacttgtacgaagaacaaaaccaggtcttggaacaagctggttatgatagatctgttggtccagaagttttcaccagagaaatcttgaacaagttcgtcaagatggactccttgattagagaaacctctagattgaggaacgagttcatttctttgccacatatgaacacctccaacaagactattactttatcaggtggtgccatgattagaccaggtgaaaatgttttcattaacttctacgccaaccaccacgacgaaaaattgcaaaaagttgctgacaatttgggcaagttcgaaccatacagattcgttaatcaagacaagaactctaccaaggtcggtgaagattttgtttttttcggtatgggtaagcacgcttgtccaggtagatggtttgctattcaagaaatcaagaccatcatctccatgttgatcagagactacaaaatctctccattgggtcctgttgttttcccagtttctgattacactagaattccaaccggtagattcaaaatcgtcccaagaaagtga

SEQ ID NO: 121 - protein, 527 aa, Absidia caerulea
MFTQYLHQLFTNFDQKKTMDHLHSLVSSKEGAIGLATAAVLMSGAAVYRSSMMDRGCPVVPSGLFTLSSTAEYRQDPASFIKKWQKELGPVYGAYLFGQYVTVVSGSQVREIFLNENFSFIDGISRDFDTYLLANAGTYHDLPTSTIADMIKKNLSPKLQFYTGRVIEHLKMALHEQCGVVPAEGKEFNHVYPFVQHMVAKASASVFVGVELAKNEALVDSFTNMVLEVGGALGPKPYMEYFPNLMKLHMWYIGKTSKNVKRHQDQLRSALKPEIDTRLKAMKEKDSSWVRPNDFLQDLLETDECPDHIDIYSRVIYWITQIIFAALHTTSENGTLALYRLLDNPELFEDLYEEQNQVLEQAGYDRSVGPEVFTREILNKFVKMDSLIRETSRLRNEFISLPHMNTSNKTITLSGGAMIRPGENVFINFYANHHDEKLQKVADNLGKFEPYRFVNQDKNSTKVGEDFVFFGMGKHACPGRWFAIQEIKTIISMLIRDYKISPLGPVVFPVSDYTRIPTGRFKIVPRK

SEQ ID NO: 122 - DNA, 1461 bp, Phycomyces blakesleeanus
atggccatcatcttgtcctctgtttacaactatcataagtggtcctccagaaccatttctaatggttgtccaagagttccacataccttgccattttttggtttgaccaaggtttaccgtaaggattctaaggctttttgcgaagaatggcatgctaaattgggtccagtttttagagcacacttgttcggtaaagaagttaccgttgtttctggtcactacgtcagagaagtttttttgaacaagcacttcgacttcatcaagggtatcgttaaggtttttgataccaggttgttgaccgataacggttctagagaagattttccaccagaagatttgagggaaatcatcactaagtacttgaccccaaagttgaacatctacactagaagattgatcaagcagttgaagcaagacgtcgaaaacattttgggtttgatcgagttcgataacttgtacccattcgttcaacacttgatcgttaatgcttccgcctctattttcttgggtgaagaaaattcccagaacaagttgttgatcgacagcatcaagaacatggttagattggttggttccgaagttaagcaaaacccatggattgaaccattcagcccaatcaaaaagatcagaatgtgggttattggtaagacctctccagttatcaggtcctacaaagaacaattgattaacgccatcaagccagttgttgagtacagattgtctgaagctagaagaaatccagactggaaaaaacctactgatgtgttgcaagacttgttggaaaattctaaaccaccagctcacatggatttgatggattacttggtctgcattatcaccatcttgattttcgttgccttgcattccactattgaaaacactaccgttctgttgtacaggatcttggaaaacccagaaatcatggatgaattggacttggaacaaagggaagtcattgaacaagaaggtttggataccaattgtggctctgaattattcaccagagacatcttgaagaagttcaccaaattggattctgtctgcagagaaaccttcagaatgaagaaccagtacatcactttgccacatgaatacgatggtaaggttccattgactttgtctaatggtgctgttattaacccaggtgatgatgttttgattgatgtttggaccaaccacaggtacaagaaagaaactacttctgttaaggatgccgacgaattcagaccattcagatttgttaatcagaacaagcagtctaccaaggtcggtgaagattacttgttttttggtatgggtagacatgcctgtccaggtagatggtttgctatgcaagaaattcaagctattaccgccatcttggttagagaatgcaagtttattccaaagggcccaattatctttccaaccgctgaaagatctccaattccaactggtagatgtatcatccagagaaagtga

SEQ ID NO: 123 - protein, 486 aa, Phycomyces blakesleeanus
MAIILSSVYNYHKWSSRTISNGCPRVPHTLPFFGLTKVYRKDSKAFCEEWHAKLGPVFRAHLFGKEVTVVSGHYVREVFLNKHFDFIKGIVKVFDTRLLTDNGSREDFPPEDLREIITKYLTPKLNIYTRRLIKQLKQDVENILGLIEFDNLYPFVQHLIVNASASIFLGEENSQNKLLIDSIKNMVRLVGSEVKQNPWIEPFSPIKKIRMWVIGKTSPVIRSYKEQLINAIKPVVEYRLSEARRNPDWKKPTDVLQDLLENSKPPAHMDLMDYLVCIITILIFVALHSTIENTTVLLYRILENPEIMDELDLEQREVIEQEGLDTNCGSELFTRDILKKFTKLDSVCRETFRMKNQYITLPHEYDGKVPLTLSNGAVINPGDDVLIDVWTNHRYKKETTSVKDADEFRPFRFVNQNKQSTKVGEDYLFFGMGRHACPGRWFAMQEIQAITAILVRECKFIPKGPIIFPTAERSPIPTGRCIIQRK

SEQ ID NO: 124 - DNA, 1608 bp, Lichtheimia corymbifera
atgtacaaggccttcttggacaacggtatcgtttcctctattatctctaccttggataacaaggacatctccgtttttttgaacgatccaaaccatgctaagaccagatctgttgctttggtttctttctgtactgttattgctgcttacgccttgtctagatcaagatctcattctaaggataaggataccccaatggttccatatacttggccattgattggttcttctagagaataccgtaaagatcctgaagcctttatcaagaagtggtcatctgaattgggtgatgtttacaaggttcacttgttcggtagaatccaaactgttgtttccggtaaacacgtttactgcttgcaaaaggatttcgactttcaacagggtatgtctaagaccttcgatatctggttgttgttggatgctccattaggtggtagattcactttggataagattagacatgccaccatcaagttcaccagaactaagatgttgactaacactccatgcgttgtcaagcaattgattgctgctgaacacgaaatgattggtgatgctcaaactccatctgaaattgctaacttgtacccattgatggaacacttggttgctattgcttccgctactaattttgttggtccaggtttgaccaaagataaggatttggttgaaacctacaagcacttggctgttgatgttggttcagaattaggtgatggtaacgaattcttggaagctttcccatggatttccagattgagaatgtggtacttgggtaaatacggtaactctgttgataagcacagaaagcgtttgttgagagctatgaagccaattatcgacgaaagattggctgctgcagaaaacggtattgaaaatccacaagatttcatccaggacatcatcgaagaatccgaaattacttctggtgatccagacaagtacattttggcagttagatggatcttggttatgattgcttctgctggtcataccactactgaaaacactaccattatcctgtacagaatcttgcaacacccagaagtcattgacgaactattggaagaacaaagacaggtcttggaaaaacatcatggtccagatgttaaggataacgaagatttggctactttgttcactggtgaagttattaaggacttggtcaagttggattctgtctgtagagaaaccatgagattgaggtccttctacattgatttgccacatacctacgttggtaaatctccattggctttgactaatacctgtaccattaagccaggtgaagatgtcttgttgaatatgtggttgaaccataacagaaccgccatgcaatatgatggtttgggtgattacaatgagttcaagccattcagatttgtcggtttggatagatcctctactaagttaggtggtgactttttgttgttcggtttgggtactcatgcttgtccaggtagatggtttgctatgcatcaaactaagaccatcctgtccatgttgttgagaagataccaaattactccccaagaaaccatcgttttcccaattggtaatagatcccatgttccatctggtaaggttacctttcaaaagagacagtaa

SEQ ID NO: 125 - protein, 535 aa, Lichtheimia corymbifera
MYKAFLDNGIVSSIISTLDNKDISVFLNDPNHAKTRSVALVSFCTVIAAYALSRSRSHSKDKDTPMVPYTWPLIGSSREYRKDPEAFIKKWSSELGDVYKVHLFGRIQTVVSGKHVYCLQKDFDFQQGMSKTFDIWLLLDAPLGGRFTLDKIRHATIKFTRTKMLTNTPCVVKQLIAAEHEMIGDAQTPSEIANLYPLMEHLVAIASATNFVGPGLTKDKDLVETYKHLAVDVGSELGDGNEFLEAFPWISRLRMWYLGKYGNSVDKHRKRLLRAMKPIIDERLAAAENGIENPQDFIQDIIEESEITSGDPDKYILAVRWILVMIASAGHTTTENTTIILYRILQHPEVIDELLEEQRQVLEKHHGPDVKDNEDLATLFTGEVIKDLVKLDSVCRETMRLRSFYIDLPHTYVGKSPLALTNTCTIKPGEDVLLNMWLNHNRTAMQYDGLGDYNEFKPFRFVGLDRSSTKLGGDFLLFGLGTHACPGRWFAMHQTKTILSMLLRRYQITPQETIVFPIGNRSHVPSGKVTFQKRQ

SEQ ID NO: 126 - DNA, 1596 bp, Hesseltinella vesiculosa
atgctgacccaatacttgcaattcgctgctgatagattgggtcaaaaaaagaccttggatcaattgcaagctgttgtcacttctaagcaaggtgttgttggtattactactgctgttgctttgattgctttggccaatcattttagatccccaaagattgatagaggttgcccacaagttgaaggtaaaggttggtttggttatgctaccgaagaattcagagaaaacccaggtaagtttttgtctgaatggcacgaaaaattgggtccagtttacggtgttaagatctttggtcattacgctactgttgtttctggtccatatgtcagagaagttttcttggatgacaggttctctttcattgctgctattaccaagttgttcgacccaaacttgatgactgattctggtcattcttctgaacaaactgctaagaatgctgccgattccattaagagatttctgtctccaaatctgaagcactacaccccaagagttattgaacatttgaacttgggtatcgaagattggtgtggtgaagttccagctgaaggtattgaaattgaaaacgctttcccattcttgcaacatttggttgctagagcttcagcttctgttttcgttggtattgaattggccaagaacgaagaattggttgactctttccaaaacatggtgtccaacatttcttctggtttgaaacctaaaccttggttggaatactttccctccttgaccaaattgggtatgtacatgattggtaagactaacccagctgttaagagacatagaactcaaatggctaacgccttaagaccagaagttgatagaagattgaaagccatggcctctaatgataccaattgggatagaccagatgatatgttgcagcacattttggaatcttatccagctcctgaaggtttggatgttattacctatttgatcaactggatgacgcagttgatttttgctgcattgcataccacatctgaaaacggtaaagttgtcttgtacagattgctacaacacccagaagtcatggaagaattatacgctgaacaaaacgaagttttggctgctgctggttatgatgaatctgctggtccagaagtttttgacagagagatgttgaacaagttcgtcaagttggattctgctgttagagaagcttgtaggttgaagaatgaattcgttggtttgccacacgaaaacactactgataagactttgactttgtccaacggtgctgttattttgccaggtgaatttgtttacatcaaccagttcgttaaccacagggatccagaattacaagctgctattgatgatgtccatcagttcaaaccattcagattcgtaggtactgatcataacgctgctaaagtttccgaaggttttgtcttttttggtatgggtagacatgcttgtccaggtagatggtttgctattcaagaaatcaagaccatcgtgtccttgttgttgagaaagtacaaggttgaacctatcgacccaatcgtgttctctaatcaagaaagagatgcctttccaattggtccatgcagaattagattgacaccaagaaaagccctgtaa

SEQ ID NO: 127 - protein, 531 aa, Hesseltinella vesiculosa
MLTQYLQFAADRLGQKKTLDQLQAVVTSKQGVVGITTAVALIALANHFRSPKIDRGCPQVEGKGWFGYATEEFRENPGKFLSEWHEKLGPVYGVKIFGHYATVVSGPYVREVFLDDRFSFIAAITKLFDPNLMTDSGHSSEQTAKNAADSIKRFLSPNLKHYTPRVIEHLNLGIEDWCGEVPAEGIEIENAFPFLQHLVARASASVFVGIELAKNEELVDSFQNMVSNISSGLKPKPWLEYFPSLTKLGMYMIGKTNPAVKRHRTQMANALRPEVDRRLKAMASNDTNWDRPDDMLQHILESYPAPEGLDVITYLINWMTQLIFAALHTTSENGKVVLYRLLQHPEVMEELYAEQNEVLAAAGYDESAGPEVFDREMLNKFVKLDSAVREACRLKNEFVGLPHENTTDKTLTLSNGAVILPGEFVYINQFVNHRDPELQAAIDDVHQFKPFRFVGTDHNAAKVSEGFVFFGMGRHACPGRWFAIQEIKTIVSLLLRKYKVEPIDPIVFSNQERDAFPIGPCRIRLTPRKAL

SEQ ID NO: 128 - DNA, 1554 bp, Nicotiana sylvetris
atggtgtctccagttgaagctatcgttggtttggttactttggctttgttgttctacttcatcaggaccaagaaatcccaaaaaccatctaaaccattgccaccaaaaattccaggtggttggccagttattggtcacttgttttacttcgatgatgactccgatgatagaccattggctagaaaattgggtgatttggctgataagtacggtccagtttttactttcagattgggtttgccattggtcttggttgtttcatcttacgaagctatcaaggattgcttctctaccaacgatgctatcttttctaatagaccagctttcttgtacggtgagtatttgggttataacaacgccatgttgttcttgactaagtatggtccatattggaggaagaacagaaagttggttatccaagaggttttgtgcgcttctagattggaaaaattgaagcacgttaggttcggtgaaatccaaacctctattaagaacttgtacaccagaatcgacggtaactcttctactattaacttgaccgattggctggaagagttgaattttggtttgatcgttaagatgatcgccggtaagaattacgaatctggtaaaggtgatgaacaggtcgaaagattcagaaaggctttcaaggatttcatcatcctgtccatggaattcgttttgtgggatgcttttccaattcctttgttcaagtgggttgatttccaaggtcatgttaaggctatgaagagaaccttcaaggatatcgactctgttttccaaaactggttggaagaacacgtcaaaaagaaagaaaagatggaagttaacgccgaaggtaacgaacaagatttcatcgatgttgtgctgtccaagatgtctaacgaatatttggatgaaggttactccagagataccgttattaaggctactgttttctccttggttttggatgctgctgatactgttgcattgcatatgaattggggtatggccctgttgattaacaatcaacatgctttgaagaaggcccaagaagaaatcgacaaaaaggttggtaaagacagatgggttgaagagtccgatattaaggatttggtttacttgcagaccatcgtcaaagaagttttgagattatatccaccaggtcctttgttggttccacacgaaaatgttgaagattgcgttgtttccggttaccatattccaaagggtactagattattcgccaacgtcatgaagttgcaaagggatccaaaattgtggtctaacccagataagttcgatccagaaagatttttcgctgccgatattgatttcagaggtcaacattacgaattcatcccatttggttctggtagaagatcttgtccaggtatgacttatgctatgcaagttgaacatttgactatcgcccatttgatccaaggtttcaattacaagactccaaacgatgaaccactggatatgaaggaaggtgctggtttgacaattagaaaggttaacccaatcgaagttgtcatcactccaagattgactccagagttgtactga

SEQ ID NO: 129 - protein, 517 aa, Nicotiana sylvestris
MVSPVEAIVGLVTLALLFYFIRTKKSQKPSKPLPPKIPGGWPVIGHLFYFDDDSDDRPLARKLGDLADKYGPVFTFRLGLPLVLVVSSYEAIKDCFSTNDAIFSNRPAFLYGEYLGYNNAMLFLTKYGPYWRKNRKLVIQEVLCASRLEKLKHVRFGEIQTSIKNLYTRIDGNSSTINLTDWLEELNFGLIVKMIAGKNYESGKGDEQVERFRKAFKDFIILSMEFVLWDAFPIPLFKWVDFQGHVKAMKRTFKDIDSVFQNWLEEHVKKKEKMEVNAEGNEQDFIDVVLSKMSNEYLDEGYSRDTVIKATVFSLVLDAADTVALHMNWGMALLINNQHALKKAQEEIDKKVGKDRWVEESDIKDLVYLQTIVKEVLRLYPPGPLLVPHENVEDCVVSGYHIPKGTRLFANVMKLQRDPKLWSNPDKFDPERFFAADIDFRGQHYEFIPFGSGRRSCPGMTYAMQVEHLTIAHLIQGFNYKTPNDEPLDMKEGAGLTIRKVNPIEVVITPRLTPELY

SEQ ID NO: 130 - DNA, 2121 bp, Lictheimia ramosa
atggctcaatctccaccagcattggatactttggatatcgttttcttgggtactatcggtttgggtacaattgcttggtttgctagaaggcaaattgctgaaagattattcggttccacctcttcctctgatgctaaatctaatggtcatgctactccagctccaccaaaaagagaaagaaacttcgttaagatcatgcaagagcaaggtagaaaggtcattttcttctacggttctcaaactggtactgctgaagattacgcttctagattggctaaagaatgctctcaaaagtacggtgttaactgtatgactgctgatttggagttgtacgacttgtcttacttggatactgttccagaagattgcctggtttttttcgttatggctacttatggtgaaggtgaacctactgataatgctgttgatttctgggatgtcttgtctgaagaagaaccacaattttctgaagccgaaggtgataagccattgcaaaatttgagatacttggttttcggcttgggtaacaagacttacgaacattataacgctgttgccagaaacgttgacaagagattggaagttttgggtgctcatagaattcatgaacgtggtgagggtgatgatgatggttctttggaagaagattttttggcctggcaagaaaacatgtggccagctttttgtgaagctttgggtgttgatgaatctaacgctcattctggtccaagacaagctacttattctgttgaagaattggtcgatgtcaacatggatgatgtttacttgggtgaattggccgaaaaacctaaagaaggtgctagagttatctacgatgctaagaggccttttaatgctccaattgccatttctcaagacttgttcactaacaccgatagacattgcttgcacatggaaatcgatatctccgattccaacttgtcataccaaaccggtgatcatattgctatttggccaactaactccgaaaacgaagttgctagactggcttctattttgggtttagctgataagttggataccgccatcaatgttaaggctattgatccagctgcttccaaaaagtacccatttccttgtccagctacttacagagctattttcagacattacttggacatttgcgctgccgtttctagacaatctttgatggcttttgttgaatacgctccaaccgaagaatccaaagaaagattgagacaattggccaaggataaggatgagtacagattgactgttggtgaagctgttagaaatttgggtgaagtattggaaatcgttgctggtaatgatgttaagccaggtttcttttcttccgttccattcgatttggttgtcgaatctatttccagattgcaacctaggtactactccatttcttcatctgcaaaagagtccccaaaaaagatcgctgttactgctgttacattgtcctatcaaccagatccaactccacaaagaactgtttatggtgtcaacactaattacttgtggcgtattcataccgcctctaagcaacaatctactgaagctgatttgccaacctatgatttgtcaggtccaagaaatgctttacatggtactaagttgccagttcacgttagaagatctcaattcaagttgccaagaaacccaaccgttccagttattatggttggtccaggtactggtgttgctccttttagaggttttgttagagaaagagccttgcagaaatctgaaggtaaaccagttggtccaactttgttgtttttcggttgtagaaactccgaacaggacttcttgtacaaagatgaatggcctgctttgtttgacaccttaggtgaatcctctagaattattaccgccttctcaagagaaaccgctcaaaaagtttacgtccagcatagattgcaagagaacggtcaagaagtttggggtttgttgcaaaggggtgcttatatctatgtttgtggtgatgcaaagaacatggccagagatgttcaacaaactttcgttaacttcggtatcgaattcggtggtttgtctgatgataaggctcatgattttgtcaagaacttgagaaacaccggtagataccaagaagatgtttggtcttga

SEQ ID NO: 131 - protein, 706 aa, Lichtheimia ramosa
MAQSPPALDTLDIVFLGTIGLGTIAWFARRQIAERLFGSTSSSDAKSNGHATPAPPKRERNFVKIMQEQGRKVIFFYGSQTGTAEDYASRLAKECSQKYGVNCMTADLELYDLSYLDTVPEDCLVFFVMATYGEGEPTDNAVDFWDVLSEEEPQFSEAEGDKPLQNLRYLVFGLGNKTYEHYNAVARNVDKRLEVLGAHRIHERGEGDDDGSLEEDFLAWQENMWPAFCEALGVDESNAHSGPRQATYSVEELVDVNMDDVYLGELAEKPKEGARVIYDAKRPFNAPIAISQDLFTNTDRHCLHMEIDISDSNLSYQTGDHIAIWPTNSENEVARLASILGLADKLDTAINVKAIDPAASKKYPFPCPATYRAIFRHYLDICAAVSRQSLMAFVEYAPTEESKERLRQLAKDKDEYRLTVGEAVRNLGEVLEIVAGNDVKPGFFSSVPFDLVVESISRLQPRYYSISSSAKESPKKIAVTAVTLSYQPDPTPQRTVYGVNTNYLWRIHTASKQQSTEADLPTYDLSGPRNALHGTKLPVHVRRSQFKLPRNPTVPVIMVGPGTGVAPFRGFVRERALQKSEGKPVGPTLLFFGCRNSEQDFLYKDEWPALFDTLGESSRIITAFSRETAQKVYVQHRLQENGQEVWGLLQRGAYIYVCGDAKNMARDVQQTFVNFGIEFGGLSDDKAHDFVKNLRNTGRYQEDVWS

SEQ ID NO: 132 - DNA, 1083 bp, Papaver somniferum
atggaaactcctatactaattaagttgggaaacggtctaagtattccttcagtgcaggagttagcaaaattaacattagcggagatcccaagccgatacacgtgcaccggcgaatccccattgaataacatcggtgcttcagtcaccgatgacgagaccgttcccgtcatcgacctacagaacttgctttctccagagccggtagtaggaaagttggagttagataagttacacagcgcatgcaaggagtggggtttctttcagctagtaaatcacggagtagatgctttactaatggataatattaagtccgagataaagggcttctttaatctgccaatgaatgagaagaccaaatacggacagcaagacggggatttcgagggcttcggccaaccttacatcgagagcgaggaccagcgtcttgactggacagaggtattttccatgctctcactgccacttcacctgaggaagccgcatttattccctgaattgccgctgccttttagagaaactctagaatcttatctatcgaaaatgaagaagttatcgacggtggttttcgaaatgttagagaagagcctacagctagtcgagattaaaggaatgacagacttattcgaggacggccttcagacaatgcgtatgaactactatccaccatgtcccagacctgagctagttttaggtttgacgtctcactcagacttttcaggtctgaccatcctgttacaactgaatgaggtcgaaggtctacagatacgcaaagaggagagatggatctctataaagcccctacccgacgctttcattgtgaatgtgggagatatattggagataatgacgaacgggatatacagatccgttgagcaccgcgctgtcgtaaactcaaccaaggaaaggttgagtatagctacgtttcacgattcgaaattagagagcgagataggccctattagttccttagtcactcccgagaccccggccttattcaaaagagggcgttacgaggatatacttaaagaaaacttaagtcgaaagctggatgggaaatcatttcttgattacatgcgaatgtag

SEQ ID NO: 133 - protein, 360 aa, Papaver somniferum
METPILIKLGNGLSIPSVQELAKLTLAEIPSRYTCTGESPLNNIGASVTDDETVPVIDLQNLLSPEPVVGKLELDKLHSACKEWGFFQLVNHGVDALLMDNIKSEIKGFFNLPMNEKTKYGQQDGDFEGFGQPYIESEDQRLDWTEVFSMLSLPLHLRKPHLFPELPLPFRETLESYLSKMKKLSTVVFEMLEKSLQLVEIKGMTDLFEDGLQTMRMNYYPPCPRPELVLGLTSHSDFSGLTILLQLNEVEGLQIRKEERWISIKPLPDAFIVNVGDILEIMTNGIYRSVEHRAVVNSTKERLSIATFHDSKLESEIGPISSLVTPETPALFKRGRYEDILKENLSRKLDGKSFLDYMRM